European Patent Application EP 4 219 722 A1, published August 2, 2023. Title: Inducable expression vector for production of recombinant protein in methanotroph. Applicant: Korea Research Institute of Bioscience and Biotechnology. The sequence listing filed with the application follows.

SEQUENCE LISTING (73 sequences)

SEQ ID NO: 1 - DNA, 1692 bp, Artificial Sequence
  dmpR
atgccgatcaagtacaagcctgaaatccagcactccgatttcaaggacctgaccaacctgatccacttccagagcacggaaggcaagatctggcttggcgaacaacgcatgctgttgctgcaggtttcagcaatggccagctttcgccgggaaatggtcaataccctgggcatcgaacgcgccaagggcttcttcctgcgccagggttaccagtccggcctgaaggatgccgaactggccaggaagcttagaccgaatgccagcgagtacgacatgttcctcgccggcccgcagctgcattcgctcaagggtctggtcaaggtccgccccaccgaggtcgatatcgacaaggaatgcgggcgcttctatgccgagatggagtggatcgactccttcgaggtggaaatctgccagaccgacctggggcagatgcaagacccggtgtgctggactctgctcggctacgcctgcgcctattcctcggcgttcatgggccgggaaatcatcttcaaggaagtcagctgccgcggctgcggcggcgacaagtgccgggtcattggcaagccggccgaagagtgggacgacgttgccagcttcaaacagtatttcaagaacgaccccatcatcgaggaactctacgagttgcaatcgcaactggtgtcgctgcgtaccaacctcgacaaacaggaaggccagtactacggcatcggtcagaccccggcctaccagaccgtgcgcaatatgatggacaaggccgcacagggcaaagtctcggtgctgctgcttggcgagaccggggtcggcaaggaggtcatcgcgcgtagcgtgcacctgcgcagcaaacgcgccgccgagccctttgtcgcggtgaactgtgcggcgatcccgccggacctgatcgagtccgaattgttcggcgtggaaaaaggcgccttcaccggcgccacccagtcacgcatgggccgcttcgagcgggccgacaagggcaccatcttccttgacgaggtgatcgaactcagcccgcgcgctcaggccagtctgctgcgcgtgctgcaagaaggcgagctggagcgagttggcgacaaccgcacgcgcaagatcgacgtaagggttatcgcagccacccacgaggacctggccgaagcggtcaaggccgggcgttttcgcgccgacctgtactaccggctgaacgttttcccggtggcgatcccggcgttgcgcgaacgccgcgaggacattccactgctggttgagcacttccttcagcgcttccaccaggagtacggcaagagaaccctcggcctttcagacaaagccctggaggcctgcctgcattacagttggccgggcaatatccgtgagctggagaacgtcatcgagcgcggcatcatcctcaccgatccgaacgaaagcatcagcgtgcaggcgctgttcccacgggcgccggaagagccgcagaccgccagcgagcgggtgtcgtcggacggcgtgctgattcagccaggcaatggccagggcagttggatcagccagttgttgagcagcggcctgagcctcgacgagatcgaggaaagcctgatgcgcaaagccatgcaacaggccaaccaaaacgtctccggtgccgcgcgcttgctcggcctaagccgaccggcactggcctatcggctgaagaaaatcggcatcgaaggctaa

SEQ ID NO: 2 - DNA, 1083 bp, Artificial Sequence
  DmpR(delta2-204)
atgaacgaccccatcatcgaggaactctacgagttgcaatcgcaactggtgtcgctgcgtaccaacctcgacaaacaggaaggccagtactacggcatcggtcagaccccggcctaccagaccgtgcgcaatatgatggacaaggccgcacagggcaaagtctcggtgctgctgcttggcgagaccggggtcggcaaggaggtcatcgcgcgtagcgtgcacctgcgcagcaaacgcgccgccgagccctttgtcgcggtgaactgtgcggcgatcccgccggacctgatcgagtccgaattgttcggcgtggaaaaaggcgccttcaccggcgccacccagtcacgcatgggccgcttcgagcgggccgacaagggcaccatcttccttgacgaggtgatcgaactcagcccgcgcgctcaggccagtctgctgcgcgtgctgcaagaaggcgagctggagcgagttggcgacaaccgcacgcgcaagatcgacgtaagggttatcgcagccacccacgaggacctggccgaagcggtcaaggccgggcgttttcgcgccgacctgtactaccggctgaacgttttcccggtggcgatcccggcgttgcgcgaacgccgcgaggacattccactgctggttgagcacttccttcagcgcttccaccaggagtacggcaagagaaccctcggcctttcagacaaagccctggaggcctgcctgcattacagttggccgggcaatatccgtgagctggagaacgtcatcgagcgcggcatcatcctcaccgatccgaacgaaagcatcagcgtgcaggcgctgttcccacgggcgccggaagagccgcagaccgccagcgagcgggtgtcgtcggacggcgtgctgattcagccaggcaatggccagggcagttggatcagccagttgttgagcagcggcctgagcctcgacgagatcgaggaaagcctgatgcgcaaagccatgcaacaggccaaccaaaacgtctccggtgccgcgcgcttgctcggcctaagccgaccggcactggcctatcggctgaagaaaatcggcatcgaaggctaa

SEQ ID NO: 3 - DNA, 171 bp, Artificial Sequence
  P0 promoter
tgagcatttgctcaagcggccttgggcaattgatcaaatgcttaaaaagcctgcgcaagcgcggcttaatttcgctcgctccgatcattctaaaaattagaaacacattgaaaaacaataccttgaagtcggttttcagaccttggcacagctgttgcactttgtcctgcg

SEQ ID NO: 4 - DNA, 23 bp, Artificial Sequence
  Ribosome Binding Site
tttgtttaactttaagaaggaga

SEQ ID NO: 5 - DNA, 36 bp, Artificial Sequence
  RBS of mxaF(MDH)
tgcagggtcggcatcaatcattcttggaggagacac

SEQ ID NO: 6 - DNA, 36 bp, Artificial Sequence
  RBS of mmoX
catcattcatagaatgtgttacggaggaaacaagta

SEQ ID NO: 7 - DNA, 36 bp, Artificial Sequence
  RBS of mmoY
cgttcgatcaacctcaaaccaaaaaggaacatcgat

SEQ ID NO: 8 - DNA, 36 bp, Artificial Sequence
  RBS of mmoZ
tggacactttttcaacggcctgttaaggagaatgac

SEQ ID NO: 9 - DNA, 36 bp, Artificial Sequence
  RBS of pmoA1
gaaaataagaaaacgacaaatttggaggtaacttta

SEQ ID NO: 10 - DNA, 36 bp, Artificial Sequence
  RBS of pmoB1
gtgacccaacagcaagaactcgaaagaggagagatc

SEQ ID NO: 11 - DNA, 36 bp, Artificial Sequence
  RBS of pmoC1
ggcccctgtcaaccatcactttaggaggaacaaaca

SEQ ID NO: 12 - DNA, 36 bp, Artificial Sequence
  RBS of pmoC2
ccggtgttcacatcgatataacagttggaggtaaaa

SEQ ID NO: 13 - DNA, 36 bp, Artificial Sequence
  RBS of pmoC3
gtggcatcaatccaacaccaactcaggagaaatcag

SEQ ID NO: 14 - DNA, 702 bp, Artificial Sequence
  dTomato
atggtgagcaagggcgaggaggtcatcaaagagttcatgcgcttcaaggtgcgcatggagggctccatgaacggccacgagttcgagatcgagggcgagggcgagggccgcccctacgagggcacccagaccgccaagctgaaggtgaccaagggcggccccctgcccttcgcctgggacatcctgtccccccagttcatgtacggctccaaggcgtacgtgaagcaccccgccgacatccccgattacaagaagctgtccttccccgagggcttcaagtgggagcgcgtgatgaacttcgaggacggcggtctggtgaccgtgacccaggactcctccctgcaggacggcacgctgatctacaaggtgaagatgcgcggcaccaacttcccccccgacggccccgtaatgcagaagaagaccatgggctgggaggcctccaccgagcgcctgtacccccgcgacggcgtgctgaagggcgagatccaccaggccctgaagctgaaggacggcggccactacctggtggagttcaagaccatctacatggccaagaagcccgtgcaactgcccggctactactacgtggacaccaagctggacatcacctcccacaacgaggactacaccatcgtggaacagtacgagcgctccgagggccgccaccacctgttcctgtacggcatggacgagctgtacaag

SEQ ID NO: 15 - DNA, 5756 bp, Artificial Sequence
  pAWP89
gaccctttccgacgctcaccgggctggttgccctcgccgctgggctggcggccgtctatggccctgcaaacgcgccagaaacgccgtcgaagccgtgtgcgagacaccgcggccgccggcgttgtggatacctcgcggaaaacttggccctcactgacagatgaggggcggacgttgacacttgaggggccgactcacccggcgcggcgttgacagatgaggggcaggctcgatttcggccggcgacgtggagctggccagcctcgcaaatcggcgaaaacgcctgattttacgcgagtttcccacagatgatgtggacaagcctggggataagtgccctgcggtattgacacttgaggggcgcgactactgacagatgaggggcgcgatccttgacacttgaggggcagagtgctgacagatgaggggcgcacctattgacatttgaggggctgtccacaggcagaaaatccagcatttgcaagggtttccgcccgtttttcggccaccgctaacctgtcttttaacctgcttttaaaccaatatttataaaccttgtttttaaccagggctgcgccctgtgcgcgtgaccgcgcacgccgaaggggggtgcccccccttctcgaaccctcccggcccgctaacgcgggcctcccatccccccaggggctgcgcccctcggccgcgaacggcctcaccccaaaaatggcagccaagctgacccgctagggacgtgaagtcgattccttcgatggttagcaatcaaagactcagagtgctgtctggagcgtgaatctaacggtacgtatctcgattgctcggtcgctattcgcactctgcgaaagttcgtaccgctcattcactaggttgcgaatcatgaccaaaatcccttaacgtgagttttcgttccactgagcgtcagaccccgtagaaaagatcaaaggatcttcttgagatcctttttttctgcgcgtaatctgctgcttgcaaacaaaaaaaccaccgctaccagcggtggtttgtttgccggatcaagagctaccaactctttttccgaaggtaactggcttcagcagagcgcagataccaaatactgtccttctagtgtagccgtagttaggccaccacttcaagaactctgtagcaccgcctacatacctcgctctgctaatcctgttaccagtggctgctgccagtggcgataagtcgtgtcttaccgggttggactcaagacgatagttaccggataaggcgcagcggtcgggctgaacggggggttcgtgcacacagcccagcttggagcgaacgacctacaccgaactgagatacctacagcgtgagctatgagaaagcgccacgcttcccgaagggagaaaggcggacaggtatccggtaagcggcagggtcggaacaggagagcgcacgagggagcttccagggggaaacgcctggtatctttatagtcctgtcgggtttcgccacctctgacttgagcgtcgatttttgtgatgctcgtcaggggggcggagcctatggaaaaacgccagcaacgcggcctttttacggttcctggccttttgctggccttttgctcacatgttctttcctgcgttatcccctgattctgtggataaccgtattaccgcctttgagtgagctgctctgaaatgagctgttgacaattaatcatcggctcgtataatgtgtggaggtattcacacaggaaacagctatggtgagcaagggcgaggaggtcatcaaagagttcatgcgcttcaaggtgcgcatggagggctccatgaacggccacgagttcgagatcgagggcgagggcgagggccgcccctacgagggcacccagaccgccaagctgaaggtgaccaagggcggccccctgcccttcgcctgggacatcctgtccccccagttcatgtacggctccaaggcgtacgtgaagcaccccgccgacatccccgattacaagaagctgtccttccccgagggcttcaagtgggagcgcgtgatgaacttcgaggacggcggtctggtgaccgtgacccaggactcctccctgcaggacggcacgctgatctacaaggtgaagatgcgcggcaccaacttcccccccgacggccccgtaatgcagaagaagaccatgggctgggaggcctccaccgagcgcctgtacccccgcgacggcgtgctgaagggcgagatccaccaggccctgaagctgaaggacggcggccactacctggtggagttcaagaccatctacatggccaagaagcccgtgcaactgcccggctactactacgtggacaccaagctggacatcacctcccacaacgaggactacaccatcgtggaacagtacgagcgctccgagggccgccaccacctgttcctgtacggcatggacgagctgtacaagtagttgtcgggaagatgcgtgatctgatccttccactcagcaaaagttcgatttattcaacaaagccgccgtcccgtcaagtcagcgtaatgctctgccagtgttacaaccaattaaccaattctgattagaaaaactcatcgagcatcaaatgaaactgcaatttattcatatcaggattatcaataccatatttttgaaaaagccgtttctgtaatgaaggagaaaactcaccgaggcagttccataggatggcaagatcctggtatcggtctgcgattccgactcgtccaacatcaatacaacctattaatttcccctcgtcaaaaataaggttatcaagtgagaaatcaccatgagtgacgactgaatccggtgagaatggcaaaagcttatgcatttctttccagacttgttcaacaggccagccattacgctcgtcatcaaaatcactcgcatcaaccaaaccgttattcattcgtgattgcgcctgagcgagacgaaatacgcgatcgctgttaaaaggacaattacaaacaggaatcgaatgcaaccggcgcaggaacactgccagcgcatcaacaatattttcacctgaatcaggatattcttctaatacctggaatgctgttttcccggggatcgcagtggtgagtaaccatgcatcatcaggagtacggataaaatgcttgatggtcggaagaggcataaattccgtcagccagtttagtctgaccatctcatctgtaacatcattggcaacgctacctttgccatgtttcagaaacaactctggcgcatcgggcttcccatacaatcgatagattgtcgcacctgattgcccgacattatcgcgagcccatttatacccatataaatcagcatccatgttggaatttaatcgcggcctcgagcaagacgtttcccgttgaatatggctcataacaccccttgtattactgtttatgtaagcagacagttttattgttcatgatgatatatttttatcttgtgcaatgtaacatcagagattttgagacacaacgtggctttcgacttccggcaagctatacgcgccctagaattgtcaattttaatcctctgtttatcggcagttcgtagagcgcgccgtgcgtcccgagcgatactgagcgaagcaagtgcgtcgagcagtgcccgcttgttcctgaaatgccagtaaagcgctggctgctgaacccccagccggaactgaccccacaaggccctagcgtttgcaatgcaccaggtcatcattgacccaggcgtgttccaccaggccgctgcctcgcaactcttcgcaggcttcgccgacctgctcgcgccacttcttcacgcgggtggaatccgatccgcacatgaggcggaaggtttccagcttgagcgggtacggctcccggtgcgagctgaaatagtcgaacatccgtcgggccgtcggcgacagcttgcggtacttctcccatatgaatttcgtgtagtggtcgccagcaaacagcacgacgatttcctcgtcgatcaggacctggcaacgggacgttttcttgccacggtccaggacgcggaagcggtgcagcagcgacaccgattccaggtgcccaacgcggtcggacgtgaagcccatcgccgtcgcctgtaggcgcgacaggcattcctcggccttcgtgtaataccggccattgatcgaccagcccaggtcctggcaaagctcgtagaacgtgaaggtgatcggctcgccgataggggtgcgcttcgcgtactccaacacctgctgccacaccagttcgtcatcgtcggcccgcagctcgacgccggtgtaggtgatcttcacgtccttgttgacgtggaaaatgaccttgttttgcagcgcctcgcgcgggattttcttgttgcgcgtggtgaacagggcagagcgggccgtgtcgtttggcatcgctcgcatcgtgtccggccacggcgcaatatcgaacaaggaaagctgcatttccttgatctgctgcttcgtgtgtttcagcaacgcggcctgcttggcctcgctgacctgttttgccaggtcctcgccggcggtttttcgcttcttggtcgtcatagttcctcgcgtgtcgatggtcatcgacttcgccaaacctgccgcctcctgttcgagacgacgcgaacgctccacggcggccgatggcgcgggcagggcagggggagccagttgcacgctgtcgcgctcgatcttggccgtagcttgctggaccatcgagccgacggactggaaggtttcgcggggcgcacgcatgacggtgcggcttgcgatggtttcggcatcctcggcggaaaaccccgcgtcgatcagttcttgcctgtatgccttccggtcaaacgtccgattcattcaccctccttgcgggattgccccgactcacgccggggcaatgtgcccttattcctgatttgacccgcctggtgccttggtgtccagataatccaccttatcggcaatgaagtcggtcccgtagaccgtctggccgtccttctcgtacttggtattccgaatcttgccctgcacgaataccagctccgcgaagtcgctcttcttgatggagcgcatggggacgtgcttggcaatcacgcgcaccccccggccgttttagcggctaaaaaagtcatggctctgccctcgggcggaccacgcccatcatgaccttgccaagctcgtcctgcttctcttcgatcttcgccagcagggcgaggatcgtggcatcaccgaaccgcgccgtgcgcgggtcgtcggtgagccagagtttcagcaggccgcccaggcggcccaggtcgccattgatgcgggccagctcgcggacgtgctcatagtccacgacgcccgtgattttgtagccctggccgacggccagcaggtaggcctacaggctcatgccggccgccgccgccttttcctcaatcgctcttcgttcgtctggaaggcagtacaccttgataggtgggctgcccttcctggttggcttggtttcatcagccatccgcttgccctcatctgttacgccggcggtagccggccagcctcgcagagcaggattcccgttgagcaccgccaggtgcgaataagggacagtgaagaaggaacacccgctcgcgggtgggcctacttcacctatcctgcccggctgacgccgttggatacaccaaggaaagtctacacgaaccctttggcaaaatcctgtatatcgtgcgaaaaaggatggatataccgaaaaaatcgctataatgaccccgaagcagggttatgcagcggaaaagatccgtc

SEQ ID NO: 16 - DNA, 632 bp, Artificial Sequence
  oriV RP4/RK2
gacgctcaccgggctggttgccctcgccgctgggctggcggccgtctatggccctgcaaacgcgccagaaacgccgtcgaagccgtgtgcgagacaccgcggccgccggcgttgtggatacctcgcggaaaacttggccctcactgacagatgaggggcggacgttgacacttgaggggccgactcacccggcgcggcgttgacagatgaggggcaggctcgatttcggccggcgacgtggagctggccagcctcgcaaatcggcgaaaacgcctgattttacgcgagtttcccacagatgatgtggacaagcctggggataagtgccctgcggtattgacacttgaggggcgcgactactgacagatgaggggcgcgatccttgacacttgaggggcagagtgctgacagatgaggggcgcacctattgacatttgaggggctgtccacaggcagaaaatccagcatttgcaagggtttccgcccgtttttcggccaccgctaacctgtcttttaacctgcttttaaaccaatatttataaaccttgtttttaaccagggctgcgccctgtgcgcgtgaccgcgcacgccgaaggggggtgcccccccttctcgaaccctcccggcccgct

SEQ ID NO: 17 - DNA, 589 bp, Artificial Sequence
  oriV ColE1
ttgagatcctttttttctgcgcgtaatctgctgcttgcaaacaaaaaaaccaccgctaccagcggtggtttgtttgccggatcaagagctaccaactctttttccgaaggtaactggcttcagcagagcgcagataccaaatactgtccttctagtgtagccgtagttaggccaccacttcaagaactctgtagcaccgcctacatacctcgctctgctaatcctgttaccagtggctgctgccagtggcgataagtcgtgtcttaccgggttggactcaagacgatagttaccggataaggcgcagcggtcgggctgaacggggggttcgtgcacacagcccagcttggagcgaacgacctacaccgaactgagatacctacagcgtgagctatgagaaagcgccacgcttcccgaagggagaaaggcggacaggtatccggtaagcggcagggtcggaacaggagagcgcacgagggagcttccagggggaaacgcctggtatctttatagtcctgtcgggtttcgccacctctgacttgagcgtcgatttttgtgatgctcgtcaggggggcggagcctatggaaa

SEQ ID NO: 18 - DNA, 110 bp, Artificial Sequence
  oriT
ccggccagcctcgcagagcaggattcccgttgagcaccgccaggtgcgaataagggacagtgaagaaggaacacccgctcgcgggtgggcctacttcacctatcctgccc

SEQ ID NO: 19 - DNA, 1149 bp, Artificial Sequence
  trfA
ctagcgtttgcaatgcaccaggtcatcattgacccaggcgtgttccaccaggccgctgcctcgcaactcttcgcaggcttcgccgacctgctcgcgccacttcttcacgcgggtggaatccgatccgcacatgaggcggaaggtttccagcttgagcgggtacggctcccggtgcgagctgaaatagtcgaacatccgtcgggccgtcggcgacagcttgcggtacttctcccatatgaatttcgtgtagtggtcgccagcaaacagcacgacgatttcctcgtcgatcaggacctggcaacgggacgttttcttgccacggtccaggacgcggaagcggtgcagcagcgacaccgattccaggtgcccaacgcggtcggacgtgaagcccatcgccgtcgcctgtaggcgcgacaggcattcctcggccttcgtgtaataccggccattgatcgaccagcccaggtcctggcaaagctcgtagaacgtgaaggtgatcggctcgccgataggggtgcgcttcgcgtactccaacacctgctgccacaccagttcgtcatcgtcggcccgcagctcgacgccggtgtaggtgatcttcacgtccttgttgacgtggaaaatgaccttgttttgcagcgcctcgcgcgggattttcttgttgcgcgtggtgaacagggcagagcgggccgtgtcgtttggcatcgctcgcatcgtgtccggccacggcgcaatatcgaacaaggaaagctgcatttccttgatctgctgcttcgtgtgtttcagcaacgcggcctgcttggcctcgctgacctgttttgccaggtcctcgccggcggtttttcgcttcttggtcgtcatagttcctcgcgtgtcgatggtcatcgacttcgccaaacctgccgcctcctgttcgagacgacgcgaacgctccacggcggccgatggcgcgggcagggcagggggagccagttgcacgctgtcgcgctcgatcttggccgtagcttgctggaccatcgagccgacggactggaaggtttcgcggggcgcacgcatgacggtgcggcttgcgatggtttcggcatcctcggcggaaaaccccgcgtcgatcagttcttgcctgtatgccttccggtcaaacgtccgattcat

SEQ ID NO: 20 - DNA, 372 bp, Artificial Sequence
  traJ
tcatggctctgccctcgggcggaccacgcccatcatgaccttgccaagctcgtcctgcttctcttcgatcttcgccagcagggcgaggatcgtggcatcaccgaaccgcgccgtgcgcgggtcgtcggtgagccagagtttcagcaggccgcccaggcggcccaggtcgccattgatgcgggccagctcgcggacgtgctcatagtccacgacgcccgtgattttgtagccctggccgacggccagcaggtaggcctacaggctcatgccggccgccgccgccttttcctcaatcgctcttcgttcgtctggaaggcagtacaccttgataggtgggctgcccttcctggttggcttggtttcatcagccat

SEQ ID NO: 21 - DNA, 117 bp, Artificial Sequence
  traJ'
atggctgatgaaaccaagccaaccaggaagggcagcccacctatcaaggtgtactgccttccagacgaacgaagagcgattgaggaaaaggcggcggcggccggcatgagcctgtag

SEQ ID NO: 22 - DNA, 816 bp, Artificial Sequence
  KanR
ttagaaaaactcatcgagcatcaaatgaaactgcaatttattcatatcaggattatcaataccatatttttgaaaaagccgtttctgtaatgaaggagaaaactcaccgaggcagttccataggatggcaagatcctggtatcggtctgcgattccgactcgtccaacatcaatacaacctattaatttcccctcgtcaaaaataaggttatcaagtgagaaatcaccatgagtgacgactgaatccggtgagaatggcaaaagcttatgcatttctttccagacttgttcaacaggccagccattacgctcgtcatcaaaatcactcgcatcaaccaaaccgttattcattcgtgattgcgcctgagcgagacgaaatacgcgatcgctgttaaaaggacaattacaaacaggaatcgaatgcaaccggcgcaggaacactgccagcgcatcaacaatattttcacctgaatcaggatattcttctaatacctggaatgctgttttcccggggatcgcagtggtgagtaaccatgcatcatcaggagtacggataaaatgcttgatggtcggaagaggcataaattccgtcagccagtttagtctgaccatctcatctgtaacatcattggcaacgctacctttgccatgtttcagaaacaactctggcgcatcgggcttcccatacaatcgatagattgtcgcacctgattgcccgacattatcgcgagcccatttatacccatataaatcagcatccatgttggaatttaatcgcggcctcgagcaagacgtttcccgttgaatatggctcat

SEQ ID NO: 23 - DNA, 20 bp, Artificial Sequence
  pAW89(NotI)-F1
agccgtgtgcgagacaccgc

SEQ ID NO: 24 - DNA, 33 bp, Artificial Sequence
  pAW89(NotI)-R1
cccgacaatctagatagctgtttcctgtgtgaa

SEQ ID NO: 25 - DNA, 32 bp, Artificial Sequence
  pAW89(HindIII)-F2
cagctatctagattgtcgggaagatgcgtgat

SEQ ID NO: 26 - DNA, 20 bp, Artificial Sequence
  pAW89(HindIII)-R2
agtctggaaagaaatgcata

SEQ ID NO: 27 - DNA, 33 bp, Artificial Sequence
  pAWPS(NotI)-R1
ttcagagactagtttcgcaacctagtgaatgag

SEQ ID NO: 28 - DNA, 33 bp, Artificial Sequence
  pAWPS(XbaI)-F2
ttgcgaaactagtctctgaaatgagctgttgac

SEQ ID NO: 29 - DNA, 20 bp, Artificial Sequence
  pAWPS(XbaI)-R2
tcacgcatcttcccgacaat

SEQ ID NO: 30 - DNA, 40 bp, Artificial Sequence
  pTet-dTomato(SpeI)-F1
tcattcactaggttgcgaaatcagagattttgagacacaa

SEQ ID NO: 31 - DNA, 30 bp, Artificial Sequence
  pTet-dTomato(SpeI)-R1
tgctcaccatatgtatatctccttcttaaa

SEQ ID NO: 32 - DNA, 30 bp, Artificial Sequence
  pTet-dTomato(XbaI)-F2
agatatacatatggtgagcaagggcgagga

SEQ ID NO: 33 - DNA, 40 bp, Artificial Sequence
  pTet-dTomato(XbaI)-R2
tcacgcatcttcccgacaatctacttgtacagctcgtcca

SEQ ID NO: 34 - DNA, 45 bp, Artificial Sequence
  pAWPS-Ptrc(SpeI)-F
ctatcaacaggagtccaagactagtttgacaccatcgaatggtgc

SEQ ID NO: 35 - DNA, 45 bp, Artificial Sequence
  pAWPS-Ptrc(XbaI)-R
aaagttaaacaaaattatttctagagtgtgaaattgttatccgct

SEQ ID NO: 36 - DNA, 45 bp, Artificial Sequence
  pAWPS-Pm(SpeI)-F
ctatcaacaggagtccaagactagtacgttcgtaatcaagccact

SEQ ID NO: 37 - DNA, 45 bp, Artificial Sequence
  pAWPS-Pm(XbaI)-R
aaagttaaacaaaattatttctagacatggtcatgactccattat

SEQ ID NO: 38 - DNA, 45 bp, Artificial Sequence
  pAWPS-P0(SpeI)-F
ctatcaacaggagtccaagactagtagcggataacaatttcacac

SEQ ID NO: 39 - DNA, 45 bp, Artificial Sequence
  pAWPS-P0(XbaI)-R
aaagttaaacaaaattatttctagatctccaggttggcggattgc

SEQ ID NO: 40 - DNA, 9154 bp, Artificial Sequence
  pSEVA-Ptet-dCas9 plasmid
aggcatcaaataaaacgaaaggctcagtcgaaagactgggcctttcgttttatctgttgtttgtcggtgaacgctctcctgagtaggacaaatccgccgccctagacagctgggcgcgccgtagaaaagatcaaaggatcttcttgagatcctttttttctgcgggggatcaggaccgctgccggagcgcaacccactcactacagcagagccatgtagggccgccggcgttgtggatacctcgcggaaaacttggccctcactgacagatgaggggcggacgttgacacttgaggggccgactcacccggcgcggcgttgacagatgaggggcaggctcgatttcggccggcgacgtggagctggccagcctcgcaaatcggcgaaaacgcctgattttacgcgagtttcccacagatgatgtggacaagcctggggataagtgccctgcggtattgacacttgaggggcgcgactactgacagatgaggggcgcgatccttgacacttgaggggcagagtgctgacagatgaggggcgcacctattgacatttgaggggctgtccacaggcagaaaatccagcatttgcaagggtttccgcccgtttttcggccaccgctaacctgtcttttaacctgcttttaaaccaatatttataaaccttgtttttaaccagggctgcgccctgtgcgcgtgaccgcgcacgccgaaggggggtgcccccccttctcgaaccctcccggcccgctaacgcgggcctcccatccccccaggggctgcgcccctcggccgcgaacggcctcaccccaaaaatggcagccacgtagaaagccagtccgcagaaacggtgctgaccccggatgaatgtcagctactgggctatctggacaagggaaaacgcaagcgcaaagagaaagcaggtagcttgcagtgggcttacatggcgatagctagactgggcggttttatggacagcaagcgaaccggaattgccagctggggcgccctctggtaaggttgggaagccctgcaaagtaaactggatggctttcttgccgccaaggatctgatggcgcaggggatcaagatcgacggatcgatccggggaattaattccggggcaatcccgcaaggagggtgaatgaatcggacgtttgaccggaaggcatacaggcaagaactgatcgacgcggggttttccgccgaggatgccgaaaccatcgcaagccgcaccgtcatgcgtgcgccccgcgaaaccttccagtccgtcggctcgatagtccagcaagctacggccaagatcgagcgcgacagcgtgcaactggctccccctgccctgcccgcgccatcggccgccgtggagcgttcgcgtcgtctcgaacaggaggcggcaggtttggcgaagtcgatgaccatcgacacgcgaggaactatgacgaccaagaagcgaaaaaccgccggcgaggacctggcaaaacaggtcagcgaagccaagcaggccgcgttgctgaaacacacgaagcagcagatcaaggaaatgcagctttccttgttcgatattgcgccgtggccggacacgatgcgagcgatgccaaacgacacggcccgctctgccctgttcaccacgcgcaacaagaaaatcccgcgcgaggcgctgcaaaacaaggtcattttccacgtcaacaaggacgtgaagatcacctacaccggcgtcgagctgcgggccgacgatgacgaactggtgtggcagcaggtgttggagtacgcgaagcgcacccctatcggcgagccgatcaccttcacgttctacgagctttgccaggacctgggctggtcgatcaatggccggtattacacgaaggccgaggaatgcctgtcgcgcctacaggcgacggcgatgggcttcacgtccgaccgcgttgggcacctggaatcggtgtcgctgctgcaccgcttccgcgtcctggaccgtggcaagaaaacgtcccgttgccaggtcctgatcgacgaggaaatcgtcgtgctgtttgctggcgaccactacacgaaattcatatgggagaagtaccgcaagctgtcgccgacggcccgacggatgttcgactatttcagctcgcaccgggagccgtacccgctcaagctggaaaccttccgcctcatgtgcggatcggattccacccgcgtgaagaagtggcgcgagcaggtcggcgaagcctgcgaagagttgcgaggcagcggcctggtggaacacgcctgggtcaatgatgacctggtgcattgcaaacgctagggccttgtggggtcagttccggctgggggttcagcagccacctgcatcgcggccggcctacggccagcctcgcagagcaggattcccgttgagcaccgccaggtgcgaataagggacagtgaagaaggaacacccgctcgcgggtgggcctacttcacctatcctgcccggctgacgccgttggatacaccaaggaaagtctacacgaaccctttggcaaaatcctgtatatcgtgcgaaaaaggatggatataccgaaaaaatcgctataatgaccccgaagcagggttatgcagcggaaaaggacaacgcgcggaccgcggtccaattaattattagaaaaattcatccagcatcagatgaaattgcagtttgttcatatccggattatcaatgccatatttctgaaacagacgtttttgcaggctcgggctaaattcgcccaggcagttccacagaatggccagatcctgataacgatccgcaatgcccacacggcccacatcaatgcagccaatcagtttgccttcatcgaaaatcaggttatccaggctaaaatcgccgtgggtcaccacgctatccgggctaaacggcagcagtttatgcatttctttccacacctgttccaccggccagccgttacgttcatcatcaaaatcgctcgcatccaccaggccgttgttcatacggctctgcgcctgggccagacgaaacacacgatcgctgttaaacgggcagttgcacaccggaatgctatgcagacgacgcagaaacacggccagcgcatccacaatgttttcgccgctatccggatattcttccagcacctgaaacgcggttttgcccggaatcgcggtggtcagcagccacgcatcatccggggtgcgaataaaatgtttaatggtcggcagcggcataaattcggtcagccagttcagacgcaccatttcatcggtcacatcgttcgccacgctgcctttgccatgtttcagaaacagttccggcgcatccggtttgccatacagacgataaatggtcgcgccgctctgacccacgttatcacgcgcccatttatagccatacagatccgcatccatgttgctgttcagacgcggacggctacagctcgtttcacgctgaatatggctcataacaccccttgtattactgtttatgtaagcagacagttttattgttcatgatgatatatttttatcttgtgcaatgtaacatcagagattttgagacacaaatttaaatcgtaattattggggacccctggattctcaccaataaaaaacgcccggcggcaaccgagcgttctgaacaaatccagatggagttctgaggtcattactggatctatcaacaggagtccaagactagtcgccagggttttcccagtcattaagacccactttcacatttaagttgtttttctaatccgcatatgatcaattcaaggccgaataagaaggctggctctgcaccttggtgatcaaataattcgatagcttgtcgtaataatggcggcatactatcagtagtaggtgtttccctttcttctttagcgacttgatgctcttgatcttccaatacgcaacctaaagtaaaatgccccacagcgctgagtgcatataatgcattctctagtgaaaaaccttgttggcataaaaaggctaattgattttcgagagtttcatactgtttttctgtaggccgtgtacctaaatgtacttttgctccatcgcgatgacttagtaaagcacatctaaaacttttagcgttattacgtaaaaaatcttgccagctttccccttctaaagggcaaaagtgagtatggtgcctatctaacatctcaatggctaaggcgtcgagcaaagcccgcttattttttacatgccaatacaatgtaggctgctctacacctagcttctgggcgagtttacgggttgttaaaccttcgattccgacctcattaagcagctctaatgcgctgttaatcactttacttttatctaatctagacatcattaattcctaatttttgttgacactctatcgttgatagagttattttaccactccctatcagtgatagagaaaagtctagaaataattttgtttaactttaagaaggagatatacatatggataagaaatactcaataggcttagctatcggcacaaatagcgtcggatgggcggtgatcactgatgaatataaggttccgtctaaaaagttcaaggttctgggaaatacagaccgccacagtatcaaaaaaaatcttataggggctcttttatttgacagtggagagacagcggaagcgactcgtctcaaacggacagctcgtagaaggtatacacgtcggaagaatcgtatttgttatctacaggagattttttcaaatgagatggcgaaagtagatgatagtttctttcatcgacttgaagagtcttttttggtggaagaagacaagaagcatgaacgtcatcctatttttggaaatatagtagatgaagttgcttatcatgagaaatatccaactatctatcatctgcgaaaaaaattggtagattctactgataaagcggatttgcgcttaatctatttggccttagcgcatatgattaagtttcgtggtcattttttgattgagggagatttaaatcctgataatagtgatgtggacaaactatttatccagttggtacaaacctacaatcaattatttgaagaaaaccctattaacgcaagtggagtagatgctaaagcgattctttctgcacgattgagtaaatcaagacgattagaaaatctcattgctcagctccccggtgagaagaaaaatggcttatttgggaatctcattgctttgtcattgggtttgacccctaattttaaatcaaattttgatttggcagaagatgctaaattacagctttcaaaagatacttacgatgatgatttagataatttattggcgcaaattggagatcaatatgctgatttgtttttggcagctaagaatttatcagatgctattttactttcagatatcctaagagtaaatactgaaataactaaggctcccctatcagcttcaatgattaaacgctacgatgaacatcatcaagacttgactcttttaaaagctttagttcgacaacaacttccagaaaagtataaagaaatcttttttgatcaatcaaaaaacggatatgcaggttatattgatgggggagctagccaagaagaattttataaatttatcaaaccaattttagaaaaaatggatggtactgaggaattattggtgaaactaaatcgtgaagatttgctgcgcaagcaacggacctttgacaacggctctattccccatcaaattcacttgggtgagctgcatgctattttgagaagacaagaagacttttatccatttttaaaagacaatcgtgagaagattgaaaaaatcttgacttttcgaattccttattatgttggtccattggcgcgtggcaatagtcgttttgcatggatgactcggaagtctgaagaaacaattaccccatggaattttgaagaagttgtcgataaaggtgcttcagctcaatcatttattgaacgcatgacaaactttgataaaaatcttccaaatgaaaaagtactaccaaaacatagtttgctttatgagtattttacggtttataacgaattgacaaaggtcaaatatgttactgaaggaatgcgaaaaccagcatttctttcaggtgaacagaagaaagccattgttgatttactcttcaaaacaaatcgaaaagtaaccgttaagcaattaaaagaagattatttcaaaaaaatagaatgttttgatagtgttgaaatttcaggagttgaagatagatttaatgcttcattaggtacctaccatgatttgctaaaaattattaaagataaagattttttggataatgaagaaaatgaagatatcttagaggatattgttttaacattgaccttatttgaagatagggagatgattgaggaaagacttaaaacatatgctcacctctttgatgataaggtgatgaaacagcttaaacgtcgccgttatactggttggggacgtttgtctcgaaaattgattaatggtattagggataagcaatctggcaaaacaatattagattttttgaaatcagatggttttgccaatcgcaattttatgcagctgatccatgatgatagtttgacatttaaagaagacattcaaaaagcacaagtgtctggacaaggcgatagtttacatgaacatattgcaaatttagctggtagccctgctattaaaaaaggtattttacagactgtaaaagttgttgatgaattggtcaaagtaatggggcggcataagccagaaaatatcgttattgaaatggcacgtgaaaatcagacaactcaaaagggccagaaaaattcgcgagagcgtatgaaacgaatcgaagaaggtatcaaagaattaggaagtcagattcttaaagagcatcctgttgaaaatactcaattgcaaaatgaaaagctctatctctattatctccaaaatggaagagacatgtatgtggaccaagaattagatattaatcgtttaagtgattatgatgtcgatgccattgttccacaaagtttccttaaagacgattcaatagacaataaggtcttaacgcgttctgataaaaatcgtggtaaatcggataacgttccaagtgaagaagtagtcaaaaagatgaaaaactattggagacaacttctaaacgccaagttaatcactcaacgtaagtttgataatttaacgaaagctgaacgtggaggtttgagtgaacttgataaagctggttttatcaaacgccaattggttgaaactcgccaaatcactaagcatgtggcacaaattttggatagtcgcatgaatactaaatacgatgaaaatgataaacttattcgagaggttaaagtgattaccttaaaatctaaattagtttctgacttccgaaaagatttccaattctataaagtacgtgagattaacaattaccatcatgcccatgatgcgtatctaaatgccgtcgttggaactgctttgattaagaaatatccaaaacttgaatcggagtttgtctatggtgattataaagtttatgatgttcgtaaaatgattgctaagtctgagcaagaaataggcaaagcaaccgcaaaatatttcttttactctaatatcatgaacttcttcaaaacagaaattacacttgcaaatggagagattcgcaaacgccctctaatcgaaactaatggggaaactggagaaattgtctgggataaagggcgagattttgccacagtgcgcaaagtattgtccatgccccaagtcaatattgtcaagaaaacagaagtacagacaggcggattctccaaggagtcaattttaccaaaaagaaattcggacaagcttattgctcgtaaaaaagactgggatccaaaaaaatatggtggttttgatagtccaacggtagcttattcagtcctagtggttgctaaggtggaaaaagggaaatcgaagaagttaaaatccgttaaagagttactagggatcacaattatggaaagaagttcctttgaaaaaaatccgattgactttttagaagctaaaggatataaggaagttaaaaaagacttaatcattaaactacctaaatatagtctttttgagttagaaaacggtcgtaaacggatgctggctagtgccggagaattacaaaaaggaaatgagctggctctgccaagcaaatatgtgaattttttatatttagctagtcattatgaaaagttgaagggtagtccagaagataacgaacaaaaacaattgtttgtggagcagcataagcattatttagatgagattattgagcaaatcagtgaattttctaagcgtgttattttagcagatgccaatttagataaagttcttagtgcatataacaaacatagagacaaaccaatacgtgaacaagcagaaaatattattcatttatttacgttgacgaatcttggagctcccgctgcttttaaatattttgatacaacaattgatcgtaaacgatatacgtctacaaaagaagttttagatgccactcttatccatcaatccatcactggtctttatgaaacacgcattgatttgagtcagctaggaggtgactaactcgagtaaggatctccaggcatcaaataaaacgaaaggctcagtcgaaagactgggcctttcgttttatctgttgtttgtcggtgaacgctctctactagagtcacactggctcaccttcgggtgggcctttctgcgtttatacctagggatatattccgcttcctcggcgaccggggcggccgcctcgaggaagcttgggcccgaacaaaaactcatctcagaagaggatctgaatagcgccgtcgaccatcatcatcatcatcattgagtttaaacggtctccagcttggctgttttggcggatgagagaagattttcagcctgatacagattaaatcagaacgcagaagcggtctgataaaacagaatttgcctggcggcagtagcgcggtggtcccacctgaccccatgccgaactcagaagtgaaacgccgtagcgccgatggtagtgtggggtctccccatgcgagagtagggaactgccaggcatcaaataaaacgaaaggctcagtcgaaagactgggcctttcgttttatctgttgtttgtcggtgaactggcgcccaatacgcaaaccgtgaaattgttatccgctttaattaa

SEQ ID NO: 41 - DNA, 5818 bp, Artificial Sequence
  pAWP89S-Ptet-dTomato
gaccctttccgacgctcaccgggctggttgccctcgccgctgggctggcggccgtctatggccctgcaaacgcgccagaaacgccgtcgaagccgtgtgcgagacaccgcggccgccggcgttgtggatacctcgcggaaaacttggccctcactgacagatgaggggcggacgttgacacttgaggggccgactcacccggcgcggcgttgacagatgaggggcaggctcgatttcggccggcgacgtggagctggccagcctcgcaaatcggcgaaaacgcctgattttacgcgagtttcccacagatgatgtggacaagcctggggataagtgccctgcggtattgacacttgaggggcgcgactactgacagatgaggggcgcgatccttgacacttgaggggcagagtgctgacagatgaggggcgcacctattgacatttgaggggctgtccacaggcagaaaatccagcatttgcaagggtttccgcccgtttttcggccaccgctaacctgtcttttaacctgcttttaaaccaatatttataaaccttgtttttaaccagggctgcgccctgtgcgcgtgaccgcgcacgccgaaggggggtgcccccccttctcgaaccctcccggcccgctaacgcgggcctcccatccccccaggggctgcgcccctcggccgcgaacggcctcaccccaaaaatggcagccaagctgacccgctagggacgtgaagtcgattccttcgatggttagcaatcaaagactcagagtgctgtctggagcgtgaatctaacggtacgtatctcgattgctcggtcgctattcgcactctgcgaaagttcgtaccgctcattcactaggttgcgaaatcagagattttgagacacaaatttaaatcgtaattattggggacccctggattctcaccaataaaaaacgcccggcggcaaccgagcgttctgaacaaatccagatggagttctgaggtcattactggatctatcaacaggagtccaagactagtcgccagggttttcccagtcattaagacccactttcacatttaagttgtttttctaatccgcatatgatcaattcaaggccgaataagaaggctggctctgcaccttggtgatcaaataattcgatagcttgtcgtaataatggcggcatactatcagtagtaggtgtttccctttcttctttagcgacttgatgctcttgatcttccaatacgcaacctaaagtaaaatgccccacagcgctgagtgcatataatgcattctctagtgaaaaaccttgttggcataaaaaggctaattgattttcgagagtttcatactgtttttctgtaggccgtgtacctaaatgtacttttgctccatcgcgatgacttagtaaagcacatctaaaacttttagcgttattacgtaaaaaatcttgccagctttccccttctaaagggcaaaagtgagtatggtgcctatctaacatctcaatggctaaggcgtcgagcaaagcccgcttattttttacatgccaatacaatgtaggctgctctacacctagcttctgggcgagtttacgggttgttaaaccttcgattccgacctcattaagcagctctaatgcgctgttaatcactttacttttatctaatctagacatcattaattcctaatttttgttgacactctatcgttgatagagttattttaccactccctatcagtgatagagaaaagtctagaaataattttgtttaactttaagaaggagatatacatatggtgagcaagggcgaggaggtcatcaaagagttcatgcgcttcaaggtgcgcatggagggctccatgaacggccacgagttcgagatcgagggcgagggcgagggccgcccctacgagggcacccagaccgccaagctgaaggtgaccaagggcggccccctgcccttcgcctgggacatcctgtccccccagttcatgtacggctccaaggcgtacgtgaagcaccccgccgacatccccgattacaagaagctgtccttccccgagggcttcaagtgggagcgcgtgatgaacttcgaggacggcggtctggtgaccgtgacccaggactcctccctgcaggacggcacgctgatctacaaggtgaagatgcgcggcaccaacttcccccccgacggccccgtaatgcagaagaagaccatgggctgggaggcctccaccgagcgcctgtacccccgcgacggcgtgctgaagggcgagatccaccaggccctgaagctgaaggacggcggccactacctggtggagttcaagaccatctacatggccaagaagcccgtgcaactgcccggctactactacgtggacaccaagctggacatcacctcccacaacgaggactacaccatcgtggaacagtacgagcgctccgagggccgccaccacctgttcctgtacggcatggacgagctgtacaagtagattgtcgggaagatgcgtgatctgatccttccactcagcaaaagttcgatttattcaacaaagccgccgtcccgtcaagtcagcgtaatgctctgccagtgttacaaccaattaaccaattctgattagaaaaactcatcgagcatcaaatgaaactgcaatttattcatatcaggattatcaataccatatttttgaaaaagccgtttctgtaatgaaggagaaaactcaccgaggcagttccataggatggcaagatcctggtatcggtctgcgattccgactcgtccaacatcaatacaacctattaatttcccctcgtcaaaaataaggttatcaagtgagaaatcaccatgagtgacgactgaatccggtgagaatggcaaaagcttatgcatttctttccagacttgttcaacaggccagccattacgctcgtcatcaaaatcactcgcatcaaccaaaccgttattcattcgtgattgcgcctgagcgagacgaaatacgcgatcgctgttaaaaggacaattacaaacaggaatcgaatgcaaccggcgcaggaacactgccagcgcatcaacaatattttcacctgaatcaggatattcttctaatacctggaatgctgttttcccggggatcgcagtggtgagtaaccatgcatcatcaggagtacggataaaatgcttgatggtcggaagaggcataaattccgtcagccagtttagtctgaccatctcatctgtaacatcattggcaacgctacctttgccatgtttcagaaacaactctggcgcatcgggcttcccatacaatcgatagattgtcgcacctgattgcccgacattatcgcgagcccatttatacccatataaatcagcatccatgttggaatttaatcgcggcctcgagcaagacgtttcccgttgaatatggctcataacaccccttgtattactgtttatgtaagcagacagttttattgttcatgatgatatatttttatcttgtgcaatgtaacatcagagattttgagacacaacgtggctttcgacttccggcaagctatacgcgccctagaattgtcaattttaatcctctgtttatcggcagttcgtagagcgcgccgtgcgtcccgagcgatactgagcgaagcaagtgcgtcgagcagtgcccgcttgttcctgaaatgccagtaaagcgctggctgctgaacccccagccggaactgaccccacaaggccctagcgtttgcaatgcaccaggtcatcattgacccaggcgtgttccaccaggccgctgcctcgcaactcttcgcaggcttcgccgacctgctcgcgccacttcttcacgcgggtggaatccgatccgcacatgaggcggaaggtttccagcttgagcgggtacggctcccggtgcgagctgaaatagtcgaacatccgtcgggccgtcggcgacagcttgcggtacttctcccatatgaatttcgtgtagtggtcgccagcaaacagcacgacgatttcctcgtcgatcaggacctggcaacgggacgttttcttgccacggtccaggacgcggaagcggtgcagcagcgacaccgattccaggtgcccaacgcggtcggacgtgaagcccatcgccgtcgcctgtaggcgcgacaggcattcctcggccttcgtgtaataccggccattgatcgaccagcccaggtcctggcaaagctcgtagaacgtgaaggtgatcggctcgccgataggggtgcgcttcgcgtactccaacacctgctgccacaccagttcgtcatcgtcggcccgcagctcgacgccggtgtaggtgatcttcacgtccttgttgacgtggaaaatgaccttgttttgcagcgcctcgcgcgggattttcttgttgcgcgtggtgaacagggcagagcgggccgtgtcgtttggcatcgctcgcatcgtgtccggccacggcgcaatatcgaacaaggaaagctgcatttccttgatctgctgcttcgtgtgtttcagcaacgcggcctgcttggcctcgctgacctgttttgccaggtcctcgccggcggtttttcgcttcttggtcgtcatagttcctcgcgtgtcgatggtcatcgacttcgccaaacctgccgcctcctgttcgagacgacgcgaacgctccacggcggccgatggcgcgggcagggcagggggagccagttgcacgctgtcgcgctcgatcttggccgtagcttgctggaccatcgagccgacggactggaaggtttcgcggggcgcacgcatgacggtgcggcttgcgatggtttcggcatcctcggcggaaaaccccgcgtcgatcagttcttgcctgtatgccttccggtcaaacgtccgattcattcaccctccttgcgggattgccccgactcacgccggggcaatgtgcccttattcctgatttgacccgcctggtgccttggtgtccagataatccaccttatcggcaatgaagtcggtcccgtagaccgtctggccgtccttctcgtacttggtattccgaatcttgccctgcacgaataccagctccgcgaagtcgctcttcttgatggagcgcatggggacgtgcttggcaatcacgcgcaccccccggccgttttagcggctaaaaaagtcatggctctgccctcgggcggaccacgcccatcatgaccttgccaagctcgtcctgcttctcttcgatcttcgccagcagggcgaggatcgtggcatcaccgaaccgcgccgtgcgcgggtcgtcggtgagccagagtttcagcaggccgcccaggcggcccaggtcgccattgatgcgggccagctcgcggacgtgctcatagtccacgacgcccgtgattttgtagccctggccgacggccagcaggtaggcctacaggctcatgccggccgccgccgccttttcctcaatcgctcttcgttcgtctggaaggcagtacaccttgataggtgggctgcccttcctggttggcttggtttcatcagccatccgcttgccctcatctgttacgccggcggtagccggccagcctcgcagagcaggattcccgttgagcaccgccaggtgcgaataagggacagtgaagaaggaacacccgctcgcgggtgggcctacttcacctatcctgcccggctgacgccgttggatacaccaaggaaagtctacacgaaccctttggcaaaatcctgtatatcgtgcgaaaaaggatggatataccgaaaaaatcgctataatgaccccgaagcagggttatgcagcggaaaagatccgtc

SEQ ID NO: 42 - DNA, 6553 bp, Artificial Sequence
  pAWP89S-Ptrc-dTomato
gaccctttccgacgctcaccgggctggttgccctcgccgctgggctggcggccgtctatggccctgcaaacgcgccagaaacgccgtcgaagccgtgtgcgagacaccgcggccgccggcgttgtggatacctcgcggaaaacttggccctcactgacagatgaggggcggacgttgacacttgaggggccgactcacccggcgcggcgttgacagatgaggggcaggctcgatttcggccggcgacgtggagctggccagcctcgcaaatcggcgaaaacgcctgattttacgcgagtttcccacagatgatgtggacaagcctggggataagtgccctgcggtattgacacttgaggggcgcgactactgacagatgaggggcgcgatccttgacacttgaggggcagagtgctgacagatgaggggcgcacctattgacatttgaggggctgtccacaggcagaaaatccagcatttgcaagggtttccgcccgtttttcggccaccgctaacctgtcttttaacctgcttttaaaccaatatttataaaccttgtttttaaccagggctgcgccctgtgcgcgtgaccgcgcacgccgaaggggggtgcccccccttctcgaaccctcccggcccgctaacgcgggcctcccatccccccaggggctgcgcccctcggccgcgaacggcctcaccccaaaaatggcagccaagctgacccgctagggacgtgaagtcgattccttcgatggttagcaatcaaagactcagagtgctgtctggagcgtgaatctaacggtacgtatctcgattgctcggtcgctattcgcactctgcgaaagttcgtaccgctcattcactaggttgcgaaatcagagattttgagacacaaatttaaatcgtaattattggggacccctggattctcaccaataaaaaacgcccggcggcaaccgagcgttctgaacaaatccagatggagttctgaggtcattactggatctatcaacaggagtccaagactagtttgacaccatcgaatggtgcaaaacctttcgcggtatggcatgatagcgcccggaagagagtcaattcagggtggtgaatgtgaaaccagtaacgttatacgatgtcgcagagtatgccggtgtctcttatcagaccgtttcccgcgtggtgaaccaggccagccacgtttctgcgaaaacgcgggaaaaagtggaagcggcgatggcggagctgaattacattcccaaccgcgtggcacaacaactggcgggcaaacagtcgttgctgattggcgttgccacctccagtctggccctgcacgcgccgtcgcaaattgtcgcggcgattaaatctcgcgccgatcaactgggtgccagcgtggtggtgtcgatggtagaacgaagcggcgtcgaagcctgtaaagcggcggtgcacaatcttctcgcgcaacgcgtcagtgggctgatcattaactatccgctggatgaccaggatgccattgctgtggaagctgcctgcactaatgttccggcgttatttcttgatgtctctgaccagacacccatcaacagtattattttctcccatgaagacggtacgcgactgggcgtggagcatctggtcgcattgggtcaccagcaaatcgcgctgttagcgggcccattaagttctgtctcggcgcgtctgcgtctggctggctggcataaatatctcactcgcaatcaaattcagccgatagcggaacgggaaggcgactggagtgccatgtccggttttcaacaaaccatgcaaatgctgaatgagggcatcgttcccactgcgatgctggttgccaacgatcagatggcgctgggcgcaatgcgcgccattaccgagtccgggctgcgcgttggtgcggatatctcggtagtgggatacgacgataccgaagacagctcatgttatatcccgccgttaaccaccatcaaacaggattttcgcctgctggggcaaaccagcgtggaccgcttgctgcaactctctcagggccaggcggtgaagggcaatcagctgttgcccgtctcactggtgaaaagaaaaaccaccctggcgcccaatacgcaaaccgcctctccccgcgcgttggccgattcattaatgcagctggcacgacaggtttcccgactggaaagcgggcagtgagcgcaacgcaattaatgtaagttagcgcgaattgatctggtttgacagcttatcatcgactgcacggtgcaccaatgcttctggcgtcaggcagccatcggaagctgtggtatggctgtgcaggtcgtaaatcactgcataattcgtgtcgctcaaggcgcactcccgttctggataatgttttttgcgccgacatcataacggttctggcaaatattctgaaatgagctgttgacaattaatcatccggctcgtataatgtgtggaattgtgagcggataacaatttcacactctagaaataattttgtttaactttaagaaggagatatacatatggtgagcaagggcgaggaggtcatcaaagagttcatgcgcttcaaggtgcgcatggagggctccatgaacggccacgagttcgagatcgagggcgagggcgagggccgcccctacgagggcacccagaccgccaagctgaaggtgaccaagggcggccccctgcccttcgcctgggacatcctgtccccccagttcatgtacggctccaaggcgtacgtgaagcaccccgccgacatccccgattacaagaagctgtccttccccgagggcttcaagtgggagcgcgtgatgaacttcgaggacggcggtctggtgaccgtgacccaggactcctccctgcaggacggcacgctgatctacaaggtgaagatgcgcggcaccaacttcccccccgacggccccgtaatgcagaagaagaccatgggctgggaggcctccaccgagcgcctgtacccccgcgacggcgtgctgaagggcgagatccaccaggccctgaagctgaaggacggcggccactacctggtggagttcaagaccatctacatggccaagaagcccgtgcaactgcccggctactactacgtggacaccaagctggacatcacctcccacaacgaggactacaccatcgtggaacagtacgagcgctccgagggccgccaccacctgttcctgtacggcatggacgagctgtacaagtagattgtcgggaagatgcgtgatctgatccttccactcagcaaaagttcgatttattcaacaaagccgccgtcccgtcaagtcagcgtaatgctctgccagtgttacaaccaattaaccaattctgattagaaaaactcatcgagcatcaaatgaaactgcaatttattcatatcaggattatcaataccatatttttgaaaaagccgtttctgtaatgaaggagaaaactcaccgaggcagttccataggatggcaagatcctggtatcggtctgcgattccgactcgtccaacatcaatacaacctattaatttcccctcgtcaaaaataaggttatcaagtgagaaatcaccatgagtgacgactgaatccggtgagaatggcaaaagcttatgcatttctttccagacttgttcaacaggccagccattacgctcgtcatcaaaatcactcgcatcaaccaaaccgttattcattcgtgattgcgcctgagcgagacgaaatacgcgatcgctgttaaaaggacaattacaaacaggaatcgaatgcaaccggcgcaggaacactgccagcgcatcaacaatattttcacctgaatcaggatattcttctaatacctggaatgctgttttcccggggatcgcagtggtgagtaaccatgcatcatcaggagtacggataaaatgcttgatggtcggaagaggcataaattccgtcagccagtttagtctgaccatctcatctgtaacatcattggcaacgctacctttgccatgtttcagaaacaactctggcgcatcgggcttcccatacaatcgatagattgtcgcacctgattgcccgacattatcgcgagcccatttatacccatataaatcagcatccatgttggaatttaatcgcggcctcgagcaagacgtttcccgttgaatatggctcataacaccccttgtattactgtttatgtaagcagacagttttattgttcatgatgatatatttttatcttgtgcaatgtaacatcagagattttgagacacaacgtggctttcgacttccggcaagctatacgcgccctagaattgtcaattttaatcctctgtttatcggcagttcgtagagcgcgccgtgcgtcccgagcgatactgagcgaagcaagtgcgtcgagcagtgcccgcttgttcctgaaatgccagtaaagcgctggctgctgaacccccagccggaactgaccccacaaggccctagcgtttgcaatgcaccaggtcatcattgacccaggcgtgttccaccaggccgctgcctcgcaactcttcgcaggcttcgccgacctgctcgcgccacttcttcacgcgggtggaatccgatccgcacatgaggcggaaggtttccagcttgagcgggtacggctcccggtgcgagctgaaatagtcgaacatccgtcgggccgtcggcgacagcttgcggtacttctcccatatgaatttcgtgtagtggtcgccagcaaacagcacgacgatttcctcgtcgatcaggacctggcaacgggacgttttcttgccacggtccaggacgcggaagcggtgcagcagcgacaccgattccaggtgcccaacgcggtcggacgtgaagcccatcgccgtcgcctgtaggcgcgacaggcattcctcggccttcgtgtaataccggccattgatcgaccagcccaggtcctggcaaagctcgtagaacgtgaaggtgatcggctcgccgataggggtgcgcttcgcgtactccaacacctgctgccacaccagttcgtcatcgtcggcccgcagctcgacgccggtgtaggtgatcttcacgtccttgttgacgtggaaaatgaccttgttttgcagcgcctcgcgcgggattttcttgttgcgcgtggtgaacagggcagagcgggccgtgtcgtttggcatcgctcgcatcgtgtccggccacggcgcaatatcgaacaaggaaagctgcatttccttgatctgctgcttcgtgtgtttcagcaacgcggcctgcttggcctcgctgacctgttttgccaggtcctcgccggcggtttttcgcttcttggtcgtcatagttcctcgcgtgtcgatggtcatcgacttcgccaaacctgccgcctcctgttcgagacgacgcgaacgctccacggcggccgatggcgcgggcagggcagggggagccagttgcacgctgtcgcgctcgatcttggccgtagcttgctggaccatcgagccgacggactggaaggtttcgcggggcgcacgcatgacggtgcggcttgcgatggtttcggcatcctcggcggaaaaccccgcgtcgatcagttcttgcctgtatgccttccggtcaaacgtccgattcattcaccctccttgcgggattgccccgactcacgccggggcaatgtgcccttattcctgatttgacccgcctggtgccttggtgtccagataatccaccttatcggcaatgaagtcggtcccgtagaccgtctggccgtccttctcgtacttggtattccgaatcttgccctgcacgaataccagctccgcgaagtcgctcttcttgatggagcgcatggggacgtgcttggcaatcacgcgcaccccccggccgttttagcggctaaaaaagtcatggctctgccctcgggcggaccacgcccatcatgaccttgccaagctcgtcctgcttctcttcgatcttcgccagcagggcgaggatcgtggcatcaccgaaccgcgccgtgcgcgggtcgtcggtgagccagagtttcagcaggccgcccaggcggcccaggtcgccattgatgcgggccagctcgcggacgtgctcatagtccacgacgcccgtgattttgtagccctggccgacggccagcaggtaggcctacaggctcatgccggccgccgccgccttttcctcaatcgctcttcgttcgtctggaaggcagtacaccttgataggtgggctgcccttcctggttggcttggtttcatcagccatccgcttgccctcatctgttacgccggcggtagccggccagcctcgcagagcaggattcccgttgagcaccgccaggtgcgaataagggacagtgaagaaggaacacccgctcgcgggtgggcctacttcacctatcctgcccggctgacgccgttggatacaccaaggaaagtctacacgaaccctttggcaaaatcctgtatatcgtgcgaaaaaggatggatataccgaaaaaatcgctataatgaccccgaagcagggttatgcagcggaaaagatccgtc

SEQ ID NO: 43 - DNA, 7084 bp, Artificial Sequence
  pAWP89S-Pm-dTomato
gaccctttccgacgctcaccgggctggttgccctcgccgctgggctggcggccgtctatggccctgcaaacgcgccagaaacgccgtcgaagccgtgtgcgagacaccgcggccgccggcgttgtggatacctcgcggaaaacttggccctcactgacagatgaggggcggacgttgacacttgaggggccgactcacccggcgcggcgttgacagatgaggggcaggctcgatttcggccggcgacgtggagctggccagcctcgcaaatcggcgaaaacgcctgattttacgcgagtttcccacagatgatgtggacaagcctggggataagtgccctgcggtattgacacttgaggggcgcgactactgacagatgaggggcgcgatccttgacacttgaggggcagagtgctgacagatgaggggcgcacctattgacatttgaggggctgtccacaggcagaaaatccagcatttgcaagggtttccgcccgtttttcggccaccgctaacctgtcttttaacctgcttttaaaccaatatttataaaccttgtttttaaccagggctgcgccctgtgcgcgtgaccgcgcacgccgaaggggggtgcccccccttctcgaaccctcccggcccgctaacgcgggcctcccatccccccaggggctgcgcccctcggccgcgaacggcctcaccccaaaaatggcagccaagctgacccgctagggacgtgaagtcgattccttcgatggttagcaatcaaagactcagagtgctgtctggagcgtgaatctaacggtacgtatctcgattgctcggtcgctattcgcactctgcgaaagttcgtaccgctcattcactaggttgcgaaatcagagattttgagacacaaatttaaatcgtaattattggggacccctggattctcaccaataaaaaacgcccggcggcaaccgagcgttctgaacaaatccagatggagttctgaggtcattactggatctatcaacaggagtccaagactagtacgttcgtaatcaagccacttcctttttgcattgacgcagggtgtcggaaggcaactcgccgaacgcgctcctatagttttcagcgaagcgtcccaaatgtaagaagccgtagtctagggctatctcagttatactacgcacattggcactgggatcgttcaagcaggcgcggatgctttcgagcttgcggttgcggatgtagttcttcggcgtggtgccggcgtgcttctcgaacaaattgtagagcgagcgtggactcatcatcgccagctccgctaaccgctcaaggctgatattccgtttgagattctcctcaatgaattgaacgactcgctcgaaagacgggttacctttgctgaaaatttcacggctgacattgctgcccagcatttcgagcagcttggaagcgatgatccccgcatagtgctcttggacccgaggcatcgactttgtatgttccgcttcgtcacaaactaacccgagtagattgataaagccatcgagttgctggagattgtgtcgcgcggcgaaacggataccctccctcggcttgtgccaattgttgtcactgcacgcccgatcaaggaccactgagggcaatttaacgataaatttctcgcaatcttctgaataggtcaggtcggcttggtcatccggattgagcagcaatagttcgcccggcgcaaaatagtgctcctggccatggccacgccacaggcaatggcctttgagtattatttgcagatgataacaggtctctaatccaggcgagattaccctcacgctaccgccgtagctgattcgacacagatcgaggcatccgaagattctgtggtgcagcctgcctgccgggcgcccgcccttgggcaggcgaatagagtgcgtaccgacatactggttaacataatcggagactgcatagggctcggcgtggacgaagatctgacttttctcgttcaataagcaaaaatccatagttcacggttctcttattttaatgtgggctgcttggtgtgatgtagaaaggcgccaagtcgatgaaaatgcatctcgacgtgatgcgtatacgggttacccccattgccacgttgcgccatcctttttgcaatcagtgaccacttttccaagcaaaaataacgccaagcagaacgaagacgttctttttaagaagcgagaacaccagaagttcgtgctgtcggggcatggggcgacgaattggcggataaaggggatctgctggatattacggcctttttaaagaccgtaaagaaaaataagcacaagttttatccggcctttattcacattcttgcccgcctgatgaatgctcatccgtaattacgtatggcaatgaaagacggtgagctggtgatatgggatagtgttcacccttgttacaccgttttccatgagcaaactgaaacgttttcatcgctctggagtgaataccacgacgatttccggcagtttctacacatatattcgcaagatgtggcgtgttacggtgaaaacctggcctatttccctaaagggtttattgagaatatgtttttcgtctcagccaatccctgggtgagtttcaccagttttgatttaaacgtggccaatatggacaacttcttcgcccccgttttcaccatgcatgggaattagcttgatctgaccaacgaccggtagcggagctatccaacggcggtataccaggaaaacacacagcaggtacatcagaacagtaccatgactgaagaacaaatagttttttcctgatccataaagcagaacggcctgctccatgacaaatctggctccccaactaatgccccatgcagccagcataaccagcataaagtgcagtgtccggtttgatagggataagtccagccttgcaagaagcggatacaggagtgcaaaaaatggctatctctagtaaggcctaccccttaggctttatgcaacagaaacaataataatggagtcatgaccatgtctagaaataattttgtttaactttaagaaggagatatacatatggtgagcaagggcgaggaggtcatcaaagagttcatgcgcttcaaggtgcgcatggagggctccatgaacggccacgagttcgagatcgagggcgagggcgagggccgcccctacgagggcacccagaccgccaagctgaaggtgaccaagggcggccccctgcccttcgcctgggacatcctgtccccccagttcatgtacggctccaaggcgtacgtgaagcaccccgccgacatccccgattacaagaagctgtccttccccgagggcttcaagtgggagcgcgtgatgaacttcgaggacggcggtctggtgaccgtgacccaggactcctccctgcaggacggcacgctgatctacaaggtgaagatgcgcggcaccaacttcccccccgacggccccgtaatgcagaagaagaccatgggctgggaggcctccaccgagcgcctgtacccccgcgacggcgtgctgaagggcgagatccaccaggccctgaagctgaaggacggcggccactacctggtggagttcaagaccatctacatggccaagaagcccgtgcaactgcccggctactactacgtggacaccaagctggacatcacctcccacaacgaggactacaccatcgtggaacagtacgagcgctccgagggccgccaccacctgttcctgtacggcatggacgagctgtacaagtagattgtcgggaagatgcgtgatctgatccttccactcagcaaaagttcgatttattcaacaaagccgccgtcccgtcaagtcagcgtaatgctctgccagtgttacaaccaattaaccaattctgattagaaaaactcatcgagcatcaaatgaaactgcaatttattcatatcaggattatcaataccatatttttgaaaaagccgtttctgtaatgaaggagaaaactcaccgaggcagttccataggatggcaagatcctggtatcggtctgcgattccgactcgtccaacatcaatacaacctattaatttcccctcgtcaaaaataaggttatcaagtgagaaatcaccatgagtgacgactgaatccggtgagaatggcaaaagcttatgcatttctttccagacttgttcaacaggccagccattacgctcgtcatcaaaatcactcgcatcaaccaaaccgttattcattcgtgattgcgcctgagcgagacgaaatacgcgatcgctgttaaaaggacaattacaaacaggaatcgaatgcaaccggcgcaggaacactgccagcgcatcaacaatattttcacctgaatcaggatattcttctaatacctggaatgctgttttcccggggatcgcagtggtgagtaaccatgcatcatcaggagtacggataaaatgcttgatggtcggaagaggcataaattccgtcagccagtttagtctgaccatctcatctgtaacatcattggcaacgctacctttgccatgtttcagaaacaactctggcgcatcgggcttcccatacaatcgatagattgtcgcacctgattgcccgacattatcgcgagcccatttatacccatataaatcagcatccatgttggaatttaatcgcggcctcgagcaagacgtttcccgttgaatatggctcataacaccccttgtattactgtttatgtaagcagacagttttattgttcatgatgatatatttttatcttgtgcaatgtaacatcagagattttgagacacaacgtggctttcgacttccggcaagctatacgcgccctagaattgtcaattttaatcctctgtttatcggcagttcgtagagcgcgccgtgcgtcccgagcgatactgagcgaagcaagtgcgtcgagcagtgcccgcttgttcctgaaatgccagtaaagcgctggctgctgaacccccagccggaactgaccccacaaggccctagcgtttgcaatgcaccaggtcatcattgacccaggcgtgttccaccaggccgctgcctcgcaactcttcgcaggcttcgccgacctgctcgcgccacttcttcacgcgggtggaatccgatccgcacatgaggcggaaggtttccagcttgagcgggtacggctcccggtgcgagctgaaatagtcgaacatccgtcgggccgtcggcgacagcttgcggtacttctcccatatgaatttcgtgtagtggtcgccagcaaacagcacgacgatttcctcgtcgatcaggacctggcaacgggacgttttcttgccacggtccaggacgcggaagcggtgcagcagcgacaccgattccaggtgcccaacgcggtcggacgtgaagcccatcgccgtcgcctgtaggcgcgacaggcattcctcggccttcgtgtaataccggccattgatcgaccagcccaggtcctggcaaagctcgtagaacgtgaaggtgatcggctcgccgataggggtgcgcttcgcgtactccaacacctgctgccacaccagttcgtcatcgtcggcccgcagctcgacgccggtgtaggtgatcttcacgtccttgttgacgtggaaaatgaccttgttttgcagcgcctcgcgcgggattttcttgttgcgcgtggtgaacagggcagagcgggccgtgtcgtttggcatcgctcgcatcgtgtccggccacggcgcaatatcgaacaaggaaagctgcatttccttgatctgctgcttcgtgtgtttcagcaacgcggcctgcttggcctcgctgacctgttttgccaggtcctcgccggcggtttttcgcttcttggtcgtcatagttcctcgcgtgtcgatggtcatcgacttcgccaaacctgccgcctcctgttcgagacgacgcgaacgctccacggcggccgatggcgcgggcagggcagggggagccagttgcacgctgtcgcgctcgatcttggccgtagcttgctggaccatcgagccgacggactggaaggtttcgcggggcgcacgcatgacggtgcggcttgcgatggtttcggcatcctcggcggaaaaccccgcgtcgatcagttcttgcctgtatgccttccggtcaaacgtccgattcattcaccctccttgcgggattgccccgactcacgccggggcaatgtgcccttattcctgatttgacccgcctggtgccttggtgtccagataatccaccttatcggcaatgaagtcggtcccgtagaccgtctggccgtccttctcgtacttggtattccgaatcttgccctgcacgaataccagctccgcgaagtcgctcttcttgatggagcgcatggggacgtgcttggcaatcacgcgcaccccccggccgttttagcggctaaaaaagtcatggctctgccctcgggcggaccacgcccatcatgaccttgccaagctcgtcctgcttctcttcgatcttcgccagcagggcgaggatcgtggcatcaccgaaccgcgccgtgcgcgggtcgtcggtgagccagagtttcagcaggccgcccaggcggcccaggtcgccattgatgcgggccagctcgcggacgtgctcatagtccacgacgcccgtgattttgtagccctggccgacggccagcaggtaggcctacaggctcatgccggccgccgccgccttttcctcaatcgctcttcgttcgtctggaaggcagtacaccttgataggtgggctgcccttcctggttggcttggtttcatcagccatccgcttgccctcatctgttacgccggcggtagccggccagcctcgcagagcaggattcccgttgagcaccgccaggtgcgaataagggacagtgaagaaggaacacccgctcgcgggtgggcctacttcacctatcctgcccggctgacgccgttggatacaccaaggaaagtctacacgaaccctttggcaaaatcctgtatatcgtgcgaaaaaggatggatataccgaaaaaatcgctataatgaccccgaagcagggttatgcagcggaaaagatccgtc

SEQ ID NO: 44 - DNA, 5984 bp, Artificial Sequence
  pSEVA131-phGESS4-sf
ttaattaaagcggataacaatttcacacaggattagccttcgatgccgattttcttcagccgataggccagtgccggtcggcttaggccgagcaagcgcgcggcaccggagacgttttggttggcctgttgcatggctttgcgcatcaggctttcctcgatctcgtcgaggctcaggccgctgctcaacaactggctgatccaactgccctggccattgcctggctgaatcagcacgccgtccgacgacacccgctcgctggcggtctgcggctcttccggcgcccgtgggaacagcgcctgcacgctgatgctttcgttcggatcggtgaggatgatgccgcgctcgatgacgttctccagctcacggatattgcccggccaactgtaatgcaggcaggcctccagggctttgtctgaaaggccgagggttctcttgccgtactcctggtggaagcgctgaaggaagtgctcaaccagcagtggaatgtcctcgcggcgttcgcgcaacgccgggatcgccaccgggaaaacgttcagccggtagtacaggtcggcgcgaaaacgcccggccttgaccgcttcggccaggtcctcgtgggtggctgcgataacccttacgtcgatcttgcgcgtgcggttgtcgccaactcgctccagctcgccttcttgcagcacgcgcagcagactggcctgagcgcgcgggctgagttcgatcacctcgtcaaggaagatggtgcccttgtcggcccgctcgaagcggcccatgcgtgactgggtggcgccggtgaaggcgcctttttccacgccgaacaattcggactcgatcaggtccggcgggatcgccgcacagttcaccgcgacaaagggctcggcggcgcgtttgctgcgcaggtgcacgctacgcgcgatgacctccttgccgaccccggtctcgccaagcagcagcaccgagactttgccctgtgcggccttgtccatcatattgcgcacggtctggtaggccggggtctgaccgatgccgtagtactggccttcctgtttgtcgaggttggtacgcagcgacaccagttgcgattgcaactcgtagagttcctcgatgatggggtcgttcttgaaatactgtttgaagctggcaacgtcgtcccactcttcggccggcttgccaatgacccggcacttgtcgccgccgcagccgcggcagctgacttccttgaagatgatttcccggcccatgaacgccgaggaataggcgcaggcgtagccgagcagagtccagcacaccgggtcttgcatctgccccaggtcggtctggcagatttccacctcgaaggagtcgatccactccatctcggcatagaagcgcccgcattccttgtcgatatcgacctcggtggggcggaccttgaccagacccttgagcgaatgcagctgcgggccggcgaggaacatgtcgtactcgctggcattcggtctaagcttcctggccagttcggcatccttcaggccggactggtaaccctggcgcaggaagaagcccttggcgcgttcgatgcccagggtattgaccatttcccggcgaaagctggccattgctgaaacctgcagcaacagcatgcgttgttcgccaagccagatcttgccttccgtgctctggaagtggatcaggttggtcaggtccttgaaatcggagtgctggatttcaggcttgtacttgatcggcatgtaagcgaggcccctatttatttttagatggggaaatcagggtcgccgctatagcgcaaggcaggcggcgattccagatggggtcatggggaaaatcggcagttttttcacctgcgccagctccccatagccgacctcagtatctggcaaaagtcaaccaaatgatcaatcgacggcagtgactttagtgctagagatcagccttcagctgcgccatgagcatttgctcaagcggccttgggcaattgatcaaatgcttaaaaagcctgcgcaagcgcggcttaatttcgctcgctccgatcattctaaaaattagaaacacattgaaaaacaataccttgaagtcggttttcagaccttggcacagctgttgcactttgtcctgcgcaatccgccaacctggagaaggagatatacatatgagcaaaggtgaagaactgtttaccggcgttgtgccgattctggtggaactggatggcgatgtgaacggtcacaaattcagcgtgcgtggtgaaggtgaaggcgatgccacgattggcaaactgacgctgaaatttatctgcaccaccggcaaactgccggtgccgtggccgacgctggtgaccaccctgacctatggcgttcagtgttttagtcgctatccggatcacatgaaacgtcacgatttctttaaatctgcaatgccggaaggctatgtgcaggaacgtacgattagctttaaagatgatggcaaatataaaacgcgcgccgttgtgaaatttgaaggcgataccctggtgaaccgcattgaactgaaaggcacggattttaaagaagatggcaatatcctgggccataaactggaatacaactttaatagccataatgtttatattacggcggataaacagaaaaatggcatcaaagcgaattttaccgttcgccataacgttgaagatggcagtgtgcagctggcagatcattatcagcagaataccccgattggtgatggtccggtgctgctgccggataatcattatctgagcacgcagaccgttctgtctaaagatccgaacgaaaaacgggaccacatggttctgcacgaatatgtgaatgcggcaggtattacgtggagccatccgcagttcgaaaaataagatcctacaaggaggtaccagtcgtgactgggaaaaccctggcgactagtcttggactcctgttgatagatccagtaatgacctcagaactccatctggatttgttcagaacgctcggttgccgccgggcgttttttattggtgagaatccaggggtccccaataattacgatttaaattagtagcccgcctaatgagcgggcttttttttaattcccctatttgtttatttttctaaatacattcaaatatgtatccgctcatgagacaataaccctgataaatgcttcaataatattgaaaaaggaagagtatgagcattcagcattttcgtgtggcgctgattccgttttttgcggcgttttgcctgccggtgtttgcgcatccggaaaccctggtgaaagtgaaagatgcggaagatcaactgggtgcgcgcgtgggctatattgaactggatctgaacagcggcaaaattctggaatcttttcgtccggaagaacgttttccgatgatgagcacctttaaagtgctgctgtgcggtgcggttctgagccgtgtggatgcgggccaggaacaactgggccgtcgtattcattatagccagaacgatctggtggaatatagcccggtgaccgaaaaacatctgaccgatggcatgaccgtgcgtgaactgtgcagcgcggcgattaccatgagcgataacaccgcggcgaacctgctgctgacgaccattggcggtccgaaagaactgaccgcgtttctgcataacatgggcgatcatgtgacccgtctggatcgttgggaaccggaactgaacgaagcgattccgaacgatgaacgtgataccaccatgccggcagcaatggcgaccaccctgcgtaaactgctgacgggtgagctgctgaccctggcaagccgccagcaactgattgattggatggaagcggataaagtggcgggtccgctgctgcgtagcgcgctgccggctggctggtttattgcggataaaagcggtgcgggcgaacgtggcagccgtggcattattgcggcgctgggcccggatggtaaaccgagccgtattgtggtgatttataccaccggcagccaggcgacgatggatgaacgtaaccgtcagattgcggaaattggcgcgagcctgattaaacattggtaaaccgatacaattaaaggctccttttggagcctttttttttggacgacccttgtccttttccgctgcataaccctgcttcggggtcattatagcgattttttcggtatatccatcctttttcgcacgatatacaggattttgccaaagggttcgtgtagactttccttggtgtatccaacggcgtcagccgggcaggataggtgaagtaggcccacccgcgagcgggtgttccttcttcactgtcccttattcgcacctggcggtgctcaacgggaatcctgctctgcgaggctggccgtaggccggccctaccggcgcggcagcgttacccgtgtcggcggctccaacggctcgccatcgtccagaaaacacggctcatcgggcatcggcaggcgctgctgcccgcgccgttcccattcctccgtttcggtcaaggctggcaggtctggttccatgcccggaatgccgggctggctgggcggctcctcgccggggccggtcggtagttgctgctcgcccggatacagggtcgggatgcggcgcaggtcgccatgccccaacagcgattcgtcctggtcgtcgtgatcaaccaccacggcggcactgaacaccgacaggcgcaactggtcgcggggctggccccacgccacgcggtcattgaccacgtaggccgacacggtgccggggccgttgagcttcacgacggagatccagcgctcggccaccaagtccttgactgcgtattggaccgtccgcaaagaacgtccgatgagcttggaaagtgtcttctggctgaccaccacggcgttctggtggcccatctgcgccacgaggtgatgcagcagcattgccgccgtgggtttcctcgcaataagcccggcccacgcctcatgcgctttgcgttccgtttgcacccagtgaccgggcttgttcttggcttgaatgccgatttctctggactgcgtggccatgcttatctccatgcggtaggggtgccgcacggttgcggcaccatgcgcaatcagctgcaacttttcggcagcgcgacaacaattatgcgttgcgtaaaagtggcagtcaattacagattttctttaacctacgcaatgagctattgcggggggtgccgcaatgagctgttgcgtaccccccttttttaagttgttgatttttaagtctttcgcatttcgccctatatctagttctttggtgcccaaagaagggcacccctgcggggttcccccacgccttcggcgcggctccccctccggcaaaaagtggcccctccggggcttgttgatcgactgcgcggccttcggccttgcccaaggtggcgctgcccccttggaacccccgcactcgccgccgtgaggctcggggggcaggcgggcgggcttcgcccttcgactgcccccactcgcataggcttgggtcgttccaggcgcgtcaaggccaagccgctgcgcggtcgctgcgcgagccttgacccgccttccacttggtgtccaaccggcaagcgaagcgcgcaggccgcaggccggaggcttttccccagagaaaattaaaaaaattgatggggcaaggccgcaggccgcgcagttggagccggtgggtatgtggtcgaaggctgggtagccggtgggcaatccctgtggtcaagctcgtgggcaggcgcagcctgtccatcagcttgtccagcagggttgtccacgggccgagcgaagcgagccagccggtggccgctcgcggccatcgtccacatatccacgggctggcaagggagcgcagcgaccgcgcagggcgaagcccggagagcaagcccgtagggggggcgcgcccagctgtctagggcggcggatttgtcctactcaggagagcgttcaccgacaaacaacagataaaacgaaaggcccagtctttcgactgagcctttcgttttatttgatgcct

SEQ ID NO: 45 - DNA, 2172 bp, Artificial Sequence
  DNA fragment containing DmpR and PO amplified with pAWPS-PO(SpeI)-F primer and pAWPS-PO(XbaI)-R primer using pSEVA131-phGESS4-sf as a template
ctatcaacaggagtccaagactagtagcggataacaatttcacacaggattagccttcgatgccgattttcttcagccgataggccagtgccggtcggcttaggccgagcaagcgcgcggcaccggagacgttttggttggcctgttgcatggctttgcgcatcaggctttcctcgatctcgtcgaggctcaggccgctgctcaacaactggctgatccaactgccctggccattgcctggctgaatcagcacgccgtccgacgacacccgctcgctggcggtctgcggctcttccggcgcccgtgggaacagcgcctgcacgctgatgctttcgttcggatcggtgaggatgatgccgcgctcgatgacgttctccagctcacggatattgcccggccaactgtaatgcaggcaggcctccagggctttgtctgaaaggccgagggttctcttgccgtactcctggtggaagcgctgaaggaagtgctcaaccagcagtggaatgtcctcgcggcgttcgcgcaacgccgggatcgccaccgggaaaacgttcagccggtagtacaggtcggcgcgaaaacgcccggccttgaccgcttcggccaggtcctcgtgggtggctgcgataacccttacgtcgatcttgcgcgtgcggttgtcgccaactcgctccagctcgccttcttgcagcacgcgcagcagactggcctgagcgcgcgggctgagttcgatcacctcgtcaaggaagatggtgcccttgtcggcccgctcgaagcggcccatgcgtgactgggtggcgccggtgaaggcgcctttttccacgccgaacaattcggactcgatcaggtccggcgggatcgccgcacagttcaccgcgacaaagggctcggcggcgcgtttgctgcgcaggtgcacgctacgcgcgatgacctccttgccgaccccggtctcgccaagcagcagcaccgagactttgccctgtgcggccttgtccatcatattgcgcacggtctggtaggccggggtctgaccgatgccgtagtactggccttcctgtttgtcgaggttggtacgcagcgacaccagttgcgattgcaactcgtagagttcctcgatgatggggtcgttcttgaaatactgtttgaagctggcaacgtcgtcccactcttcggccggcttgccaatgacccggcacttgtcgccgccgcagccgcggcagctgacttccttgaagatgatttcccggcccatgaacgccgaggaataggcgcaggcgtagccgagcagagtccagcacaccgggtcttgcatctgccccaggtcggtctggcagatttccacctcgaaggagtcgatccactccatctcggcatagaagcgcccgcattccttgtcgatatcgacctcggtggggcggaccttgaccagacccttgagcgaatgcagctgcgggccggcgaggaacatgtcgtactcgctggcattcggtctaagcttcctggccagttcggcatccttcaggccggactggtaaccctggcgcaggaagaagcccttggcgcgttcgatgcccagggtattgaccatttcccggcgaaagctggccattgctgaaacctgcagcaacagcatgcgttgttcgccaagccagatcttgccttccgtgctctggaagtggatcaggttggtcaggtccttgaaatcggagtgctggatttcaggcttgtacttgatcggcatgtaagcgaggcccctatttatttttagatggggaaatcagggtcgccgctatagcgcaaggcaggcggcgattccagatggggtcatggggaaaatcggcagttttttcacctgcgccagctccccatagccgacctcagtatctggcaaaagtcaaccaaatgatcaatcgacggcagtgactttagtgctagagatcagccttcagctgcgccatgagcatttgctcaagcggccttgggcaattgatcaaatgcttaaaaagcctgcgcaagcgcggcttaatttcgctcgctccgatcattctaaaaattagaaacacattgaaaaacaataccttgaagtcggttttcagaccttggcacagctgttgcactttgtcctgcgcaatccgccaacctggagatctagaaataattttgtttaacttt

SEQ ID NO: 46 - DNA, 7219 bp, Artificial Sequence
  pAWP89S-Po-dTomato
gaccctttccgacgctcaccgggctggttgccctcgccgctgggctggcggccgtctatggccctgcaaacgcgccagaaacgccgtcgaagccgtgtgcgagacaccgcggccgccggcgttgtggatacctcgcggaaaacttggccctcactgacagatgaggggcggacgttgacacttgaggggccgactcacccggcgcggcgttgacagatgaggggcaggctcgatttcggccggcgacgtggagctggccagcctcgcaaatcggcgaaaacgcctgattttacgcgagtttcccacagatgatgtggacaagcctggggataagtgccctgcggtattgacacttgaggggcgcgactactgacagatgaggggcgcgatccttgacacttgaggggcagagtgctgacagatgaggggcgcacctattgacatttgaggggctgtccacaggcagaaaatccagcatttgcaagggtttccgcccgtttttcggccaccgctaacctgtcttttaacctgcttttaaaccaatatttataaaccttgtttttaaccagggctgcgccctgtgcgcgtgaccgcgcacgccgaaggggggtgcccccccttctcgaaccctcccggcccgctaacgcgggcctcccatccccccaggggctgcgcccctcggccgcgaacggcctcaccccaaaaatggcagccaagctgacccgctagggacgtgaagtcgattccttcgatggttagcaatcaaagactcagagtgctgtctggagcgtgaatctaacggtacgtatctcgattgctcggtcgctattcgcactctgcgaaagttcgtaccgctcattcactaggttgcgaaatcagagattttgagacacaaatttaaatcgtaattattggggacccctggattctcaccaataaaaaacgcccggcggcaaccgagcgttctgaacaaatccagatggagttctgaggtcattactggatctatcaacaggagtccaagactagtagcggataacaatttcacacaggattagccttcgatgccgattttcttcagccgataggccagtgccggtcggcttaggccgagcaagcgcgcggcaccggagacgttttggttggcctgttgcatggctttgcgcatcaggctttcctcgatctcgtcgaggctcaggccgctgctcaacaactggctgatccaactgccctggccattgcctggctgaatcagcacgccgtccgacgacacccgctcgctggcggtctgcggctcttccggcgcccgtgggaacagcgcctgcacgctgatgctttcgttcggatcggtgaggatgatgccgcgctcgatgacgttctccagctcacggatattgcccggccaactgtaatgcaggcaggcctccagggctttgtctgaaaggccgagggttctcttgccgtactcctggtggaagcgctgaaggaagtgctcaaccagcagtggaatgtcctcgcggcgttcgcgcaacgccgggatcgccaccgggaaaacgttcagccggtagtacaggtcggcgcgaaaacgcccggccttgaccgcttcggccaggtcctcgtgggtggctgcgataacccttacgtcgatcttgcgcgtgcggttgtcgccaactcgctccagctcgccttcttgcagcacgcgcagcagactggcctgagcgcgcgggctgagttcgatcacctcgtcaaggaagatggtgcccttgtcggcccgctcgaagcggcccatgcgtgactgggtggcgccggtgaaggcgcctttttccacgccgaacaattcggactcgatcaggtccggcgggatcgccgcacagttcaccgcgacaaagggctcggcggcgcgtttgctgcgcaggtgcacgctacgcgcgatgacctccttgccgaccccggtctcgccaagcagcagcaccgagactttgccctgtgcggccttgtccatcatattgcgcacggtctggtaggccggggtctgaccgatgccgtagtactggccttcctgtttgtcgaggttggtacgcagcgacaccagttgcgattgcaactcgtagagttcctcgatgatggggtcgttcttgaaatactgtttgaagctggcaacgtcgtcccactcttcggccggcttgccaatgacccggcacttgtcgccgccgcagccgcggcagctgacttccttgaagatgatttcccggcccatgaacgccgaggaataggcgcaggcgtagccgagcagagtccagcacaccgggtcttgcatctgccccaggtcggtctggcagatttccacctcgaaggagtcgatccactccatctcggcatagaagcgcccgcattccttgtcgatatcgacctcggtggggcggaccttgaccagacccttgagcgaatgcagctgcgggccggcgaggaacatgtcgtactcgctggcattcggtctaagcttcctggccagttcggcatccttcaggccggactggtaaccctggcgcaggaagaagcccttggcgcgttcgatgcccagggtattgaccatttcccggcgaaagctggccattgctgaaacctgcagcaacagcatgcgttgttcgccaagccagatcttgccttccgtgctctggaagtggatcaggttggtcaggtccttgaaatcggagtgctggatttcaggcttgtacttgatcggcatgtaagcgaggcccctatttatttttagatggggaaatcagggtcgccgctatagcgcaaggcaggcggcgattccagatggggtcatggggaaaatcggcagttttttcacctgcgccagctccccatagccgacctcagtatctggcaaaagtcaaccaaatgatcaatcgacggcagtgactttagtgctagagatcagccttcagctgcgccatgagcatttgctcaagcggccttgggcaattgatcaaatgcttaaaaagcctgcgcaagcgcggcttaatttcgctcgctccgatcattctaaaaattagaaacacattgaaaaacaataccttgaagtcggttttcagaccttggcacagctgttgcactttgtcctgcgcaatccgccaacctggagatctagaaataattttgtttaactttaagaaggagatatacatatggtgagcaagggcgaggaggtcatcaaagagttcatgcgcttcaaggtgcgcatggagggctccatgaacggccacgagttcgagatcgagggcgagggcgagggccgcccctacgagggcacccagaccgccaagctgaaggtgaccaagggcggccccctgcccttcgcctgggacatcctgtccccccagttcatgtacggctccaaggcgtacgtgaagcaccccgccgacatccccgattacaagaagctgtccttccccgagggcttcaagtgggagcgcgtgatgaacttcgaggacggcggtctggtgaccgtgacccaggactcctccctgcaggacggcacgctgatctacaaggtgaagatgcgcggcaccaacttcccccccgacggccccgtaatgcagaagaagaccatgggctgggaggcctccaccgagcgcctgtacccccgcgacggcgtgctgaagggcgagatccaccaggccctgaagctgaaggacggcggccactacctggtggagttcaagaccatctacatggccaagaagcccgtgcaactgcccggctactactacgtggacaccaagctggacatcacctcccacaacgaggactacaccatcgtggaacagtacgagcgctccgagggccgccaccacctgttcctgtacggcatggacgagctgtacaagtagattgtcgggaagatgcgtgatctgatccttccactcagcaaaagttcgatttattcaacaaagccgccgtcccgtcaagtcagcgtaatgctctgccagtgttacaaccaattaaccaattctgattagaaaaactcatcgagcatcaaatgaaactgcaatttattcatatcaggattatcaataccatatttttgaaaaagccgtttctgtaatgaaggagaaaactcaccgaggcagttccataggatggcaagatcctggtatcggtctgcgattccgactcgtccaacatcaatacaacctattaatttcccctcgtcaaaaataaggttatcaagtgagaaatcaccatgagtgacgactgaatccggtgagaatggcaaaagcttatgcatttctttccagacttgttcaacaggccagccattacgctcgtcatcaaaatcactcgcatcaaccaaaccgttattcattcgtgattgcgcctgagcgagacgaaatacgcgatcgctgttaaaaggacaattacaaacaggaatcgaatgcaaccggcgcaggaacactgccagcgcatcaacaatattttcacctgaatcaggatattcttctaatacctggaatgctgttttcccggggatcgcagtggtgagtaaccatgcatcatcaggagtacggataaaatgcttgatggtcggaagaggcataaattccgtcagccagtttagtctgaccatctcatctgtaacatcattggcaacgctacctttgccatgtttcagaaacaactctggcgcatcgggcttcccatacaatcgatagattgtcgcacctgattgcccgacattatcgcgagcccatttatacccatataaatcagcatccatgttggaatttaatcgcggcctcgagcaagacgtttcccgttgaatatggctcataacaccccttgtattactgtttatgtaagcagacagttttattgttcatgatgatatatttttatcttgtgcaatgtaacatcagagattttgagacacaacgtggctttcgacttccggcaagctatacgcgccctagaattgtcaattttaatcctctgtttatcggcagttcgtagagcgcgccgtgcgtcccgagcgatactgagcgaagcaagtgcgtcgagcagtgcccgcttgttcctgaaatgccagtaaagcgctggctgctgaacccccagccggaactgaccccacaaggccctagcgtttgcaatgcaccaggtcatcattgacccaggcgtgttccaccaggccgctgcctcgcaactcttcgcaggcttcgccgacctgctcgcgccacttcttcacgcgggtggaatccgatccgcacatgaggcggaaggtttccagcttgagcgggtacggctcccggtgcgagctgaaatagtcgaacatccgtcgggccgtcggcgacagcttgcggtacttctcccatatgaatttcgtgtagtggtcgccagcaaacagcacgacgatttcctcgtcgatcaggacctggcaacgggacgttttcttgccacggtccaggacgcggaagcggtgcagcagcgacaccgattccaggtgcccaacgcggtcggacgtgaagcccatcgccgtcgcctgtaggcgcgacaggcattcctcggccttcgtgtaataccggccattgatcgaccagcccaggtcctggcaaagctcgtagaacgtgaaggtgatcggctcgccgataggggtgcgcttcgcgtactccaacacctgctgccacaccagttcgtcatcgtcggcccgcagctcgacgccggtgtaggtgatcttcacgtccttgttgacgtggaaaatgaccttgttttgcagcgcctcgcgcgggattttcttgttgcgcgtggtgaacagggcagagcgggccgtgtcgtttggcatcgctcgcatcgtgtccggccacggcgcaatatcgaacaaggaaagctgcatttccttgatctgctgcttcgtgtgtttcagcaacgcggcctgcttggcctcgctgacctgttttgccaggtcctcgccggcggtttttcgcttcttggtcgtcatagttcctcgcgtgtcgatggtcatcgacttcgccaaacctgccgcctcctgttcgagacgacgcgaacgctccacggcggccgatggcgcgggcagggcagggggagccagttgcacgctgtcgcgctcgatcttggccgtagcttgctggaccatcgagccgacggactggaaggtttcgcggggcgcacgcatgacggtgcggcttgcgatggtttcggcatcctcggcggaaaaccccgcgtcgatcagttcttgcctgtatgccttccggtcaaacgtccgattcattcaccctccttgcgggattgccccgactcacgccggggcaatgtgcccttattcctgatttgacccgcctggtgccttggtgtccagataatccaccttatcggcaatgaagtcggtcccgtagaccgtctggccgtccttctcgtacttggtattccgaatcttgccctgcacgaataccagctccgcgaagtcgctcttcttgatggagcgcatggggacgtgcttggcaatcacgcgcaccccccggccgttttagcggctaaaaaagtcatggctctgccctcgggcggaccacgcccatcatgaccttgccaagctcgtcctgcttctcttcgatcttcgccagcagggcgaggatcgtggcatcaccgaaccgcgccgtgcgcgggtcgtcggtgagccagagtttcagcaggccgcccaggcggcccaggtcgccattgatgcgggccagctcgcggacgtgctcatagtccacgacgcccgtgattttgtagccctggccgacggccagcaggtaggcctacaggctcatgccggccgccgccgccttttcctcaatcgctcttcgttcgtctggaaggcagtacaccttgataggtgggctgcccttcctggttggcttggtttcatcagccatccgcttgccctcatctgttacgccggcggtagccggccagcctcgcagagcaggattcccgttgagcaccgccaggtgcgaataagggacagtgaagaaggaacacccgctcgcgggtgggcctacttcacctatcctgcccggctgacgccgttggatacaccaaggaaagtctacacgaaccctttggcaaaatcctgtatatcgtgcgaaaaaggatggatataccgaaaaaatcgctataatgaccccgaagcagggttatgcagcggaaaagatccgtc

SEQ ID NO: 47 - protein, 560 aa, Artificial Sequence
  DmpR wild type
MPIKYKPEIQHSDFKDLTNLIHFQSTEGKIWLGEQRMLLLQVSAMASFRREMVNTLGIERAKGFFLRQGYQSGLKDAELARKLRPNASEYDMFLAGPQLHSLKGLVKVRPTEVDIDKECGRFYAEMEWIDSFEVEICQTDLGQMQDPVCWTLLGYACAYSSAFMGREIIFKEVSCRGCGGDKCRVIGKPAEEWDDVASFKQYFKNDPIIEELYELQSQLVSLRTNLDKQEGQYYGIGQTPAYQTVRNMMDKAAQGKVSVLLLGETGVGKEVIARSVHLRSKRAAEPFVAVNCAAIPPDLIESELFGVEKGAFTGATQSRMGRFERADKGTIFLDEVIELSPRAQASLLRVLQEGELERVGDNRTRKIDVRVIAATHEDLAEAVKAGRFRADLYYRLNVFPVAIPALRERREDIPLLVEHFLQRFHQEYGKRTLGLSDKALEACLHYSWPGNIRELENVIERGIILTDPNESISVQALFPRAPEEPQTASERVSSDGVLIQPGNGQGSWISQLLSSGLSLDEIEESLMRKAMQQANQNVSGAARLLGLSRPALAYRLKKIG

SEQ ID NO: 48 - DNA, 6610 bp, Artificial Sequence
  pAWP89S-Po-dTomato-DmpR(d2-204)
gaccctttccgacgctcaccgggctggttgccctcgccgctgggctggcggccgtctatggccctgcaaacgcgccagaaacgccgtcgaagccgtgtgcgagacaccgcggccgccggcgttgtggatacctcgcggaaaacttggccctcactgacagatgaggggcggacgttgacacttgaggggccgactcacccggcgcggcgttgacagatgaggggcaggctcgatttcggccggcgacgtggagctggccagcctcgcaaatcggcgaaaacgcctgattttacgcgagtttcccacagatgatgtggacaagcctggggataagtgccctgcggtattgacacttgaggggcgcgactactgacagatgaggggcgcgatccttgacacttgaggggcagagtgctgacagatgaggggcgcacctattgacatttgaggggctgtccacaggcagaaaatccagcatttgcaagggtttccgcccgtttttcggccaccgctaacctgtcttttaacctgcttttaaaccaatatttataaaccttgtttttaaccagggctgcgccctgtgcgcgtgaccgcgcacgccgaaggggggtgcccccccttctcgaaccctcccggcccgctaacgcgggcctcccatccccccaggggctgcgcccctcggccgcgaacggcctcaccccaaaaatggcagccaagctgacccgctagggacgtgaagtcgattccttcgatggttagcaatcaaagactcagagtgctgtctggagcgtgaatctaacggtacgtatctcgattgctcggtcgctattcgcactctgcgaaagttcgtaccgctcattcactaggttgcgaaatcagagattttgagacacaaatttaaatcgtaattattggggacccctggattctcaccaataaaaaacgcccggcggcaaccgagcgttctgaacaaatccagatggagttctgaggtcattactggatctatcaacaggagtccaagactagtagcggataacaatttcacacaggattagccttcgatgccgattttcttcagccgataggccagtgccggtcggcttaggccgagcaagcgcgcggcaccggagacgttttggttggcctgttgcatggctttgcgcatcaggctttcctcgatctcgtcgaggctcaggccgctgctcaacaactggctgatccaactgccctggccattgcctggctgaatcagcacgccgtccgacgacacccgctcgctggcggtctgcggctcttccggcgcccgtgggaacagcgcctgcacgctgatgctttcgttcggatcggtgaggatgatgccgcgctcgatgacgttctccagctcacggatattgcccggccaactgtaatgcaggcaggcctccagggctttgtctgaaaggccgagggttctcttgccgtactcctggtggaagcgctgaaggaagtgctcaaccagcagtggaatgtcctcgcggcgttcgcgcaacgccgggatcgccaccgggaaaacgttcagccggtagtacaggtcggcgcgaaaacgcccggccttgaccgcttcggccaggtcctcgtgggtggctgcgataacccttacgtcgatcttgcgcgtgcggttgtcgccaactcgctccagctcgccttcttgcagcacgcgcagcagactggcctgagcgcgcgggctgagttcgatcacctcgtcaaggaagatggtgcccttgtcggcccgctcgaagcggcccatgcgtgactgggtggcgccggtgaaggcgcctttttccacgccgaacaattcggactcgatcaggtccggcgggatcgccgcacagttcaccgcgacaaagggctcggcggcgcgtttgctgcgcaggtgcacgctacgcgcgatgacctccttgccgaccccggtctcgccaagcagcagcaccgagactttgccctgtgcggccttgtccatcatattgcgcacggtctggtaggccggggtctgaccgatgccgtagtactggccttcctgtttgtcgaggttggtacgcagcgacaccagttgcgattgcaactcgtagagttcctcgatgatggggtcgttcatgtaagcgaggcccctatttatttttagatggggaaatcagggtcgccgctatagcgcaaggcaggcggcgattccagatggggtcatggggaaaatcggcagttttttcacctgcgccagctccccatagccgacctcagtatctggcaaaagtcaaccaaatgatcaatcgacggcagtgactttagtgctagagatcagccttcagctgcgccatgagcatttgctcaagcggccttgggcaattgatcaaatgcttaaaaagcctgcgcaagcgcggcttaatttcgctcgctccgatcattctaaaaattagaaacacattgaaaaacaataccttgaagtcggttttcagaccttggcacagctgttgcactttgtcctgcgcaatccgccaacctggagatctagaaataattttgtttaactttaagaaggagatatacatatggtgagcaagggcgaggaggtcatcaaagagttcatgcgcttcaaggtgcgcatggagggctccatgaacggccacgagttcgagatcgagggcgagggcgagggccgcccctacgagggcacccagaccgccaagctgaaggtgaccaagggcggccccctgcccttcgcctgggacatcctgtccccccagttcatgtacggctccaaggcgtacgtgaagcaccccgccgacatccccgattacaagaagctgtccttccccgagggcttcaagtgggagcgcgtgatgaacttcgaggacggcggtctggtgaccgtgacccaggactcctccctgcaggacggcacgctgatctacaaggtgaagatgcgcggcaccaacttcccccccgacggccccgtaatgcagaagaagaccatgggctgggaggcctccaccgagcgcctgtacccccgcgacggcgtgctgaagggcgagatccaccaggccctgaagctgaaggacggcggccactacctggtggagttcaagaccatctacatggccaagaagcccgtgcaactgcccggctactactacgtggacaccaagctggacatcacctcccacaacgaggactacaccatcgtggaacagtacgagcgctccgagggccgccaccacctgttcctgtacggcatggacgagctgtacaagtagattgtcgggaagatgcgtgatctgatccttccactcagcaaaagttcgatttattcaacaaagccgccgtcccgtcaagtcagcgtaatgctctgccagtgttacaaccaattaaccaattctgattagaaaaactcatcgagcatcaaatgaaactgcaatttattcatatcaggattatcaataccatatttttgaaaaagccgtttctgtaatgaaggagaaaactcaccgaggcagttccataggatggcaagatcctggtatcggtctgcgattccgactcgtccaacatcaatacaacctattaatttcccctcgtcaaaaataaggttatcaagtgagaaatcaccatgagtgacgactgaatccggtgagaatggcaaaagcttatgcatttctttccagacttgttcaacaggccagccattacgctcgtcatcaaaatcactcgcatcaaccaaaccgttattcattcgtgattgcgcctgagcgagacgaaatacgcgatcgctgttaaaaggacaattacaaacaggaatcgaatgcaaccggcgcaggaacactgccagcgcatcaacaatattttcacctgaatcaggatattcttctaatacctggaatgctgttttcccggggatcgcagtggtgagtaaccatgcatcatcaggagtacggataaaatgcttgatggtcggaagaggcataaattccgtcagccagtttagtctgaccatctcatctgtaacatcattggcaacgctacctttgccatgtttcagaaacaactctggcgcatcgggcttcccatacaatcgatagattgtcgcacctgattgcccgacattatcgcgagcccatttatacccatataaatcagcatccatgttggaatttaatcgcggcctcgagcaagacgtttcccgttgaatatggctcataacaccccttgtattactgtttatgtaagcagacagttttattgttcatgatgatatatttttatcttgtgcaatgtaacatcagagattttgagacacaacgtggctttcgacttccggcaagctatacgcgccctagaattgtcaattttaatcctctgtttatcggcagttcgtagagcgcgccgtgcgtcccgagcgatactgagcgaagcaagtgcgtcgagcagtgcccgcttgttcctgaaatgccagtaaagcgctggctgctgaacccccagccggaactgaccccacaaggccctagcgtttgcaatgcaccaggtcatcattgacccaggcgtgttccaccaggccgctgcctcgcaactcttcgcaggcttcgccgacctgctcgcgccacttcttcacgcgggtggaatccgatccgcacatgaggcggaaggtttccagcttgagcgggtacggctcccggtgcgagctgaaatagtcgaacatccgtcgggccgtcggcgacagcttgcggtacttctcccatatgaatttcgtgtagtggtcgccagcaaacagcacgacgatttcctcgtcgatcaggacctggcaacgggacgttttcttgccacggtccaggacgcggaagcggtgcagcagcgacaccgattccaggtgcccaacgcggtcggacgtgaagcccatcgccgtcgcctgtaggcgcgacaggcattcctcggccttcgtgtaataccggccattgatcgaccagcccaggtcctggcaaagctcgtagaacgtgaaggtgatcggctcgccgataggggtgcgcttcgcgtactccaacacctgctgccacaccagttcgtcatcgtcggcccgcagctcgacgccggtgtaggtgatcttcacgtccttgttgacgtggaaaatgaccttgttttgcagcgcctcgcgcgggattttcttgttgcgcgtggtgaacagggcagagcgggccgtgtcgtttggcatcgctcgcatcgtgtccggccacggcgcaatatcgaacaaggaaagctgcatttccttgatctgctgcttcgtgtgtttcagcaacgcggcctgcttggcctcgctgacctgttttgccaggtcctcgccggcggtttttcgcttcttggtcgtcatagttcctcgcgtgtcgatggtcatcgacttcgccaaacctgccgcctcctgttcgagacgacgcgaacgctccacggcggccgatggcgcgggcagggcagggggagccagttgcacgctgtcgcgctcgatcttggccgtagcttgctggaccatcgagccgacggactggaaggtttcgcggggcgcacgcatgacggtgcggcttgcgatggtttcggcatcctcggcggaaaaccccgcgtcgatcagttcttgcctgtatgccttccggtcaaacgtccgattcattcaccctccttgcgggattgccccgactcacgccggggcaatgtgcccttattcctgatttgacccgcctggtgccttggtgtccagataatccaccttatcggcaatgaagtcggtcccgtagaccgtctggccgtccttctcgtacttggtattccgaatcttgccctgcacgaataccagctccgcgaagtcgctcttcttgatggagcgcatggggacgtgcttggcaatcacgcgcaccccccggccgttttagcggctaaaaaagtcatggctctgccctcgggcggaccacgcccatcatgaccttgccaagctcgtcctgcttctcttcgatcttcgccagcagggcgaggatcgtggcatcaccgaaccgcgccgtgcgcgggtcgtcggtgagccagagtttcagcaggccgcccaggcggcccaggtcgccattgatgcgggccagctcgcggacgtgctcatagtccacgacgcccgtgattttgtagccctggccgacggccagcaggtaggcctacaggctcatgccggccgccgccgccttttcctcaatcgctcttcgttcgtctggaaggcagtacaccttgataggtgggctgcccttcctggttggcttggtttcatcagccatccgcttgccctcatctgttacgccggcggtagccggccagcctcgcagagcaggattcccgttgagcaccgccaggtgcgaataagggacagtgaagaaggaacacccgctcgcgggtgggcctacttcacctatcctgcccggctgacgccgttggatacaccaaggaaagtctacacgaaccctttggcaaaatcctgtatatcgtgcgaaaaaggatggatataccgaaaaaatcgctataatgaccccgaagcagggttatgcagcggaaaagatccgtc

SEQ ID NO: 49 - DNA, 7219 bp, Artificial Sequence
  pAWP89S-Po-dTomato-RBS(MDH)
gaccctttccgacgctcaccgggctggttgccctcgccgctgggctggcggccgtctatggccctgcaaacgcgccagaaacgccgtcgaagccgtgtgcgagacaccgcggccgccggcgttgtggatacctcgcggaaaacttggccctcactgacagatgaggggcggacgttgacacttgaggggccgactcacccggcgcggcgttgacagatgaggggcaggctcgatttcggccggcgacgtggagctggccagcctcgcaaatcggcgaaaacgcctgattttacgcgagtttcccacagatgatgtggacaagcctggggataagtgccctgcggtattgacacttgaggggcgcgactactgacagatgaggggcgcgatccttgacacttgaggggcagagtgctgacagatgaggggcgcacctattgacatttgaggggctgtccacaggcagaaaatccagcatttgcaagggtttccgcccgtttttcggccaccgctaacctgtcttttaacctgcttttaaaccaatatttataaaccttgtttttaaccagggctgcgccctgtgcgcgtgaccgcgcacgccgaaggggggtgcccccccttctcgaaccctcccggcccgctaacgcgggcctcccatccccccaggggctgcgcccctcggccgcgaacggcctcaccccaaaaatggcagccaagctgacccgctagggacgtgaagtcgattccttcgatggttagcaatcaaagactcagagtgctgtctggagcgtgaatctaacggtacgtatctcgattgctcggtcgctattcgcactctgcgaaagttcgtaccgctcattcactaggttgcgaaatcagagattttgagacacaaatttaaatcgtaattattggggacccctggattctcaccaataaaaaacgcccggcggcaaccgagcgttctgaacaaatccagatggagttctgaggtcattactggatctatcaacaggagtccaagactagtagcggataacaatttcacacaggattagccttcgatgccgattttcttcagccgataggccagtgccggtcggcttaggccgagcaagcgcgcggcaccggagacgttttggttggcctgttgcatggctttgcgcatcaggctttcctcgatctcgtcgaggctcaggccgctgctcaacaactggctgatccaactgccctggccattgcctggctgaatcagcacgccgtccgacgacacccgctcgctggcggtctgcggctcttccggcgcccgtgggaacagcgcctgcacgctgatgctttcgttcggatcggtgaggatgatgccgcgctcgatgacgttctccagctcacggatattgcccggccaactgtaatgcaggcaggcctccagggctttgtctgaaaggccgagggttctcttgccgtactcctggtggaagcgctgaaggaagtgctcaaccagcagtggaatgtcctcgcggcgttcgcgcaacgccgggatcgccaccgggaaaacgttcagccggtagtacaggtcggcgcgaaaacgcccggccttgaccgcttcggccaggtcctcgtgggtggctgcgataacccttacgtcgatcttgcgcgtgcggttgtcgccaactcgctccagctcgccttcttgcagcacgcgcagcagactggcctgagcgcgcgggctgagttcgatcacctcgtcaaggaagatggtgcccttgtcggcccgctcgaagcggcccatgcgtgactgggtggcgccggtgaaggcgcctttttccacgccgaacaattcggactcgatcaggtccggcgggatcgccgcacagttcaccgcgacaaagggctcggcggcgcgtttgctgcgcaggtgcacgctacgcgcgatgacctccttgccgaccccggtctcgccaagcagcagcaccgagactttgccctgtgcggccttgtccatcatattgcgcacggtctggtaggccggggtctgaccgatgccgtagtactggccttcctgtttgtcgaggttggtacgcagcgacaccagttgcgattgcaactcgtagagttcctcgatgatggggtcgttcttgaaatactgtttgaagctggcaacgtcgtcccactcttcggccggcttgccaatgacccggcacttgtcgccgccgcagccgcggcagctgacttccttgaagatgatttcccggcccatgaacgccgaggaataggcgcaggcgtagccgagcagagtccagcacaccgggtcttgcatctgccccaggtcggtctggcagatttccacctcgaaggagtcgatccactccatctcggcatagaagcgcccgcattccttgtcgatatcgacctcggtggggcggaccttgaccagacccttgagcgaatgcagctgcgggccggcgaggaacatgtcgtactcgctggcattcggtctaagcttcctggccagttcggcatccttcaggccggactggtaaccctggcgcaggaagaagcccttggcgcgttcgatgcccagggtattgaccatttcccggcgaaagctggccattgctgaaacctgcagcaacagcatgcgttgttcgccaagccagatcttgccttccgtgctctggaagtggatcaggttggtcaggtccttgaaatcggagtgctggatttcaggcttgtacttgatcggcatgtaagcgaggcccctatttatttttagatggggaaatcagggtcgccgctatagcgcaaggcaggcggcgattccagatggggtcatggggaaaatcggcagttttttcacctgcgccagctccccatagccgacctcagtatctggcaaaagtcaaccaaatgatcaatcgacggcagtgactttagtgctagagatcagccttcagctgcgccatgagcatttgctcaagcggccttgggcaattgatcaaatgcttaaaaagcctgcgcaagcgcggcttaatttcgctcgctccgatcattctaaaaattagaaacacattgaaaaacaataccttgaagtcggttttcagaccttggcacagctgttgcactttgtcctgcgcaatccgccaacctggagatctagatgcagggtcggcatcaatcattcttggaggagacacatggtgagcaagggcgaggaggtcatcaaagagttcatgcgcttcaaggtgcgcatggagggctccatgaacggccacgagttcgagatcgagggcgagggcgagggccgcccctacgagggcacccagaccgccaagctgaaggtgaccaagggcggccccctgcccttcgcctgggacatcctgtccccccagttcatgtacggctccaaggcgtacgtgaagcaccccgccgacatccccgattacaagaagctgtccttccccgagggcttcaagtgggagcgcgtgatgaacttcgaggacggcggtctggtgaccgtgacccaggactcctccctgcaggacggcacgctgatctacaaggtgaagatgcgcggcaccaacttcccccccgacggccccgtaatgcagaagaagaccatgggctgggaggcctccaccgagcgcctgtacccccgcgacggcgtgctgaagggcgagatccaccaggccctgaagctgaaggacggcggccactacctggtggagttcaagaccatctacatggccaagaagcccgtgcaactgcccggctactactacgtggacaccaagctggacatcacctcccacaacgaggactacaccatcgtggaacagtacgagcgctccgagggccgccaccacctgttcctgtacggcatggacgagctgtacaagtagattgtcgggaagatgcgtgatctgatccttccactcagcaaaagttcgatttattcaacaaagccgccgtcccgtcaagtcagcgtaatgctctgccagtgttacaaccaattaaccaattctgattagaaaaactcatcgagcatcaaatgaaactgcaatttattcatatcaggattatcaataccatatttttgaaaaagccgtttctgtaatgaaggagaaaactcaccgaggcagttccataggatggcaagatcctggtatcggtctgcgattccgactcgtccaacatcaatacaacctattaatttcccctcgtcaaaaataaggttatcaagtgagaaatcaccatgagtgacgactgaatccggtgagaatggcaaaagcttatgcatttctttccagacttgttcaacaggccagccattacgctcgtcatcaaaatcactcgcatcaaccaaaccgttattcattcgtgattgcgcctgagcgagacgaaatacgcgatcgctgttaaaaggacaattacaaacaggaatcgaatgcaaccggcgcaggaacactgccagcgcatcaacaatattttcacctgaatcaggatattcttctaatacctggaatgctgttttcccggggatcgcagtggtgagtaaccatgcatcatcaggagtacggataaaatgcttgatggtcggaagaggcataaattccgtcagccagtttagtctgaccatctcatctgtaacatcattggcaacgctacctttgccatgtttcagaaacaactctggcgcatcgggcttcccatacaatcgatagattgtcgcacctgattgcccgacattatcgcgagcccatttatacccatataaatcagcatccatgttggaatttaatcgcggcctcgagcaagacgtttcccgttgaatatggctcataacaccccttgtattactgtttatgtaagcagacagttttattgttcatgatgatatatttttatcttgtgcaatgtaacatcagagattttgagacacaacgtggctttcgacttccggcaagctatacgcgccctagaattgtcaattttaatcctctgtttatcggcagttcgtagagcgcgccgtgcgtcccgagcgatactgagcgaagcaagtgcgtcgagcagtgcccgcttgttcctgaaatgccagtaaagcgctggctgctgaacccccagccggaactgaccccacaaggccctagcgtttgcaatgcaccaggtcatcattgacccaggcgtgttccaccaggccgctgcctcgcaactcttcgcaggcttcgccgacctgctcgcgccacttcttcacgcgggtggaatccgatccgcacatgaggcggaaggtttccagcttgagcgggtacggctcccggtgcgagctgaaatagtcgaacatccgtcgggccgtcggcgacagcttgcggtacttctcccatatgaatttcgtgtagtggtcgccagcaaacagcacgacgatttcctcgtcgatcaggacctggcaacgggacgttttcttgccacggtccaggacgcggaagcggtgcagcagcgacaccgattccaggtgcccaacgcggtcggacgtgaagcccatcgccgtcgcctgtaggcgcgacaggcattcctcggccttcgtgtaataccggccattgatcgaccagcccaggtcctggcaaagctcgtagaacgtgaaggtgatcggctcgccgataggggtgcgcttcgcgtactccaacacctgctgccacaccagttcgtcatcgtcggcccgcagctcgacgccggtgtaggtgatcttcacgtccttgttgacgtggaaaatgaccttgttttgcagcgcctcgcgcgggattttcttgttgcgcgtggtgaacagggcagagcgggccgtgtcgtttggcatcgctcgcatcgtgtccggccacggcgcaatatcgaacaaggaaagctgcatttccttgatctgctgcttcgtgtgtttcagcaacgcggcctgcttggcctcgctgacctgttttgccaggtcctcgccggcggtttttcgcttcttggtcgtcatagttcctcgcgtgtcgatggtcatcgacttcgccaaacctgccgcctcctgttcgagacgacgcgaacgctccacggcggccgatggcgcgggcagggcagggggagccagttgcacgctgtcgcgctcgatcttggccgtagcttgctggaccatcgagccgacggactggaaggtttcgcggggcgcacgcatgacggtgcggcttgcgatggtttcggcatcctcggcggaaaaccccgcgtcgatcagttcttgcctgtatgccttccggtcaaacgtccgattcattcaccctccttgcgggattgccccgactcacgccggggcaatgtgcccttattcctgatttgacccgcctggtgccttggtgtccagataatccaccttatcggcaatgaagtcggtcccgtagaccgtctggccgtccttctcgtacttggtattccgaatcttgccctgcacgaataccagctccgcgaagtcgctcttcttgatggagcgcatggggacgtgcttggcaatcacgcgcaccccccggccgttttagcggctaaaaaagtcatggctctgccctcgggcggaccacgcccatcatgaccttgccaagctcgtcctgcttctcttcgatcttcgccagcagggcgaggatcgtggcatcaccgaaccgcgccgtgcgcgggtcgtcggtgagccagagtttcagcaggccgcccaggcggcccaggtcgccattgatgcgggccagctcgcggacgtgctcatagtccacgacgcccgtgattttgtagccctggccgacggccagcaggtaggcctacaggctcatgccggccgccgccgccttttcctcaatcgctcttcgttcgtctggaaggcagtacaccttgataggtgggctgcccttcctggttggcttggtttcatcagccatccgcttgccctcatctgttacgccggcggtagccggccagcctcgcagagcaggattcccgttgagcaccgccaggtgcgaataagggacagtgaagaaggaacacccgctcgcgggtgggcctacttcacctatcctgcccggctgacgccgttggatacaccaaggaaagtctacacgaaccctttggcaaaatcctgtatatcgtgcgaaaaaggatggatataccgaaaaaatcgctataatgaccccgaagcagggttatgcagcggaaaagatccgtc

SEQ ID NO: 50 - DNA, 7219 bp, Artificial Sequence
  pAWP89S-Po-dTomato-RBS(MmoX)
gaccctttccgacgctcaccgggctggttgccctcgccgctgggctggcggccgtctatggccctgcaaacgcgccagaaacgccgtcgaagccgtgtgcgagacaccgcggccgccggcgttgtggatacctcgcggaaaacttggccctcactgacagatgaggggcggacgttgacacttgaggggccgactcacccggcgcggcgttgacagatgaggggcaggctcgatttcggccggcgacgtggagctggccagcctcgcaaatcggcgaaaacgcctgattttacgcgagtttcccacagatgatgtggacaagcctggggataagtgccctgcggtattgacacttgaggggcgcgactactgacagatgaggggcgcgatccttgacacttgaggggcagagtgctgacagatgaggggcgcacctattgacatttgaggggctgtccacaggcagaaaatccagcatttgcaagggtttccgcccgtttttcggccaccgctaacctgtcttttaacctgcttttaaaccaatatttataaaccttgtttttaaccagggctgcgccctgtgcgcgtgaccgcgcacgccgaaggggggtgcccccccttctcgaaccctcccggcccgctaacgcgggcctcccatccccccaggggctgcgcccctcggccgcgaacggcctcaccccaaaaatggcagccaagctgacccgctagggacgtgaagtcgattccttcgatggttagcaatcaaagactcagagtgctgtctggagcgtgaatctaacggtacgtatctcgattgctcggtcgctattcgcactctgcgaaagttcgtaccgctcattcactaggttgcgaaatcagagattttgagacacaaatttaaatcgtaattattggggacccctggattctcaccaataaaaaacgcccggcggcaaccgagcgttctgaacaaatccagatggagttctgaggtcattactggatctatcaacaggagtccaagactagtagcggataacaatttcacacaggattagccttcgatgccgattttcttcagccgataggccagtgccggtcggcttaggccgagcaagcgcgcggcaccggagacgttttggttggcctgttgcatggctttgcgcatcaggctttcctcgatctcgtcgaggctcaggccgctgctcaacaactggctgatccaactgccctggccattgcctggctgaatcagcacgccgtccgacgacacccgctcgctggcggtctgcggctcttccggcgcccgtgggaacagcgcctgcacgctgatgctttcgttcggatcggtgaggatgatgccgcgctcgatgacgttctccagctcacggatattgcccggccaactgtaatgcaggcaggcctccagggctttgtctgaaaggccgagggttctcttgccgtactcctggtggaagcgctgaaggaagtgctcaaccagcagtggaatgtcctcgcggcgttcgcgcaacgccgggatcgccaccgggaaaacgttcagccggtagtacaggtcggcgcgaaaacgcccggccttgaccgcttcggccaggtcctcgtgggtggctgcgataacccttacgtcgatcttgcgcgtgcggttgtcgccaactcgctccagctcgccttcttgcagcacgcgcagcagactggcctgagcgcgcgggctgagttcgatcacctcgtcaaggaagatggtgcccttgtcggcccgctcgaagcggcccatgcgtgactgggtggcgccggtgaaggcgcctttttccacgccgaacaattcggactcgatcaggtccggcgggatcgccgcacagttcaccgcgacaaagggctcggcggcgcgtttgctgcgcaggtgcacgctacgcgcgatgacctccttgccgaccccggtctcgccaagcagcagcaccgagactttgccctgtgcggccttgtccatcatattgcgcacggtctggtaggccggggtctgaccgatgccgtagtactggccttcctgtttgtcgaggttggtacgcagcgacaccagttgcgattgcaactcgtagagttcctcgatgatggggtcgttcttgaaatactgtttgaagctggcaacgtcgtcccactcttcggccggcttgccaatgacccggcacttgtcgccgccgcagccgcggcagctgacttccttgaagatgatttcccggcccatgaacgccgaggaataggcgcaggcgtagccgagcagagtccagcacaccgggtcttgcatctgccccaggtcggtctggcagatttccacctcgaaggagtcgatccactccatctcggcatagaagcgcccgcattccttgtcgatatcgacctcggtggggcggaccttgaccagacccttgagcgaatgcagctgcgggccggcgaggaacatgtcgtactcgctggcattcggtctaagcttcctggccagttcggcatccttcaggccggactggtaaccctggcgcaggaagaagcccttggcgcgttcgatgcccagggtattgaccatttcccggcgaaagctggccattgctgaaacctgcagcaacagcatgcgttgttcgccaagccagatcttgccttccgtgctctggaagtggatcaggttggtcaggtccttgaaatcggagtgctggatttcaggcttgtacttgatcggcatgtaagcgaggcccctatttatttttagatggggaaatcagggtcgccgctatagcgcaaggcaggcggcgattccagatggggtcatggggaaaatcggcagttttttcacctgcgccagctccccatagccgacctcagtatctggcaaaagtcaaccaaatgatcaatcgacggcagtgactttagtgctagagatcagccttcagctgcgccatgagcatttgctcaagcggccttgggcaattgatcaaatgcttaaaaagcctgcgcaagcgcggcttaatttcgctcgctccgatcattctaaaaattagaaacacattgaaaaacaataccttgaagtcggttttcagaccttggcacagctgttgcactttgtcctgcgcaatccgccaacctggagatctagacatcattcatagaatgtgttacggaggaaacaagtaatggtgagcaagggcgaggaggtcatcaaagagttcatgcgcttcaaggtgcgcatggagggctccatgaacggccacgagttcgagatcgagggcgagggcgagggccgcccctacgagggcacccagaccgccaagctgaaggtgaccaagggcggccccctgcccttcgcctgggacatcctgtccccccagttcatgtacggctccaaggcgtacgtgaagcaccccgccgacatccccgattacaagaagctgtccttccccgagggcttcaagtgggagcgcgtgatgaacttcgaggacggcggtctggtgaccgtgacccaggactcctccctgcaggacggcacgctgatctacaaggtgaagatgcgcggcaccaacttcccccccgacggccccgtaatgcagaagaagaccatgggctgggaggcctccaccgagcgcctgtacccccgcgacggcgtgctgaagggcgagatccaccaggccctgaagctgaaggacggcggccactacctggtggagttcaagaccatctacatggccaagaagcccgtgcaactgcccggctactactacgtggacaccaagctggacatcacctcccacaacgaggactacaccatcgtggaacagtacgagcgctccgagggccgccaccacctgttcctgtacggcatggacgagctgtacaagtagattgtcgggaagatgcgtgatctgatccttccactcagcaaaagttcgatttattcaacaaagccgccgtcccgtcaagtcagcgtaatgctctgccagtgttacaaccaattaaccaattctgattagaaaaactcatcgagcatcaaatgaaactgcaatttattcatatcaggattatcaataccatatttttgaaaaagccgtttctgtaatgaaggagaaaactcaccgaggcagttccataggatggcaagatcctggtatcggtctgcgattccgactcgtccaacatcaatacaacctattaatttcccctcgtcaaaaataaggttatcaagtgagaaatcaccatgagtgacgactgaatccggtgagaatggcaaaagcttatgcatttctttccagacttgttcaacaggccagccattacgctcgtcatcaaaatcactcgcatcaaccaaaccgttattcattcgtgattgcgcctgagcgagacgaaatacgcgatcgctgttaaaaggacaattacaaacaggaatcgaatgcaaccggcgcaggaacactgccagcgcatcaacaatattttcacctgaatcaggatattcttctaatacctggaatgctgttttcccggggatcgcagtggtgagtaaccatgcatcatcaggagtacggataaaatgcttgatggtcggaagaggcataaattccgtcagccagtttagtctgaccatctcatctgtaacatcattggcaacgctacctttgccatgtttcagaaacaactctggcgcatcgggcttcccatacaatcgatagattgtcgcacctgattgcccgacattatcgcgagcccatttatacccatataaatcagcatccatgttggaatttaatcgcggcctcgagcaagacgtttcccgttgaatatggctcataacaccccttgtattactgtttatgtaagcagacagttttattgttcatgatgatatatttttatcttgtgcaatgtaacatcagagattttgagacacaacgtggctttcgacttccggcaagctatacgcgccctagaattgtcaattttaatcctctgtttatcggcagttcgtagagcgcgccgtgcgtcccgagcgatactgagcgaagcaagtgcgtcgagcagtgcccgcttgttcctgaaatgccagtaaagcgctggctgctgaacccccagccggaactgaccccacaaggccctagcgtttgcaatgcaccaggtcatcattgacccaggcgtgttccaccaggccgctgcctcgcaactcttcgcaggcttcgccgacctgctcgcgccacttcttcacgcgggtggaatccgatccgcacatgaggcggaaggtttccagcttgagcgggtacggctcccggtgcgagctgaaatagtcgaacatccgtcgggccgtcggcgacagcttgcggtacttctcccatatgaatttcgtgtagtggtcgccagcaaacagcacgacgatttcctcgtcgatcaggacctggcaacgggacgttttcttgccacggtccaggacgcggaagcggtgcagcagcgacaccgattccaggtgcccaacgcggtcggacgtgaagcccatcgccgtcgcctgtaggcgcgacaggcattcctcggccttcgtgtaataccggccattgatcgaccagcccaggtcctggcaaagctcgtagaacgtgaaggtgatcggctcgccgataggggtgcgcttcgcgtactccaacacctgctgccacaccagttcgtcatcgtcggcccgcagctcgacgccggtgtaggtgatcttcacgtccttgttgacgtggaaaatgaccttgttttgcagcgcctcgcgcgggattttcttgttgcgcgtggtgaacagggcagagcgggccgtgtcgtttggcatcgctcgcatcgtgtccggccacggcgcaatatcgaacaaggaaagctgcatttccttgatctgctgcttcgtgtgtttcagcaacgcggcctgcttggcctcgctgacctgttttgccaggtcctcgccggcggtttttcgcttcttggtcgtcatagttcctcgcgtgtcgatggtcatcgacttcgccaaacctgccgcctcctgttcgagacgacgcgaacgctccacggcggccgatggcgcgggcagggcagggggagccagttgcacgctgtcgcgctcgatcttggccgtagcttgctggaccatcgagccgacggactggaaggtttcgcggggcgcacgcatgacggtgcggcttgcgatggtttcggcatcctcggcggaaaaccccgcgtcgatcagttcttgcctgtatgccttccggtcaaacgtccgattcattcaccctccttgcgggattgccccgactcacgccggggcaatgtgcccttattcctgatttgacccgcctggtgccttggtgtccagataatccaccttatcggcaatgaagtcggtcccgtagaccgtctggccgtccttctcgtacttggtattccgaatcttgccctgcacgaataccagctccgcgaagtcgctcttcttgatggagcgcatggggacgtgcttggcaatcacgcgcaccccccggccgttttagcggctaaaaaagtcatggctctgccctcgggcggaccacgcccatcatgaccttgccaagctcgtcctgcttctcttcgatcttcgccagcagggcgaggatcgtggcatcaccgaaccgcgccgtgcgcgggtcgtcggtgagccagagtttcagcaggccgcccaggcggcccaggtcgccattgatgcgggccagctcgcggacgtgctcatagtccacgacgcccgtgattttgtagccctggccgacggccagcaggtaggcctacaggctcatgccggccgccgccgccttttcctcaatcgctcttcgttcgtctggaaggcagtacaccttgataggtgggctgcccttcctggttggcttggtttcatcagccatccgcttgccctcatctgttacgccggcggtagccggccagcctcgcagagcaggattcccgttgagcaccgccaggtgcgaataagggacagtgaagaaggaacacccgctcgcgggtgggcctacttcacctatcctgcccggctgacgccgttggatacaccaaggaaagtctacacgaaccctttggcaaaatcctgtatatcgtgcgaaaaaggatggatataccgaaaaaatcgctataatgaccccgaagcagggttatgcagcggaaaagatccgtc

SEQ ID NO: 51 - DNA, 7219 bp, Artificial Sequence
  pAWP89S-Po-dTomato-RBS(MmoY)
gaccctttccgacgctcaccgggctggttgccctcgccgctgggctggcggccgtctatggccctgcaaacgcgccagaaacgccgtcgaagccgtgtgcgagacaccgcggccgccggcgttgtggatacctcgcggaaaacttggccctcactgacagatgaggggcggacgttgacacttgaggggccgactcacccggcgcggcgttgacagatgaggggcaggctcgatttcggccggcgacgtggagctggccagcctcgcaaatcggcgaaaacgcctgattttacgcgagtttcccacagatgatgtggacaagcctggggataagtgccctgcggtattgacacttgaggggcgcgactactgacagatgaggggcgcgatccttgacacttgaggggcagagtgctgacagatgaggggcgcacctattgacatttgaggggctgtccacaggcagaaaatccagcatttgcaagggtttccgcccgtttttcggccaccgctaacctgtcttttaacctgcttttaaaccaatatttataaaccttgtttttaaccagggctgcgccctgtgcgcgtgaccgcgcacgccgaaggggggtgcccccccttctcgaaccctcccggcccgctaacgcgggcctcccatccccccaggggctgcgcccctcggccgcgaacggcctcaccccaaaaatggcagccaagctgacccgctagggacgtgaagtcgattccttcgatggttagcaatcaaagactcagagtgctgtctggagcgtgaatctaacggtacgtatctcgattgctcggtcgctattcgcactctgcgaaagttcgtaccgctcattcactaggttgcgaaatcagagattttgagacacaaatttaaatcgtaattattggggacccctggattctcaccaataaaaaacgcccggcggcaaccgagcgttctgaacaaatccagatggagttctgaggtcattactggatctatcaacaggagtccaagactagtagcggataacaatttcacacaggattagccttcgatgccgattttcttcagccgataggccagtgccggtcggcttaggccgagcaagcgcgcggcaccggagacgttttggttggcctgttgcatggctttgcgcatcaggctttcctcgatctcgtcgaggctcaggccgctgctcaacaactggctgatccaactgccctggccattgcctggctgaatcagcacgccgtccgacgacacccgctcgctggcggtctgcggctcttccggcgcccgtgggaacagcgcctgcacgctgatgctttcgttcggatcggtgaggatgatgccgcgctcgatgacgttctccagctcacggatattgcccggccaactgtaatgcaggcaggcctccagggctttgtctgaaaggccgagggttctcttgccgtactcctggtggaagcgctgaaggaagtgctcaaccagcagtggaatgtcctcgcggcgttcgcgcaacgccgggatcgccaccgggaaaacgttcagccggtagtacaggtcggcgcgaaaacgcccggccttgaccgcttcggccaggtcctcgtgggtggctgcgataacccttacgtcgatcttgcgcgtgcggttgtcgccaactcgctccagctcgccttcttgcagcacgcgcagcagactggcctgagcgcgcgggctgagttcgatcacctcgtcaaggaagatggtgcccttgtcggcccgctcgaagcggcccatgcgtgactgggtggcgccggtgaaggcgcctttttccacgccgaacaattcggactcgatcaggtccggcgggatcgccgcacagttcaccgcgacaaagggctcggcggcgcgtttgctgcgcaggtgcacgctacgcgcgatgacctccttgccgaccccggtctcgccaagcagcagcaccgagactttgccctgtgcggccttgtccatcatattgcgcacggtctggtaggccggggtctgaccgatgccgtagtactggccttcctgtttgtcgaggttggtacgcagcgacaccagttgcgattgcaactcgtagagttcctcgatgatggggtcgttcttgaaatactgtttgaagctggcaacgtcgtcccactcttcggccggcttgccaatgacccggcacttgtcgccgccgcagccgcggcagctgacttccttgaagatgatttcccggcccatgaacgccgaggaataggcgcaggcgtagccgagcagagtccagcacaccgggtcttgcatctgccccaggtcggtctggcagatttccacctcgaaggagtcgatccactccatctcggcatagaagcgcccgcattccttgtcgatatcgacctcggtggggcggaccttgaccagacccttgagcgaatgcagctgcgggccggcgaggaacatgtcgtactcgctggcattcggtctaagcttcctggccagttcggcatccttcaggccggactggtaaccctggcgcaggaagaagcccttggcgcgttcgatgcccagggtattgaccatttcccggcgaaagctggccattgctgaaacctgcagcaacagcatgcgttgttcgccaagccagatcttgccttccgtgctctggaagtggatcaggttggtcaggtccttgaaatcggagtgctggatttcaggcttgtacttgatcggcatgtaagcgaggcccctatttatttttagatggggaaatcagggtcgccgctatagcgcaaggcaggcggcgattccagatggggtcatggggaaaatcggcagttttttcacctgcgccagctccccatagccgacctcagtatctggcaaaagtcaaccaaatgatcaatcgacggcagtgactttagtgctagagatcagccttcagctgcgccatgagcatttgctcaagcggccttgggcaattgatcaaatgcttaaaaagcctgcgcaagcgcggcttaatttcgctcgctccgatcattctaaaaattagaaacacattgaaaaacaataccttgaagtcggttttcagaccttggcacagctgttgcactttgtcctgcgcaatccgccaacctggagatctagacgttcgatcaacctcaaaccaaaaaggaacatcgatatggtgagcaagggcgaggaggtcatcaaagagttcatgcgcttcaaggtgcgcatggagggctccatgaacggccacgagttcgagatcgagggcgagggcgagggccgcccctacgagggcacccagaccgccaagctgaaggtgaccaagggcggccccctgcccttcgcctgggacatcctgtccccccagttcatgtacggctccaaggcgtacgtgaagcaccccgccgacatccccgattacaagaagctgtccttccccgagggcttcaagtgggagcgcgtgatgaacttcgaggacggcggtctggtgaccgtgacccaggactcctccctgcaggacggcacgctgatctacaaggtgaagatgcgcggcaccaacttcccccccgacggccccgtaatgcagaagaagaccatgggctgggaggcctccaccgagcgcctgtacccccgcgacggcgtgctgaagggcgagatccaccaggccctgaagctgaaggacggcggccactacctggtggagttcaagaccatctacatggccaagaagcccgtgcaactgcccggctactactacgtggacaccaagctggacatcacctcccacaacgaggactacaccatcgtggaacagtacgagcgctccgagggccgccaccacctgttcctgtacggcatggacgagctgtacaagtagattgtcgggaagatgcgtgatctgatccttccactcagcaaaagttcgatttattcaacaaagccgccgtcccgtcaagtcagcgtaatgctctgccagtgttacaaccaattaaccaattctgattagaaaaactcatcgagcatcaaatgaaactgcaatttattcatatcaggattatcaataccatatttttgaaaaagccgtttctgtaatgaaggagaaaactcaccgaggcagttccataggatggcaagatcctggtatcggtctgcgattccgactcgtccaacatcaatacaacctattaatttcccctcgtcaaaaataaggttatcaagtgagaaatcaccatgagtgacgactgaatccggtgagaatggcaaaagcttatgcatttctttccagacttgttcaacaggccagccattacgctcgtcatcaaaatcactcgcatcaaccaaaccgttattcattcgtgattgcgcctgagcgagacgaaatacgcgatcgctgttaaaaggacaattacaaacaggaatcgaatgcaaccggcgcaggaacactgccagcgcatcaacaatattttcacctgaatcaggatattcttctaatacctggaatgctgttttcccggggatcgcagtggtgagtaaccatgcatcatcaggagtacggataaaatgcttgatggtcggaagaggcataaattccgtcagccagtttagtctgaccatctcatctgtaacatcattggcaacgctacctttgccatgtttcagaaacaactctggcgcatcgggcttcccatacaatcgatagattgtcgcacctgattgcccgacattatcgcgagcccatttatacccatataaatcagcatccatgttggaatttaatcgcggcctcgagcaagacgtttcccgttgaatatggctcataacaccccttgtattactgtttatgtaagcagacagttttattgttcatgatgatatatttttatcttgtgcaatgtaacatcagagattttgagacacaacgtggctttcgacttccggcaagctatacgcgccctagaattgtcaattttaatcctctgtttatcggcagttcgtagagcgcgccgtgcgtcccgagcgatactgagcgaagcaagtgcgtcgagcagtgcccgcttgttcctgaaatgccagtaaagcgctggctgctgaacccccagccggaactgaccccacaaggccctagcgtttgcaatgcaccaggtcatcattgacccaggcgtgttccaccaggccgctgcctcgcaactcttcgcaggcttcgccgacctgctcgcgccacttcttcacgcgggtggaatccgatccgcacatgaggcggaaggtttccagcttgagcgggtacggctcccggtgcgagctgaaatagtcgaacatccgtcgggccgtcggcgacagcttgcggtacttctcccatatgaatttcgtgtagtggtcgccagcaaacagcacgacgatttcctcgtcgatcaggacctggcaacgggacgttttcttgccacggtccaggacgcggaagcggtgcagcagcgacaccgattccaggtgcccaacgcggtcggacgtgaagcccatcgccgtcgcctgtaggcgcgacaggcattcctcggccttcgtgtaataccggccattgatcgaccagcccaggtcctggcaaagctcgtagaacgtgaaggtgatcggctcgccgataggggtgcgcttcgcgtactccaacacctgctgccacaccagttcgtcatcgtcggcccgcagctcgacgccggtgtaggtgatcttcacgtccttgttgacgtggaaaatgaccttgttttgcagcgcctcgcgcgggattttcttgttgcgcgtggtgaacagggcagagcgggccgtgtcgtttggcatcgctcgcatcgtgtccggccacggcgcaatatcgaacaaggaaagctgcatttccttgatctgctgcttcgtgtgtttcagcaacgcggcctgcttggcctcgctgacctgttttgccaggtcctcgccggcggtttttcgcttcttggtcgtcatagttcctcgcgtgtcgatggtcatcgacttcgccaaacctgccgcctcctgttcgagacgacgcgaacgctccacggcggccgatggcgcgggcagggcagggggagccagttgcacgctgtcgcgctcgatcttggccgtagcttgctggaccatcgagccgacggactggaaggtttcgcggggcgcacgcatgacggtgcggcttgcgatggtttcggcatcctcggcggaaaaccccgcgtcgatcagttcttgcctgtatgccttccggtcaaacgtccgattcattcaccctccttgcgggattgccccgactcacgccggggcaatgtgcccttattcctgatttgacccgcctggtgccttggtgtccagataatccaccttatcggcaatgaagtcggtcccgtagaccgtctggccgtccttctcgtacttggtattccgaatcttgccctgcacgaataccagctccgcgaagtcgctcttcttgatggagcgcatggggacgtgcttggcaatcacgcgcaccccccggccgttttagcggctaaaaaagtcatggctctgccctcgggcggaccacgcccatcatgaccttgccaagctcgtcctgcttctcttcgatcttcgccagcagggcgaggatcgtggcatcaccgaaccgcgccgtgcgcgggtcgtcggtgagccagagtttcagcaggccgcccaggcggcccaggtcgccattgatgcgggccagctcgcggacgtgctcatagtccacgacgcccgtgattttgtagccctggccgacggccagcaggtaggcctacaggctcatgccggccgccgccgccttttcctcaatcgctcttcgttcgtctggaaggcagtacaccttgataggtgggctgcccttcctggttggcttggtttcatcagccatccgcttgccctcatctgttacgccggcggtagccggccagcctcgcagagcaggattcccgttgagcaccgccaggtgcgaataagggacagtgaagaaggaacacccgctcgcgggtgggcctacttcacctatcctgcccggctgacgccgttggatacaccaaggaaagtctacacgaaccctttggcaaaatcctgtatatcgtgcgaaaaaggatggatataccgaaaaaatcgctataatgaccccgaagcagggttatgcagcggaaaagatccgtc

SEQ ID NO: 52 - DNA, 7219 bp, Artificial Sequence
  pAWP89S-Po-dTomato-RBS(MmoZ)
gaccctttccgacgctcaccgggctggttgccctcgccgctgggctggcggccgtctatggccctgcaaacgcgccagaaacgccgtcgaagccgtgtgcgagacaccgcggccgccggcgttgtggatacctcgcggaaaacttggccctcactgacagatgaggggcggacgttgacacttgaggggccgactcacccggcgcggcgttgacagatgaggggcaggctcgatttcggccggcgacgtggagctggccagcctcgcaaatcggcgaaaacgcctgattttacgcgagtttcccacagatgatgtggacaagcctggggataagtgccctgcggtattgacacttgaggggcgcgactactgacagatgaggggcgcgatccttgacacttgaggggcagagtgctgacagatgaggggcgcacctattgacatttgaggggctgtccacaggcagaaaatccagcatttgcaagggtttccgcccgtttttcggccaccgctaacctgtcttttaacctgcttttaaaccaatatttataaaccttgtttttaaccagggctgcgccctgtgcgcgtgaccgcgcacgccgaaggggggtgcccccccttctcgaaccctcccggcccgctaacgcgggcctcccatccccccaggggctgcgcccctcggccgcgaacggcctcaccccaaaaatggcagccaagctgacccgctagggacgtgaagtcgattccttcgatggttagcaatcaaagactcagagtgctgtctggagcgtgaatctaacggtacgtatctcgattgctcggtcgctattcgcactctgcgaaagttcgtaccgctcattcactaggttgcgaaatcagagattttgagacacaaatttaaatcgtaattattggggacccctggattctcaccaataaaaaacgcccggcggcaaccgagcgttctgaacaaatccagatggagttctgaggtcattactggatctatcaacaggagtccaagactagtagcggataacaatttcacacaggattagccttcgatgccgattttcttcagccgataggccagtgccggtcggcttaggccgagcaagcgcgcggcaccggagacgttttggttggcctgttgcatggctttgcgcatcaggctttcctcgatctcgtcgaggctcaggccgctgctcaacaactggctgatccaactgccctggccattgcctggctgaatcagcacgccgtccgacgacacccgctcgctggcggtctgcggctcttccggcgcccgtgggaacagcgcctgcacgctgatgctttcgttcggatcggtgaggatgatgccgcgctcgatgacgttctccagctcacggatattgcccggccaactgtaatgcaggcaggcctccagggctttgtctgaaaggccgagggttctcttgccgtactcctggtggaagcgctgaaggaagtgctcaaccagcagtggaatgtcctcgcggcgttcgcgcaacgccgggatcgccaccgggaaaacgttcagccggtagtacaggtcggcgcgaaaacgcccggccttgaccgcttcggccaggtcctcgtgggtggctgcgataacccttacgtcgatcttgcgcgtgcggttgtcgccaactcgctccagctcgccttcttgcagcacgcgcagcagactggcctgagcgcgcgggctgagttcgatcacctcgtcaaggaagatggtgcccttgtcggcccgctcgaagcggcccatgcgtgactgggtggcgccggtgaaggcgcctttttccacgccgaacaattcggactcgatcaggtccggcgggatcgccgcacagttcaccgcgacaaagggctcggcggcgcgtttgctgcgcaggtgcacgctacgcgcgatgacctccttgccgaccccggtctcgccaagcagcagcaccgagactttgccctgtgcggccttgtccatcatattgcgcacggtctggtaggccggggtctgaccgatgccgtagtactggccttcctgtttgtcgaggttggtacgcagcgacaccagttgcgattgcaactcgtagagttcctcgatgatggggtcgttcttgaaatactgtttgaagctggcaacgtcgtcccactcttcggccggcttgccaatgacccggcacttgtcgccgccgcagccgcggcagctgacttccttgaagatgatttcccggcccatgaacgccgaggaataggcgcaggcgtagccgagcagagtccagcacaccgggtcttgcatctgccccaggtcggtctggcagatttccacctcgaaggagtcgatccactccatctcggcatagaagcgcccgcattccttgtcgatatcgacctcggtggggcggaccttgaccagacccttgagcgaatgcagctgcgggccggcgaggaacatgtcgtactcgctggcattcggtctaagcttcctggccagttcggcatccttcaggccggactggtaaccctggcgcaggaagaagcccttggcgcgttcgatgcccagggtattgaccatttcccggcgaaagctggccattgctgaaacctgcagcaacagcatgcgttgttcgccaagccagatcttgccttccgtgctctggaagtggatcaggttggtcaggtccttgaaatcggagtgctggatttcaggcttgtacttgatcggcatgtaagcgaggcccctatttatttttagatggggaaatcagggtcgccgctatagcgcaaggcaggcggcgattccagatggggtcatggggaaaatcggcagttttttcacctgcgccagctccccatagccgacctcagtatctggcaaaagtcaaccaaatgatcaatcgacggcagtgactttagtgctagagatcagccttcagctgcgccatgagcatttgctcaagcggccttgggcaattgatcaaatgcttaaaaagcctgcgcaagcgcggcttaatttcgctcgctccgatcattctaaaaattagaaacacattgaaaaacaataccttgaagtcggttttcagaccttggcacagctgttgcactttgtcctgcgcaatccgccaacctggagatctagatggacactttttcaacggcctgttaaggagaatgacatggtgagcaagggcgaggaggtcatcaaagagttcatgcgcttcaaggtgcgcatggagggctccatgaacggccacgagttcgagatcgagggcgagggcgagggccgcccctacgagggcacccagaccgccaagctgaaggtgaccaagggcggccccctgcccttcgcctgggacatcctgtccccccagttcatgtacggctccaaggcgtacgtgaagcaccccgccgacatccccgattacaagaagctgtccttccccgagggcttcaagtgggagcgcgtgatgaacttcgaggacggcggtctggtgaccgtgacccaggactcctccctgcaggacggcacgctgatctacaaggtgaagatgcgcggcaccaacttcccccccgacggccccgtaatgcagaagaagaccatgggctgggaggcctccaccgagcgcctgtacccccgcgacggcgtgctgaagggcgagatccaccaggccctgaagctgaaggacggcggccactacctggtggagttcaagaccatctacatggccaagaagcccgtgcaactgcccggctactactacgtggacaccaagctggacatcacctcccacaacgaggactacaccatcgtggaacagtacgagcgctccgagggccgccaccacctgttcctgtacggcatggacgagctgtacaagtagattgtcgggaagatgcgtgatctgatccttccactcagcaaaagttcgatttattcaacaaagccgccgtcccgtcaagtcagcgtaatgctctgccagtgttacaaccaattaaccaattctgattagaaaaactcatcgagcatcaaatgaaactgcaatttattcatatcaggattatcaataccatatttttgaaaaagccgtttctgtaatgaaggagaaaactcaccgaggcagttccataggatggcaagatcctggtatcggtctgcgattccgactcgtccaacatcaatacaacctattaatttcccctcgtcaaaaataaggttatcaagtgagaaatcaccatgagtgacgactgaatccggtgagaatggcaaaagcttatgcatttctttccagacttgttcaacaggccagccattacgctcgtcatcaaaatcactcgcatcaaccaaaccgttattcattcgtgattgcgcctgagcgagacgaaatacgcgatcgctgttaaaaggacaattacaaacaggaatcgaatgcaaccggcgcaggaacactgccagcgcatcaacaatattttcacctgaatcaggatattcttctaatacctggaatgctgttttcccggggatcgcagtggtgagtaaccatgcatcatcaggagtacggataaaatgcttgatggtcggaagaggcataaattccgtcagccagtttagtctgaccatctcatctgtaacatcattggcaacgctacctttgccatgtttcagaaacaactctggcgcatcgggcttcccatacaatcgatagattgtcgcacctgattgcccgacattatcgcgagcccatttatacccatataaatcagcatccatgttggaatttaatcgcggcctcgagcaagacgtttcccgttgaatatggctcataacaccccttgtattactgtttatgtaagcagacagttttattgttcatgatgatatatttttatcttgtgcaatgtaacatcagagattttgagacacaacgtggctttcgacttccggcaagctatacgcgccctagaattgtcaattttaatcctctgtttatcggcagttcgtagagcgcgccgtgcgtcccgagcgatactgagcgaagcaagtgcgtcgagcagtgcccgcttgttcctgaaatgccagtaaagcgctggctgctgaacccccagccggaactgaccccacaaggccctagcgtttgcaatgcaccaggtcatcattgacccaggcgtgttccaccaggccgctgcctcgcaactcttcgcaggcttcgccgacctgctcgcgccacttcttcacgcgggtggaatccgatccgcacatgaggcggaaggtttccagcttgagcgggtacggctcccggtgcgagctgaaatagtcgaacatccgtcgggccgtcggcgacagcttgcggtacttctcccatatgaatttcgtgtagtggtcgccagcaaacagcacgacgatttcctcgtcgatcaggacctggcaacgggacgttttcttgccacggtccaggacgcggaagcggtgcagcagcgacaccgattccaggtgcccaacgcggtcggacgtgaagcccatcgccgtcgcctgtaggcgcgacaggcattcctcggccttcgtgtaataccggccattgatcgaccagcccaggtcctggcaaagctcgtagaacgtgaaggtgatcggctcgccgataggggtgcgcttcgcgtactccaacacctgctgccacaccagttcgtcatcgtcggcccgcagctcgacgccggtgtaggtgatcttcacgtccttgttgacgtggaaaatgaccttgttttgcagcgcctcgcgcgggattttcttgttgcgcgtggtgaacagggcagagcgggccgtgtcgtttggcatcgctcgcatcgtgtccggccacggcgcaatatcgaacaaggaaagctgcatttccttgatctgctgcttcgtgtgtttcagcaacgcggcctgcttggcctcgctgacctgttttgccaggtcctcgccggcggtttttcgcttcttggtcgtcatagttcctcgcgtgtcgatggtcatcgacttcgccaaacctgccgcctcctgttcgagacgacgcgaacgctccacggcggccgatggcgcgggcagggcagggggagccagttgcacgctgtcgcgctcgatcttggccgtagcttgctggaccatcgagccgacggactggaaggtttcgcggggcgcacgcatgacggtgcggcttgcgatggtttcggcatcctcggcggaaaaccccgcgtcgatcagttcttgcctgtatgccttccggtcaaacgtccgattcattcaccctccttgcgggattgccccgactcacgccggggcaatgtgcccttattcctgatttgacccgcctggtgccttggtgtccagataatccaccttatcggcaatgaagtcggtcccgtagaccgtctggccgtccttctcgtacttggtattccgaatcttgccctgcacgaataccagctccgcgaagtcgctcttcttgatggagcgcatggggacgtgcttggcaatcacgcgcaccccccggccgttttagcggctaaaaaagtcatggctctgccctcgggcggaccacgcccatcatgaccttgccaagctcgtcctgcttctcttcgatcttcgccagcagggcgaggatcgtggcatcaccgaaccgcgccgtgcgcgggtcgtcggtgagccagagtttcagcaggccgcccaggcggcccaggtcgccattgatgcgggccagctcgcggacgtgctcatagtccacgacgcccgtgattttgtagccctggccgacggccagcaggtaggcctacaggctcatgccggccgccgccgccttttcctcaatcgctcttcgttcgtctggaaggcagtacaccttgataggtgggctgcccttcctggttggcttggtttcatcagccatccgcttgccctcatctgttacgccggcggtagccggccagcctcgcagagcaggattcccgttgagcaccgccaggtgcgaataagggacagtgaagaaggaacacccgctcgcgggtgggcctacttcacctatcctgcccggctgacgccgttggatacaccaaggaaagtctacacgaaccctttggcaaaatcctgtatatcgtgcgaaaaaggatggatataccgaaaaaatcgctataatgaccccgaagcagggttatgcagcggaaaagatccgtc

SEQ ID NO: 53 - DNA, 7219 bp, Artificial Sequence
  pAWP89S-Po-dTomato-RBS(PmoA1)
gaccctttccgacgctcaccgggctggttgccctcgccgctgggctggcggccgtctatggccctgcaaacgcgccagaaacgccgtcgaagccgtgtgcgagacaccgcggccgccggcgttgtggatacctcgcggaaaacttggccctcactgacagatgaggggcggacgttgacacttgaggggccgactcacccggcgcggcgttgacagatgaggggcaggctcgatttcggccggcgacgtggagctggccagcctcgcaaatcggcgaaaacgcctgattttacgcgagtttcccacagatgatgtggacaagcctggggataagtgccctgcggtattgacacttgaggggcgcgactactgacagatgaggggcgcgatccttgacacttgaggggcagagtgctgacagatgaggggcgcacctattgacatttgaggggctgtccacaggcagaaaatccagcatttgcaagggtttccgcccgtttttcggccaccgctaacctgtcttttaacctgcttttaaaccaatatttataaaccttgtttttaaccagggctgcgccctgtgcgcgtgaccgcgcacgccgaaggggggtgcccccccttctcgaaccctcccggcccgctaacgcgggcctcccatccccccaggggctgcgcccctcggccgcgaacggcctcaccccaaaaatggcagccaagctgacccgctagggacgtgaagtcgattccttcgatggttagcaatcaaagactcagagtgctgtctggagcgtgaatctaacggtacgtatctcgattgctcggtcgctattcgcactctgcgaaagttcgtaccgctcattcactaggttgcgaaatcagagattttgagacacaaatttaaatcgtaattattggggacccctggattctcaccaataaaaaacgcccggcggcaaccgagcgttctgaacaaatccagatggagttctgaggtcattactggatctatcaacaggagtccaagactagtagcggataacaatttcacacaggattagccttcgatgccgattttcttcagccgataggccagtgccggtcggcttaggccgagcaagcgcgcggcaccggagacgttttggttggcctgttgcatggctttgcgcatcaggctttcctcgatctcgtcgaggctcaggccgctgctcaacaactggctgatccaactgccctggccattgcctggctgaatcagcacgccgtccgacgacacccgctcgctggcggtctgcggctcttccggcgcccgtgggaacagcgcctgcacgctgatgctttcgttcggatcggtgaggatgatgccgcgctcgatgacgttctccagctcacggatattgcccggccaactgtaatgcaggcaggcctccagggctttgtctgaaaggccgagggttctcttgccgtactcctggtggaagcgctgaaggaagtgctcaaccagcagtggaatgtcctcgcggcgttcgcgcaacgccgggatcgccaccgggaaaacgttcagccggtagtacaggtcggcgcgaaaacgcccggccttgaccgcttcggccaggtcctcgtgggtggctgcgataacccttacgtcgatcttgcgcgtgcggttgtcgccaactcgctccagctcgccttcttgcagcacgcgcagcagactggcctgagcgcgcgggctgagttcgatcacctcgtcaaggaagatggtgcccttgtcggcccgctcgaagcggcccatgcgtgactgggtggcgccggtgaaggcgcctttttccacgccgaacaattcggactcgatcaggtccggcgggatcgccgcacagttcaccgcgacaaagggctcggcggcgcgtttgctgcgcaggtgcacgctacgcgcgatgacctccttgccgaccccggtctcgccaagcagcagcaccgagactttgccctgtgcggccttgtccatcatattgcgcacggtctggtaggccggggtctgaccgatgccgtagtactggccttcctgtttgtcgaggttggtacgcagcgacaccagttgcgattgcaactcgtagagttcctcgatgatggggtcgttcttgaaatactgtttgaagctggcaacgtcgtcccactcttcggccggcttgccaatgacccggcacttgtcgccgccgcagccgcggcagctgacttccttgaagatgatttcccggcccatgaacgccgaggaataggcgcaggcgtagccgagcagagtccagcacaccgggtcttgcatctgccccaggtcggtctggcagatttccacctcgaaggagtcgatccactccatctcggcatagaagcgcccgcattccttgtcgatatcgacctcggtggggcggaccttgaccagacccttgagcgaatgcagctgcgggccggcgaggaacatgtcgtactcgctggcattcggtctaagcttcctggccagttcggcatccttcaggccggactggtaaccctggcgcaggaagaagcccttggcgcgttcgatgcccagggtattgaccatttcccggcgaaagctggccattgctgaaacctgcagcaacagcatgcgttgttcgccaagccagatcttgccttccgtgctctggaagtggatcaggttggtcaggtccttgaaatcggagtgctggatttcaggcttgtacttgatcggcatgtaagcgaggcccctatttatttttagatggggaaatcagggtcgccgctatagcgcaaggcaggcggcgattccagatggggtcatggggaaaatcggcagttttttcacctgcgccagctccccatagccgacctcagtatctggcaaaagtcaaccaaatgatcaatcgacggcagtgactttagtgctagagatcagccttcagctgcgccatgagcatttgctcaagcggccttgggcaattgatcaaatgcttaaaaagcctgcgcaagcgcggcttaatttcgctcgctccgatcattctaaaaattagaaacacattgaaaaacaataccttgaagtcggttttcagaccttggcacagctgttgcactttgtcctgcgcaatccgccaacctggagatctagagaaaataagaaaacgacaaatttggaggtaactttaatggtgagcaagggcgaggaggtcatcaaagagttcatgcgcttcaaggtgcgcatggagggctccatgaacggccacgagttcgagatcgagggcgagggcgagggccgcccctacgagggcacccagaccgccaagctgaaggtgaccaagggcggccccctgcccttcgcctgggacatcctgtccccccagttcatgtacggctccaaggcgtacgtgaagcaccccgccgacatccccgattacaagaagctgtccttccccgagggcttcaagtgggagcgcgtgatgaacttcgaggacggcggtctggtgaccgtgacccaggactcctccctgcaggacggcacgctgatctacaaggtgaagatgcgcggcaccaacttcccccccgacggccccgtaatgcagaagaagaccatgggctgggaggcctccaccgagcgcctgtacccccgcgacggcgtgctgaagggcgagatccaccaggccctgaagctgaaggacggcggccactacctggtggagttcaagaccatctacatggccaagaagcccgtgcaactgcccggctactactacgtggacaccaagctggacatcacctcccacaacgaggactacaccatcgtggaacagtacgagcgctccgagggccgccaccacctgttcctgtacggcatggacgagctgtacaagtagattgtcgggaagatgcgtgatctgatccttccactcagcaaaagttcgatttattcaacaaagccgccgtcccgtcaagtcagcgtaatgctctgccagtgttacaaccaattaaccaattctgattagaaaaactcatcgagcatcaaatgaaactgcaatttattcatatcaggattatcaataccatatttttgaaaaagccgtttctgtaatgaaggagaaaactcaccgaggcagttccataggatggcaagatcctggtatcggtctgcgattccgactcgtccaacatcaatacaacctattaatttcccctcgtcaaaaataaggttatcaagtgagaaatcaccatgagtgacgactgaatccggtgagaatggcaaaagcttatgcatttctttccagacttgttcaacaggccagccattacgctcgtcatcaaaatcactcgcatcaaccaaaccgttattcattcgtgattgcgcctgagcgagacgaaatacgcgatcgctgttaaaaggacaattacaaacaggaatcgaatgcaaccggcgcaggaacactgccagcgcatcaacaatattttcacctgaatcaggatattcttctaatacctggaatgctgttttcccggggatcgcagtggtgagtaaccatgcatcatcaggagtacggataaaatgcttgatggtcggaagaggcataaattccgtcagccagtttagtctgaccatctcatctgtaacatcattggcaacgctacctttgccatgtttcagaaacaactctggcgcatcgggcttcccatacaatcgatagattgtcgcacctgattgcccgacattatcgcgagcccatttatacccatataaatcagcatccatgttggaatttaatcgcggcctcgagcaagacgtttcccgttgaatatggctcataacaccccttgtattactgtttatgtaagcagacagttttattgttcatgatgatatatttttatcttgtgcaatgtaacatcagagattttgagacacaacgtggctttcgacttccggcaagctatacgcgccctagaattgtcaattttaatcctctgtttatcggcagttcgtagagcgcgccgtgcgtcccgagcgatactgagcgaagcaagtgcgtcgagcagtgcccgcttgttcctgaaatgccagtaaagcgctggctgctgaacccccagccggaactgaccccacaaggccctagcgtttgcaatgcaccaggtcatcattgacccaggcgtgttccaccaggccgctgcctcgcaactcttcgcaggcttcgccgacctgctcgcgccacttcttcacgcgggtggaatccgatccgcacatgaggcggaaggtttccagcttgagcgggtacggctcccggtgcgagctgaaatagtcgaacatccgtcgggccgtcggcgacagcttgcggtacttctcccatatgaatttcgtgtagtggtcgccagcaaacagcacgacgatttcctcgtcgatcaggacctggcaacgggacgttttcttgccacggtccaggacgcggaagcggtgcagcagcgacaccgattccaggtgcccaacgcggtcggacgtgaagcccatcgccgtcgcctgtaggcgcgacaggcattcctcggccttcgtgtaataccggccattgatcgaccagcccaggtcctggcaaagctcgtagaacgtgaaggtgatcggctcgccgataggggtgcgcttcgcgtactccaacacctgctgccacaccagttcgtcatcgtcggcccgcagctcgacgccggtgtaggtgatcttcacgtccttgttgacgtggaaaatgaccttgttttgcagcgcctcgcgcgggattttcttgttgcgcgtggtgaacagggcagagcgggccgtgtcgtttggcatcgctcgcatcgtgtccggccacggcgcaatatcgaacaaggaaagctgcatttccttgatctgctgcttcgtgtgtttcagcaacgcggcctgcttggcctcgctgacctgttttgccaggtcctcgccggcggtttttcgcttcttggtcgtcatagttcctcgcgtgtcgatggtcatcgacttcgccaaacctgccgcctcctgttcgagacgacgcgaacgctccacggcggccgatggcgcgggcagggcagggggagccagttgcacgctgtcgcgctcgatcttggccgtagcttgctggaccatcgagccgacggactggaaggtttcgcggggcgcacgcatgacggtgcggcttgcgatggtttcggcatcctcggcggaaaaccccgcgtcgatcagttcttgcctgtatgccttccggtcaaacgtccgattcattcaccctccttgcgggattgccccgactcacgccggggcaatgtgcccttattcctgatttgacccgcctggtgccttggtgtccagataatccaccttatcggcaatgaagtcggtcccgtagaccgtctggccgtccttctcgtacttggtattccgaatcttgccctgcacgaataccagctccgcgaagtcgctcttcttgatggagcgcatggggacgtgcttggcaatcacgcgcaccccccggccgttttagcggctaaaaaagtcatggctctgccctcgggcggaccacgcccatcatgaccttgccaagctcgtcctgcttctcttcgatcttcgccagcagggcgaggatcgtggcatcaccgaaccgcgccgtgcgcgggtcgtcggtgagccagagtttcagcaggccgcccaggcggcccaggtcgccattgatgcgggccagctcgcggacgtgctcatagtccacgacgcccgtgattttgtagccctggccgacggccagcaggtaggcctacaggctcatgccggccgccgccgccttttcctcaatcgctcttcgttcgtctggaaggcagtacaccttgataggtgggctgcccttcctggttggcttggtttcatcagccatccgcttgccctcatctgttacgccggcggtagccggccagcctcgcagagcaggattcccgttgagcaccgccaggtgcgaataagggacagtgaagaaggaacacccgctcgcgggtgggcctacttcacctatcctgcccggctgacgccgttggatacaccaaggaaagtctacacgaaccctttggcaaaatcctgtatatcgtgcgaaaaaggatggatataccgaaaaaatcgctataatgaccccgaagcagggttatgcagcggaaaagatccgtc

SEQ ID NO: 54 - DNA, 7219 bp, Artificial Sequence
  pAWP89S-Po-dTomato-RBS(PmoB1)
gaccctttccgacgctcaccgggctggttgccctcgccgctgggctggcggccgtctatggccctgcaaacgcgccagaaacgccgtcgaagccgtgtgcgagacaccgcggccgccggcgttgtggatacctcgcggaaaacttggccctcactgacagatgaggggcggacgttgacacttgaggggccgactcacccggcgcggcgttgacagatgaggggcaggctcgatttcggccggcgacgtggagctggccagcctcgcaaatcggcgaaaacgcctgattttacgcgagtttcccacagatgatgtggacaagcctggggataagtgccctgcggtattgacacttgaggggcgcgactactgacagatgaggggcgcgatccttgacacttgaggggcagagtgctgacagatgaggggcgcacctattgacatttgaggggctgtccacaggcagaaaatccagcatttgcaagggtttccgcccgtttttcggccaccgctaacctgtcttttaacctgcttttaaaccaatatttataaaccttgtttttaaccagggctgcgccctgtgcgcgtgaccgcgcacgccgaaggggggtgcccccccttctcgaaccctcccggcccgctaacgcgggcctcccatccccccaggggctgcgcccctcggccgcgaacggcctcaccccaaaaatggcagccaagctgacccgctagggacgtgaagtcgattccttcgatggttagcaatcaaagactcagagtgctgtctggagcgtgaatctaacggtacgtatctcgattgctcggtcgctattcgcactctgcgaaagttcgtaccgctcattcactaggttgcgaaatcagagattttgagacacaaatttaaatcgtaattattggggacccctggattctcaccaataaaaaacgcccggcggcaaccgagcgttctgaacaaatccagatggagttctgaggtcattactggatctatcaacaggagtccaagactagtagcggataacaatttcacacaggattagccttcgatgccgattttcttcagccgataggccagtgccggtcggcttaggccgagcaagcgcgcggcaccggagacgttttggttggcctgttgcatggctttgcgcatcaggctttcctcgatctcgtcgaggctcaggccgctgctcaacaactggctgatccaactgccctggccattgcctggctgaatcagcacgccgtccgacgacacccgctcgctggcggtctgcggctcttccggcgcccgtgggaacagcgcctgcacgctgatgctttcgttcggatcggtgaggatgatgccgcgctcgatgacgttctccagctcacggatattgcccggccaactgtaatgcaggcaggcctccagggctttgtctgaaaggccgagggttctcttgccgtactcctggtggaagcgctgaaggaagtgctcaaccagcagtggaatgtcctcgcggcgttcgcgcaacgccgggatcgccaccgggaaaacgttcagccggtagtacaggtcggcgcgaaaacgcccggccttgaccgcttcggccaggtcctcgtgggtggctgcgataacccttacgtcgatcttgcgcgtgcggttgtcgccaactcgctccagctcgccttcttgcagcacgcgcagcagactggcctgagcgcgcgggctgagttcgatcacctcgtcaaggaagatggtgcccttgtcggcccgctcgaagcggcccatgcgtgactgggtggcgccggtgaaggcgcctttttccacgccgaacaattcggactcgatcaggtccggcgggatcgccgcacagttcaccgcgacaaagggctcggcggcgcgtttgctgcgcaggtgcacgctacgcgcgatgacctccttgccgaccccggtctcgccaagcagcagcaccgagactttgccctgtgcggccttgtccatcatattgcgcacggtctggtaggccggggtctgaccgatgccgtagtactggccttcctgtttgtcgaggttggtacgcagcgacaccagttgcgattgcaactcgtagagttcctcgatgatggggtcgttcttgaaatactgtttgaagctggcaacgtcgtcccactcttcggccggcttgccaatgacccggcacttgtcgccgccgcagccgcggcagctgacttccttgaagatgatttcccggcccatgaacgccgaggaataggcgcaggcgtagccgagcagagtccagcacaccgggtcttgcatctgccccaggtcggtctggcagatttccacctcgaaggagtcgatccactccatctcggcatagaagcgcccgcattccttgtcgatatcgacctcggtggggcggaccttgaccagacccttgagcgaatgcagctgcgggccggcgaggaacatgtcgtactcgctggcattcggtctaagcttcctggccagttcggcatccttcaggccggactggtaaccctggcgcaggaagaagcccttggcgcgttcgatgcccagggtattgaccatttcccggcgaaagctggccattgctgaaacctgcagcaacagcatgcgttgttcgccaagccagatcttgccttccgtgctctggaagtggatcaggttggtcaggtccttgaaatcggagtgctggatttcaggcttgtacttgatcggcatgtaagcgaggcccctatttatttttagatggggaaatcagggtcgccgctatagcgcaaggcaggcggcgattccagatggggtcatggggaaaatcggcagttttttcacctgcgccagctccccatagccgacctcagtatctggcaaaagtcaaccaaatgatcaatcgacggcagtgactttagtgctagagatcagccttcagctgcgccatgagcatttgctcaagcggccttgggcaattgatcaaatgcttaaaaagcctgcgcaagcgcggcttaatttcgctcgctccgatcattctaaaaattagaaacacattgaaaaacaataccttgaagtcggttttcagaccttggcacagctgttgcactttgtcctgcgcaatccgccaacctggagatctagagtgacccaacagcaagaactcgaaagaggagagatcatggtgagcaagggcgaggaggtcatcaaagagttcatgcgcttcaaggtgcgcatggagggctccatgaacggccacgagttcgagatcgagggcgagggcgagggccgcccctacgagggcacccagaccgccaagctgaaggtgaccaagggcggccccctgcccttcgcctgggacatcctgtccccccagttcatgtacggctccaaggcgtacgtgaagcaccccgccgacatccccgattacaagaagctgtccttccccgagggcttcaagtgggagcgcgtgatgaacttcgaggacggcggtctggtgaccgtgacccaggactcctccctgcaggacggcacgctgatctacaaggtgaagatgcgcggcaccaacttcccccccgacggccccgtaatgcagaagaagaccatgggctgggaggcctccaccgagcgcctgtacccccgcgacggcgtgctgaagggcgagatccaccaggccctgaagctgaaggacggcggccactacctggtggagttcaagaccatctacatggccaagaagcccgtgcaactgcccggctactactacgtggacaccaagctggacatcacctcccacaacgaggactacaccatcgtggaacagtacgagcgctccgagggccgccaccacctgttcctgtacggcatggacgagctgtacaagtagattgtcgggaagatgcgtgatctgatccttccactcagcaaaagttcgatttattcaacaaagccgccgtcccgtcaagtcagcgtaatgctctgccagtgttacaaccaattaaccaattctgattagaaaaactcatcgagcatcaaatgaaactgcaatttattcatatcaggattatcaataccatatttttgaaaaagccgtttctgtaatgaaggagaaaactcaccgaggcagttccataggatggcaagatcctggtatcggtctgcgattccgactcgtccaacatcaatacaacctattaatttcccctcgtcaaaaataaggttatcaagtgagaaatcaccatgagtgacgactgaatccggtgagaatggcaaaagcttatgcatttctttccagacttgttcaacaggccagccattacgctcgtcatcaaaatcactcgcatcaaccaaaccgttattcattcgtgattgcgcctgagcgagacgaaatacgcgatcgctgttaaaaggacaattacaaacaggaatcgaatgcaaccggcgcaggaacactgccagcgcatcaacaatattttcacctgaatcaggatattcttctaatacctggaatgctgttttcccggggatcgcagtggtgagtaaccatgcatcatcaggagtacggataaaatgcttgatggtcggaagaggcataaattccgtcagccagtttagtctgaccatctcatctgtaacatcattggcaacgctacctttgccatgtttcagaaacaactctggcgcatcgggcttcccatacaatcgatagattgtcgcacctgattgcccgacattatcgcgagcccatttatacccatataaatcagcatccatgttggaatttaatcgcggcctcgagcaagacgtttcccgttgaatatggctcataacaccccttgtattactgtttatgtaagcagacagttttattgttcatgatgatatatttttatcttgtgcaatgtaacatcagagattttgagacacaacgtggctttcgacttccggcaagctatacgcgccctagaattgtcaattttaatcctctgtttatcggcagttcgtagagcgcgccgtgcgtcccgagcgatactgagcgaagcaagtgcgtcgagcagtgcccgcttgttcctgaaatgccagtaaagcgctggctgctgaacccccagccggaactgaccccacaaggccctagcgtttgcaatgcaccaggtcatcattgacccaggcgtgttccaccaggccgctgcctcgcaactcttcgcaggcttcgccgacctgctcgcgccacttcttcacgcgggtggaatccgatccgcacatgaggcggaaggtttccagcttgagcgggtacggctcccggtgcgagctgaaatagtcgaacatccgtcgggccgtcggcgacagcttgcggtacttctcccatatgaatttcgtgtagtggtcgccagcaaacagcacgacgatttcctcgtcgatcaggacctggcaacgggacgttttcttgccacggtccaggacgcggaagcggtgcagcagcgacaccgattccaggtgcccaacgcggtcggacgtgaagcccatcgccgtcgcctgtaggcgcgacaggcattcctcggccttcgtgtaataccggccattgatcgaccagcccaggtcctggcaaagctcgtagaacgtgaaggtgatcggctcgccgataggggtgcgcttcgcgtactccaacacctgctgccacaccagttcgtcatcgtcggcccgcagctcgacgccggtgtaggtgatcttcacgtccttgttgacgtggaaaatgaccttgttttgcagcgcctcgcgcgggattttcttgttgcgcgtggtgaacagggcagagcgggccgtgtcgtttggcatcgctcgcatcgtgtccggccacggcgcaatatcgaacaaggaaagctgcatttccttgatctgctgcttcgtgtgtttcagcaacgcggcctgcttggcctcgctgacctgttttgccaggtcctcgccggcggtttttcgcttcttggtcgtcatagttcctcgcgtgtcgatggtcatcgacttcgccaaacctgccgcctcctgttcgagacgacgcgaacgctccacggcggccgatggcgcgggcagggcagggggagccagttgcacgctgtcgcgctcgatcttggccgtagcttgctggaccatcgagccgacggactggaaggtttcgcggggcgcacgcatgacggtgcggcttgcgatggtttcggcatcctcggcggaaaaccccgcgtcgatcagttcttgcctgtatgccttccggtcaaacgtccgattcattcaccctccttgcgggattgccccgactcacgccggggcaatgtgcccttattcctgatttgacccgcctggtgccttggtgtccagataatccaccttatcggcaatgaagtcggtcccgtagaccgtctggccgtccttctcgtacttggtattccgaatcttgccctgcacgaataccagctccgcgaagtcgctcttcttgatggagcgcatggggacgtgcttggcaatcacgcgcaccccccggccgttttagcggctaaaaaagtcatggctctgccctcgggcggaccacgcccatcatgaccttgccaagctcgtcctgcttctcttcgatcttcgccagcagggcgaggatcgtggcatcaccgaaccgcgccgtgcgcgggtcgtcggtgagccagagtttcagcaggccgcccaggcggcccaggtcgccattgatgcgggccagctcgcggacgtgctcatagtccacgacgcccgtgattttgtagccctggccgacggccagcaggtaggcctacaggctcatgccggccgccgccgccttttcctcaatcgctcttcgttcgtctggaaggcagtacaccttgataggtgggctgcccttcctggttggcttggtttcatcagccatccgcttgccctcatctgttacgccggcggtagccggccagcctcgcagagcaggattcccgttgagcaccgccaggtgcgaataagggacagtgaagaaggaacacccgctcgcgggtgggcctacttcacctatcctgcccggctgacgccgttggatacaccaaggaaagtctacacgaaccctttggcaaaatcctgtatatcgtgcgaaaaaggatggatataccgaaaaaatcgctataatgaccccgaagcagggttatgcagcggaaaagatccgtc

SEQ ID NO: 55 - DNA, 7219 bp, Artificial Sequence
  pAWP89S-Po-dTomato-RBS(PmoC1)
gaccctttccgacgctcaccgggctggttgccctcgccgctgggctggcggccgtctatggccctgcaaacgcgccagaaacgccgtcgaagccgtgtgcgagacaccgcggccgccggcgttgtggatacctcgcggaaaacttggccctcactgacagatgaggggcggacgttgacacttgaggggccgactcacccggcgcggcgttgacagatgaggggcaggctcgatttcggccggcgacgtggagctggccagcctcgcaaatcggcgaaaacgcctgattttacgcgagtttcccacagatgatgtggacaagcctggggataagtgccctgcggtattgacacttgaggggcgcgactactgacagatgaggggcgcgatccttgacacttgaggggcagagtgctgacagatgaggggcgcacctattgacatttgaggggctgtccacaggcagaaaatccagcatttgcaagggtttccgcccgtttttcggccaccgctaacctgtcttttaacctgcttttaaaccaatatttataaaccttgtttttaaccagggctgcgccctgtgcgcgtgaccgcgcacgccgaaggggggtgcccccccttctcgaaccctcccggcccgctaacgcgggcctcccatccccccaggggctgcgcccctcggccgcgaacggcctcaccccaaaaatggcagccaagctgacccgctagggacgtgaagtcgattccttcgatggttagcaatcaaagactcagagtgctgtctggagcgtgaatctaacggtacgtatctcgattgctcggtcgctattcgcactctgcgaaagttcgtaccgctcattcactaggttgcgaaatcagagattttgagacacaaatttaaatcgtaattattggggacccctggattctcaccaataaaaaacgcccggcggcaaccgagcgttctgaacaaatccagatggagttctgaggtcattactggatctatcaacaggagtccaagactagtagcggataacaatttcacacaggattagccttcgatgccgattttcttcagccgataggccagtgccggtcggcttaggccgagcaagcgcgcggcaccggagacgttttggttggcctgttgcatggctttgcgcatcaggctttcctcgatctcgtcgaggctcaggccgctgctcaacaactggctgatccaactgccctggccattgcctggctgaatcagcacgccgtccgacgacacccgctcgctggcggtctgcggctcttccggcgcccgtgggaacagcgcctgcacgctgatgctttcgttcggatcggtgaggatgatgccgcgctcgatgacgttctccagctcacggatattgcccggccaactgtaatgcaggcaggcctccagggctttgtctgaaaggccgagggttctcttgccgtactcctggtggaagcgctgaaggaagtgctcaaccagcagtggaatgtcctcgcggcgttcgcgcaacgccgggatcgccaccgggaaaacgttcagccggtagtacaggtcggcgcgaaaacgcccggccttgaccgcttcggccaggtcctcgtgggtggctgcgataacccttacgtcgatcttgcgcgtgcggttgtcgccaactcgctccagctcgccttcttgcagcacgcgcagcagactggcctgagcgcgcgggctgagttcgatcacctcgtcaaggaagatggtgcccttgtcggcccgctcgaagcggcccatgcgtgactgggtggcgccggtgaaggcgcctttttccacgccgaacaattcggactcgatcaggtccggcgggatcgccgcacagttcaccgcgacaaagggctcggcggcgcgtttgctgcgcaggtgcacgctacgcgcgatgacctccttgccgaccccggtctcgccaagcagcagcaccgagactttgccctgtgcggccttgtccatcatattgcgcacggtctggtaggccggggtctgaccgatgccgtagtactggccttcctgtttgtcgaggttggtacgcagcgacaccagttgcgattgcaactcgtagagttcctcgatgatggggtcgttcttgaaatactgtttgaagctggcaacgtcgtcccactcttcggccggcttgccaatgacccggcacttgtcgccgccgcagccgcggcagctgacttccttgaagatgatttcccggcccatgaacgccgaggaataggcgcaggcgtagccgagcagagtccagcacaccgggtcttgcatctgccccaggtcggtctggcagatttccacctcgaaggagtcgatccactccatctcggcatagaagcgcccgcattccttgtcgatatcgacctcggtggggcggaccttgaccagacccttgagcgaatgcagctgcgggccggcgaggaacatgtcgtactcgctggcattcggtctaagcttcctggccagttcggcatccttcaggccggactggtaaccctggcgcaggaagaagcccttggcgcgttcgatgcccagggtattgaccatttcccggcgaaagctggccattgctgaaacctgcagcaacagcatgcgttgttcgccaagccagatcttgccttccgtgctctggaagtggatcaggttggtcaggtccttgaaatcggagtgctggatttcaggcttgtacttgatcggcatgtaagcgaggcccctatttatttttagatggggaaatcagggtcgccgctatagcgcaaggcaggcggcgattccagatggggtcatggggaaaatcggcagttttttcacctgcgccagctccccatagccgacctcagtatctggcaaaagtcaaccaaatgatcaatcgacggcagtgactttagtgctagagatcagccttcagctgcgccatgagcatttgctcaagcggccttgggcaattgatcaaatgcttaaaaagcctgcgcaagcgcggcttaatttcgctcgctccgatcattctaaaaattagaaacacattgaaaaacaataccttgaagtcggttttcagaccttggcacagctgttgcactttgtcctgcgcaatccgccaacctggagatctagaggcccctgtcaaccatcactttaggaggaacaaacaatggtgagcaagggcgaggaggtcatcaaagagttcatgcgcttcaaggtgcgcatggagggctccatgaacggccacgagttcgagatcgagggcgagggcgagggccgcccctacgagggcacccagaccgccaagctgaaggtgaccaagggcggccccctgcccttcgcctgggacatcctgtccccccagttcatgtacggctccaaggcgtacgtgaagcaccccgccgacatccccgattacaagaagctgtccttccccgagggcttcaagtgggagcgcgtgatgaacttcgaggacggcggtctggtgaccgtgacccaggactcctccctgcaggacggcacgctgatctacaaggtgaagatgcgcggcaccaacttcccccccgacggccccgtaatgcagaagaagaccatgggctgggaggcctccaccgagcgcctgtacccccgcgacggcgtgctgaagggcgagatccaccaggccctgaagctgaaggacggcggccactacctggtggagttcaagaccatctacatggccaagaagcccgtgcaactgcccggctactactacgtggacaccaagctggacatcacctcccacaacgaggactacaccatcgtggaacagtacgagcgctccgagggccgccaccacctgttcctgtacggcatggacgagctgtacaagtagattgtcgggaagatgcgtgatctgatccttccactcagcaaaagttcgatttattcaacaaagccgccgtcccgtcaagtcagcgtaatgctctgccagtgttacaaccaattaaccaattctgattagaaaaactcatcgagcatcaaatgaaactgcaatttattcatatcaggattatcaataccatatttttgaaaaagccgtttctgtaatgaaggagaaaactcaccgaggcagttccataggatggcaagatcctggtatcggtctgcgattccgactcgtccaacatcaatacaacctattaatttcccctcgtcaaaaataaggttatcaagtgagaaatcaccatgagtgacgactgaatccggtgagaatggcaaaagcttatgcatttctttccagacttgttcaacaggccagccattacgctcgtcatcaaaatcactcgcatcaaccaaaccgttattcattcgtgattgcgcctgagcgagacgaaatacgcgatcgctgttaaaaggacaattacaaacaggaatcgaatgcaaccggcgcaggaacactgccagcgcatcaacaatattttcacctgaatcaggatattcttctaatacctggaatgctgttttcccggggatcgcagtggtgagtaaccatgcatcatcaggagtacggataaaatgcttgatggtcggaagaggcataaattccgtcagccagtttagtctgaccatctcatctgtaacatcattggcaacgctacctttgccatgtttcagaaacaactctggcgcatcgggcttcccatacaatcgatagattgtcgcacctgattgcccgacattatcgcgagcccatttatacccatataaatcagcatccatgttggaatttaatcgcggcctcgagcaagacgtttcccgttgaatatggctcataacaccccttgtattactgtttatgtaagcagacagttttattgttcatgatgatatatttttatcttgtgcaatgtaacatcagagattttgagacacaacgtggctttcgacttccggcaagctatacgcgccctagaattgtcaattttaatcctctgtttatcggcagttcgtagagcgcgccgtgcgtcccgagcgatactgagcgaagcaagtgcgtcgagcagtgcccgcttgttcctgaaatgccagtaaagcgctggctgctgaacccccagccggaactgaccccacaaggccctagcgtttgcaatgcaccaggtcatcattgacccaggcgtgttccaccaggccgctgcctcgcaactcttcgcaggcttcgccgacctgctcgcgccacttcttcacgcgggtggaatccgatccgcacatgaggcggaaggtttccagcttgagcgggtacggctcccggtgcgagctgaaatagtcgaacatccgtcgggccgtcggcgacagcttgcggtacttctcccatatgaatttcgtgtagtggtcgccagcaaacagcacgacgatttcctcgtcgatcaggacctggcaacgggacgttttcttgccacggtccaggacgcggaagcggtgcagcagcgacaccgattccaggtgcccaacgcggtcggacgtgaagcccatcgccgtcgcctgtaggcgcgacaggcattcctcggccttcgtgtaataccggccattgatcgaccagcccaggtcctggcaaagctcgtagaacgtgaaggtgatcggctcgccgataggggtgcgcttcgcgtactccaacacctgctgccacaccagttcgtcatcgtcggcccgcagctcgacgccggtgtaggtgatcttcacgtccttgttgacgtggaaaatgaccttgttttgcagcgcctcgcgcgggattttcttgttgcgcgtggtgaacagggcagagcgggccgtgtcgtttggcatcgctcgcatcgtgtccggccacggcgcaatatcgaacaaggaaagctgcatttccttgatctgctgcttcgtgtgtttcagcaacgcggcctgcttggcctcgctgacctgttttgccaggtcctcgccggcggtttttcgcttcttggtcgtcatagttcctcgcgtgtcgatggtcatcgacttcgccaaacctgccgcctcctgttcgagacgacgcgaacgctccacggcggccgatggcgcgggcagggcagggggagccagttgcacgctgtcgcgctcgatcttggccgtagcttgctggaccatcgagccgacggactggaaggtttcgcggggcgcacgcatgacggtgcggcttgcgatggtttcggcatcctcggcggaaaaccccgcgtcgatcagttcttgcctgtatgccttccggtcaaacgtccgattcattcaccctccttgcgggattgccccgactcacgccggggcaatgtgcccttattcctgatttgacccgcctggtgccttggtgtccagataatccaccttatcggcaatgaagtcggtcccgtagaccgtctggccgtccttctcgtacttggtattccgaatcttgccctgcacgaataccagctccgcgaagtcgctcttcttgatggagcgcatggggacgtgcttggcaatcacgcgcaccccccggccgttttagcggctaaaaaagtcatggctctgccctcgggcggaccacgcccatcatgaccttgccaagctcgtcctgcttctcttcgatcttcgccagcagggcgaggatcgtggcatcaccgaaccgcgccgtgcgcgggtcgtcggtgagccagagtttcagcaggccgcccaggcggcccaggtcgccattgatgcgggccagctcgcggacgtgctcatagtccacgacgcccgtgattttgtagccctggccgacggccagcaggtaggcctacaggctcatgccggccgccgccgccttttcctcaatcgctcttcgttcgtctggaaggcagtacaccttgataggtgggctgcccttcctggttggcttggtttcatcagccatccgcttgccctcatctgttacgccggcggtagccggccagcctcgcagagcaggattcccgttgagcaccgccaggtgcgaataagggacagtgaagaaggaacacccgctcgcgggtgggcctacttcacctatcctgcccggctgacgccgttggatacaccaaggaaagtctacacgaaccctttggcaaaatcctgtatatcgtgcgaaaaaggatggatataccgaaaaaatcgctataatgaccccgaagcagggttatgcagcggaaaagatccgtc

SEQ ID NO: 56 - DNA, 7219 bp, Artificial Sequence
  pAWP89S-Po-dTomato-RBS(PmoC2)
gaccctttccgacgctcaccgggctggttgccctcgccgctgggctggcggccgtctatggccctgcaaacgcgccagaaacgccgtcgaagccgtgtgcgagacaccgcggccgccggcgttgtggatacctcgcggaaaacttggccctcactgacagatgaggggcggacgttgacacttgaggggccgactcacccggcgcggcgttgacagatgaggggcaggctcgatttcggccggcgacgtggagctggccagcctcgcaaatcggcgaaaacgcctgattttacgcgagtttcccacagatgatgtggacaagcctggggataagtgccctgcggtattgacacttgaggggcgcgactactgacagatgaggggcgcgatccttgacacttgaggggcagagtgctgacagatgaggggcgcacctattgacatttgaggggctgtccacaggcagaaaatccagcatttgcaagggtttccgcccgtttttcggccaccgctaacctgtcttttaacctgcttttaaaccaatatttataaaccttgtttttaaccagggctgcgccctgtgcgcgtgaccgcgcacgccgaaggggggtgcccccccttctcgaaccctcccggcccgctaacgcgggcctcccatccccccaggggctgcgcccctcggccgcgaacggcctcaccccaaaaatggcagccaagctgacccgctagggacgtgaagtcgattccttcgatggttagcaatcaaagactcagagtgctgtctggagcgtgaatctaacggtacgtatctcgattgctcggtcgctattcgcactctgcgaaagttcgtaccgctcattcactaggttgcgaaatcagagattttgagacacaaatttaaatcgtaattattggggacccctggattctcaccaataaaaaacgcccggcggcaaccgagcgttctgaacaaatccagatggagttctgaggtcattactggatctatcaacaggagtccaagactagtagcggataacaatttcacacaggattagccttcgatgccgattttcttcagccgataggccagtgccggtcggcttaggccgagcaagcgcgcggcaccggagacgttttggttggcctgttgcatggctttgcgcatcaggctttcctcgatctcgtcgaggctcaggccgctgctcaacaactggctgatccaactgccctggccattgcctggctgaatcagcacgccgtccgacgacacccgctcgctggcggtctgcggctcttccggcgcccgtgggaacagcgcctgcacgctgatgctttcgttcggatcggtgaggatgatgccgcgctcgatgacgttctccagctcacggatattgcccggccaactgtaatgcaggcaggcctccagggctttgtctgaaaggccgagggttctcttgccgtactcctggtggaagcgctgaaggaagtgctcaaccagcagtggaatgtcctcgcggcgttcgcgcaacgccgggatcgccaccgggaaaacgttcagccggtagtacaggtcggcgcgaaaacgcccggccttgaccgcttcggccaggtcctcgtgggtggctgcgataacccttacgtcgatcttgcgcgtgcggttgtcgccaactcgctccagctcgccttcttgcagcacgcgcagcagactggcctgagcgcgcgggctgagttcgatcacctcgtcaaggaagatggtgcccttgtcggcccgctcgaagcggcccatgcgtgactgggtggcgccggtgaaggcgcctttttccacgccgaacaattcggactcgatcaggtccggcgggatcgccgcacagttcaccgcgacaaagggctcggcggcgcgtttgctgcgcaggtgcacgctacgcgcgatgacctccttgccgaccccggtctcgccaagcagcagcaccgagactttgccctgtgcggccttgtccatcatattgcgcacggtctggtaggccggggtctgaccgatgccgtagtactggccttcctgtttgtcgaggttggtacgcagcgacaccagttgcgattgcaactcgtagagttcctcgatgatggggtcgttcttgaaatactgtttgaagctggcaacgtcgtcccactcttcggccggcttgccaatgacccggcacttgtcgccgccgcagccgcggcagctgacttccttgaagatgatttcccggcccatgaacgccgaggaataggcgcaggcgtagccgagcagagtccagcacaccgggtcttgcatctgccccaggtcggtctggcagatttccacctcgaaggagtcgatccactccatctcggcatagaagcgcccgcattccttgtcgatatcgacctcggtggggcggaccttgaccagacccttgagcgaatgcagctgcgggccggcgaggaacatgtcgtactcgctggcattcggtctaagcttcctggccagttcggcatccttcaggccggactggtaaccctggcgcaggaagaagcccttggcgcgttcgatgcccagggtattgaccatttcccggcgaaagctggccattgctgaaacctgcagcaacagcatgcgttgttcgccaagccagatcttgccttccgtgctctggaagtggatcaggttggtcaggtccttgaaatcggagtgctggatttcaggcttgtacttgatcggcatgtaagcgaggcccctatttatttttagatggggaaatcagggtcgccgctatagcgcaaggcaggcggcgattccagatggggtcatggggaaaatcggcagttttttcacctgcgccagctccccatagccgacctcagtatctggcaaaagtcaaccaaatgatcaatcgacggcagtgactttagtgctagagatcagccttcagctgcgccatgagcatttgctcaagcggccttgggcaattgatcaaatgcttaaaaagcctgcgcaagcgcggcttaatttcgctcgctccgatcattctaaaaattagaaacacattgaaaaacaataccttgaagtcggttttcagaccttggcacagctgttgcactttgtcctgcgcaatccgccaacctggagatctagaccggtgttcacatcgatataacagttggaggtaaaaatggtgagcaagggcgaggaggtcatcaaagagttcatgcgcttcaaggtgcgcatggagggctccatgaacggccacgagttcgagatcgagggcgagggcgagggccgcccctacgagggcacccagaccgccaagctgaaggtgaccaagggcggccccctgcccttcgcctgggacatcctgtccccccagttcatgtacggctccaaggcgtacgtgaagcaccccgccgacatccccgattacaagaagctgtccttccccgagggcttcaagtgggagcgcgtgatgaacttcgaggacggcggtctggtgaccgtgacccaggactcctccctgcaggacggcacgctgatctacaaggtgaagatgcgcggcaccaacttcccccccgacggccccgtaatgcagaagaagaccatgggctgggaggcctccaccgagcgcctgtacccccgcgacggcgtgctgaagggcgagatccaccaggccctgaagctgaaggacggcggccactacctggtggagttcaagaccatctacatggccaagaagcccgtgcaactgcccggctactactacgtggacaccaagctggacatcacctcccacaacgaggactacaccatcgtggaacagtacgagcgctccgagggccgccaccacctgttcctgtacggcatggacgagctgtacaagtagattgtcgggaagatgcgtgatctgatccttccactcagcaaaagttcgatttattcaacaaagccgccgtcccgtcaagtcagcgtaatgctctgccagtgttacaaccaattaaccaattctgattagaaaaactcatcgagcatcaaatgaaactgcaatttattcatatcaggattatcaataccatatttttgaaaaagccgtttctgtaatgaaggagaaaactcaccgaggcagttccataggatggcaagatcctggtatcggtctgcgattccgactcgtccaacatcaatacaacctattaatttcccctcgtcaaaaataaggttatcaagtgagaaatcaccatgagtgacgactgaatccggtgagaatggcaaaagcttatgcatttctttccagacttgttcaacaggccagccattacgctcgtcatcaaaatcactcgcatcaaccaaaccgttattcattcgtgattgcgcctgagcgagacgaaatacgcgatcgctgttaaaaggacaattacaaacaggaatcgaatgcaaccggcgcaggaacactgccagcgcatcaacaatattttcacctgaatcaggatattcttctaatacctggaatgctgttttcccggggatcgcagtggtgagtaaccatgcatcatcaggagtacggataaaatgcttgatggtcggaagaggcataaattccgtcagccagtttagtctgaccatctcatctgtaacatcattggcaacgctacctttgccatgtttcagaaacaactctggcgcatcgggcttcccatacaatcgatagattgtcgcacctgattgcccgacattatcgcgagcccatttatacccatataaatcagcatccatgttggaatttaatcgcggcctcgagcaagacgtttcccgttgaatatggctcataacaccccttgtattactgtttatgtaagcagacagttttattgttcatgatgatatatttttatcttgtgcaatgtaacatcagagattttgagacacaacgtggctttcgacttccggcaagctatacgcgccctagaattgtcaattttaatcctctgtttatcggcagttcgtagagcgcgccgtgcgtcccgagcgatactgagcgaagcaagtgcgtcgagcagtgcccgcttgttcctgaaatgccagtaaagcgctggctgctgaacccccagccggaactgaccccacaaggccctagcgtttgcaatgcaccaggtcatcattgacccaggcgtgttccaccaggccgctgcctcgcaactcttcgcaggcttcgccgacctgctcgcgccacttcttcacgcgggtggaatccgatccgcacatgaggcggaaggtttccagcttgagcgggtacggctcccggtgcgagctgaaatagtcgaacatccgtcgggccgtcggcgacagcttgcggtacttctcccatatgaatttcgtgtagtggtcgccagcaaacagcacgacgatttcctcgtcgatcaggacctggcaacgggacgttttcttgccacggtccaggacgcggaagcggtgcagcagcgacaccgattccaggtgcccaacgcggtcggacgtgaagcccatcgccgtcgcctgtaggcgcgacaggcattcctcggccttcgtgtaataccggccattgatcgaccagcccaggtcctggcaaagctcgtagaacgtgaaggtgatcggctcgccgataggggtgcgcttcgcgtactccaacacctgctgccacaccagttcgtcatcgtcggcccgcagctcgacgccggtgtaggtgatcttcacgtccttgttgacgtggaaaatgaccttgttttgcagcgcctcgcgcgggattttcttgttgcgcgtggtgaacagggcagagcgggccgtgtcgtttggcatcgctcgcatcgtgtccggccacggcgcaatatcgaacaaggaaagctgcatttccttgatctgctgcttcgtgtgtttcagcaacgcggcctgcttggcctcgctgacctgttttgccaggtcctcgccggcggtttttcgcttcttggtcgtcatagttcctcgcgtgtcgatggtcatcgacttcgccaaacctgccgcctcctgttcgagacgacgcgaacgctccacggcggccgatggcgcgggcagggcagggggagccagttgcacgctgtcgcgctcgatcttggccgtagcttgctggaccatcgagccgacggactggaaggtttcgcggggcgcacgcatgacggtgcggcttgcgatggtttcggcatcctcggcggaaaaccccgcgtcgatcagttcttgcctgtatgccttccggtcaaacgtccgattcattcaccctccttgcgggattgccccgactcacgccggggcaatgtgcccttattcctgatttgacccgcctggtgccttggtgtccagataatccaccttatcggcaatgaagtcggtcccgtagaccgtctggccgtccttctcgtacttggtattccgaatcttgccctgcacgaataccagctccgcgaagtcgctcttcttgatggagcgcatggggacgtgcttggcaatcacgcgcaccccccggccgttttagcggctaaaaaagtcatggctctgccctcgggcggaccacgcccatcatgaccttgccaagctcgtcctgcttctcttcgatcttcgccagcagggcgaggatcgtggcatcaccgaaccgcgccgtgcgcgggtcgtcggtgagccagagtttcagcaggccgcccaggcggcccaggtcgccattgatgcgggccagctcgcggacgtgctcatagtccacgacgcccgtgattttgtagccctggccgacggccagcaggtaggcctacaggctcatgccggccgccgccgccttttcctcaatcgctcttcgttcgtctggaaggcagtacaccttgataggtgggctgcccttcctggttggcttggtttcatcagccatccgcttgccctcatctgttacgccggcggtagccggccagcctcgcagagcaggattcccgttgagcaccgccaggtgcgaataagggacagtgaagaaggaacacccgctcgcgggtgggcctacttcacctatcctgcccggctgacgccgttggatacaccaaggaaagtctacacgaaccctttggcaaaatcctgtatatcgtgcgaaaaaggatggatataccgaaaaaatcgctataatgaccccgaagcagggttatgcagcggaaaagatccgtc

SEQ ID NO: 57 - DNA, 7219 bp, Artificial Sequence
  pAWP89S-Po-dTomato-RBS(PmoC3)
gaccctttccgacgctcaccgggctggttgccctcgccgctgggctggcggccgtctatggccctgcaaacgcgccagaaacgccgtcgaagccgtgtgcgagacaccgcggccgccggcgttgtggatacctcgcggaaaacttggccctcactgacagatgaggggcggacgttgacacttgaggggccgactcacccggcgcggcgttgacagatgaggggcaggctcgatttcggccggcgacgtggagctggccagcctcgcaaatcggcgaaaacgcctgattttacgcgagtttcccacagatgatgtggacaagcctggggataagtgccctgcggtattgacacttgaggggcgcgactactgacagatgaggggcgcgatccttgacacttgaggggcagagtgctgacagatgaggggcgcacctattgacatttgaggggctgtccacaggcagaaaatccagcatttgcaagggtttccgcccgtttttcggccaccgctaacctgtcttttaacctgcttttaaaccaatatttataaaccttgtttttaaccagggctgcgccctgtgcgcgtgaccgcgcacgccgaaggggggtgcccccccttctcgaaccctcccggcccgctaacgcgggcctcccatccccccaggggctgcgcccctcggccgcgaacggcctcaccccaaaaatggcagccaagctgacccgctagggacgtgaagtcgattccttcgatggttagcaatcaaagactcagagtgctgtctggagcgtgaatctaacggtacgtatctcgattgctcggtcgctattcgcactctgcgaaagttcgtaccgctcattcactaggttgcgaaatcagagattttgagacacaaatttaaatcgtaattattggggacccctggattctcaccaataaaaaacgcccggcggcaaccgagcgttctgaacaaatccagatggagttctgaggtcattactggatctatcaacaggagtccaagactagtagcggataacaatttcacacaggattagccttcgatgccgattttcttcagccgataggccagtgccggtcggcttaggccgagcaagcgcgcggcaccggagacgttttggttggcctgttgcatggctttgcgcatcaggctttcctcgatctcgtcgaggctcaggccgctgctcaacaactggctgatccaactgccctggccattgcctggctgaatcagcacgccgtccgacgacacccgctcgctggcggtctgcggctcttccggcgcccgtgggaacagcgcctgcacgctgatgctttcgttcggatcggtgaggatgatgccgcgctcgatgacgttctccagctcacggatattgcccggccaactgtaatgcaggcaggcctccagggctttgtctgaaaggccgagggttctcttgccgtactcctggtggaagcgctgaaggaagtgctcaaccagcagtggaatgtcctcgcggcgttcgcgcaacgccgggatcgccaccgggaaaacgttcagccggtagtacaggtcggcgcgaaaacgcccggccttgaccgcttcggccaggtcctcgtgggtggctgcgataacccttacgtcgatcttgcgcgtgcggttgtcgccaactcgctccagctcgccttcttgcagcacgcgcagcagactggcctgagcgcgcgggctgagttcgatcacctcgtcaaggaagatggtgcccttgtcggcccgctcgaagcggcccatgcgtgactgggtggcgccggtgaaggcgcctttttccacgccgaacaattcggactcgatcaggtccggcgggatcgccgcacagttcaccgcgacaaagggctcggcggcgcgtttgctgcgcaggtgcacgctacgcgcgatgacctccttgccgaccccggtctcgccaagcagcagcaccgagactttgccctgtgcggccttgtccatcatattgcgcacggtctggtaggccggggtctgaccgatgccgtagtactggccttcctgtttgtcgaggttggtacgcagcgacaccagttgcgattgcaactcgtagagttcctcgatgatggggtcgttcttgaaatactgtttgaagctggcaacgtcgtcccactcttcggccggcttgccaatgacccggcacttgtcgccgccgcagccgcggcagctgacttccttgaagatgatttcccggcccatgaacgccgaggaataggcgcaggcgtagccgagcagagtccagcacaccgggtcttgcatctgccccaggtcggtctggcagatttccacctcgaaggagtcgatccactccatctcggcatagaagcgcccgcattccttgtcgatatcgacctcggtggggcggaccttgaccagacccttgagcgaatgcagctgcgggccggcgaggaacatgtcgtactcgctggcattcggtctaagcttcctggccagttcggcatccttcaggccggactggtaaccctggcgcaggaagaagcccttggcgcgttcgatgcccagggtattgaccatttcccggcgaaagctggccattgctgaaacctgcagcaacagcatgcgttgttcgccaagccagatcttgccttccgtgctctggaagtggatcaggttggtcaggtccttgaaatcggagtgctggatttcaggcttgtacttgatcggcatgtaagcgaggcccctatttatttttagatggggaaatcagggtcgccgctatagcgcaaggcaggcggcgattccagatggggtcatggggaaaatcggcagttttttcacctgcgccagctccccatagccgacctcagtatctggcaaaagtcaaccaaatgatcaatcgacggcagtgactttagtgctagagatcagccttcagctgcgccatgagcatttgctcaagcggccttgggcaattgatcaaatgcttaaaaagcctgcgcaagcgcggcttaatttcgctcgctccgatcattctaaaaattagaaacacattgaaaaacaataccttgaagtcggttttcagaccttggcacagctgttgcactttgtcctgcgcaatccgccaacctggagatctagagtggcatcaatccaacaccaactcaggagaaatcagatggtgagcaagggcgaggaggtcatcaaagagttcatgcgcttcaaggtgcgcatggagggctccatgaacggccacgagttcgagatcgagggcgagggcgagggccgcccctacgagggcacccagaccgccaagctgaaggtgaccaagggcggccccctgcccttcgcctgggacatcctgtccccccagttcatgtacggctccaaggcgtacgtgaagcaccccgccgacatccccgattacaagaagctgtccttccccgagggcttcaagtgggagcgcgtgatgaacttcgaggacggcggtctggtgaccgtgacccaggactcctccctgcaggacggcacgctgatctacaaggtgaagatgcgcggcaccaacttcccccccgacggccccgtaatgcagaagaagaccatgggctgggaggcctccaccgagcgcctgtacccccgcgacggcgtgctgaagggcgagatccaccaggccctgaagctgaaggacggcggccactacctggtggagttcaagaccatctacatggccaagaagcccgtgcaactgcccggctactactacgtggacaccaagctggacatcacctcccacaacgaggactacaccatcgtggaacagtacgagcgctccgagggccgccaccacctgttcctgtacggcatggacgagctgtacaagtagattgtcgggaagatgcgtgatctgatccttccactcagcaaaagttcgatttattcaacaaagccgccgtcccgtcaagtcagcgtaatgctctgccagtgttacaaccaattaaccaattctgattagaaaaactcatcgagcatcaaatgaaactgcaatttattcatatcaggattatcaataccatatttttgaaaaagccgtttctgtaatgaaggagaaaactcaccgaggcagttccataggatggcaagatcctggtatcggtctgcgattccgactcgtccaacatcaatacaacctattaatttcccctcgtcaaaaataaggttatcaagtgagaaatcaccatgagtgacgactgaatccggtgagaatggcaaaagcttatgcatttctttccagacttgttcaacaggccagccattacgctcgtcatcaaaatcactcgcatcaaccaaaccgttattcattcgtgattgcgcctgagcgagacgaaatacgcgatcgctgttaaaaggacaattacaaacaggaatcgaatgcaaccggcgcaggaacactgccagcgcatcaacaatattttcacctgaatcaggatattcttctaatacctggaatgctgttttcccggggatcgcagtggtgagtaaccatgcatcatcaggagtacggataaaatgcttgatggtcggaagaggcataaattccgtcagccagtttagtctgaccatctcatctgtaacatcattggcaacgctacctttgccatgtttcagaaacaactctggcgcatcgggcttcccatacaatcgatagattgtcgcacctgattgcccgacattatcgcgagcccatttatacccatataaatcagcatccatgttggaatttaatcgcggcctcgagcaagacgtttcccgttgaatatggctcataacaccccttgtattactgtttatgtaagcagacagttttattgttcatgatgatatatttttatcttgtgcaatgtaacatcagagattttgagacacaacgtggctttcgacttccggcaagctatacgcgccctagaattgtcaattttaatcctctgtttatcggcagttcgtagagcgcgccgtgcgtcccgagcgatactgagcgaagcaagtgcgtcgagcagtgcccgcttgttcctgaaatgccagtaaagcgctggctgctgaacccccagccggaactgaccccacaaggccctagcgtttgcaatgcaccaggtcatcattgacccaggcgtgttccaccaggccgctgcctcgcaactcttcgcaggcttcgccgacctgctcgcgccacttcttcacgcgggtggaatccgatccgcacatgaggcggaaggtttccagcttgagcgggtacggctcccggtgcgagctgaaatagtcgaacatccgtcgggccgtcggcgacagcttgcggtacttctcccatatgaatttcgtgtagtggtcgccagcaaacagcacgacgatttcctcgtcgatcaggacctggcaacgggacgttttcttgccacggtccaggacgcggaagcggtgcagcagcgacaccgattccaggtgcccaacgcggtcggacgtgaagcccatcgccgtcgcctgtaggcgcgacaggcattcctcggccttcgtgtaataccggccattgatcgaccagcccaggtcctggcaaagctcgtagaacgtgaaggtgatcggctcgccgataggggtgcgcttcgcgtactccaacacctgctgccacaccagttcgtcatcgtcggcccgcagctcgacgccggtgtaggtgatcttcacgtccttgttgacgtggaaaatgaccttgttttgcagcgcctcgcgcgggattttcttgttgcgcgtggtgaacagggcagagcgggccgtgtcgtttggcatcgctcgcatcgtgtccggccacggcgcaatatcgaacaaggaaagctgcatttccttgatctgctgcttcgtgtgtttcagcaacgcggcctgcttggcctcgctgacctgttttgccaggtcctcgccggcggtttttcgcttcttggtcgtcatagttcctcgcgtgtcgatggtcatcgacttcgccaaacctgccgcctcctgttcgagacgacgcgaacgctccacggcggccgatggcgcgggcagggcagggggagccagttgcacgctgtcgcgctcgatcttggccgtagcttgctggaccatcgagccgacggactggaaggtttcgcggggcgcacgcatgacggtgcggcttgcgatggtttcggcatcctcggcggaaaaccccgcgtcgatcagttcttgcctgtatgccttccggtcaaacgtccgattcattcaccctccttgcgggattgccccgactcacgccggggcaatgtgcccttattcctgatttgacccgcctggtgccttggtgtccagataatccaccttatcggcaatgaagtcggtcccgtagaccgtctggccgtccttctcgtacttggtattccgaatcttgccctgcacgaataccagctccgcgaagtcgctcttcttgatggagcgcatggggacgtgcttggcaatcacgcgcaccccccggccgttttagcggctaaaaaagtcatggctctgccctcgggcggaccacgcccatcatgaccttgccaagctcgtcctgcttctcttcgatcttcgccagcagggcgaggatcgtggcatcaccgaaccgcgccgtgcgcgggtcgtcggtgagccagagtttcagcaggccgcccaggcggcccaggtcgccattgatgcgggccagctcgcggacgtgctcatagtccacgacgcccgtgattttgtagccctggccgacggccagcaggtaggcctacaggctcatgccggccgccgccgccttttcctcaatcgctcttcgttcgtctggaaggcagtacaccttgataggtgggctgcccttcctggttggcttggtttcatcagccatccgcttgccctcatctgttacgccggcggtagccggccagcctcgcagagcaggattcccgttgagcaccgccaggtgcgaataagggacagtgaagaaggaacacccgctcgcgggtgggcctacttcacctatcctgcccggctgacgccgttggatacaccaaggaaagtctacacgaaccctttggcaaaatcctgtatatcgtgcgaaaaaggatggatataccgaaaaaatcgctataatgaccccgaagcagggttatgcagcggaaaagatccgtc

SEQ ID NO: 58 - DNA, 11948 bp, Artificial Sequence
  pAWPSG-Po-nCas9-BE-RiboJ-sgRNA(McglgA4)
gaccctttccgacgctcaccgggctggttgccctcgccgctgggctggcggccgtctatggccctgcaaacgcgccagaaacgccgtcgaagccgtgtgcgagacaccgcggccgccggcgttgtggatacctcgcggaaaacttggccctcactgacagatgaggggcggacgttgacacttgaggggccgactcacccggcgcggcgttgacagatgaggggcaggctcgatttcggccggcgacgtggagctggccagcctcgcaaatcggcgaaaacgcctgattttacgcgagtttcccacagatgatgtggacaagcctggggataagtgccctgcggtattgacacttgaggggcgcgactactgacagatgaggggcgcgatccttgacacttgaggggcagagtgctgacagatgaggggcgcacctattgacatttgaggggctgtccacaggcagaaaatccagcatttgcaagggtttccgcccgtttttcggccaccgctaacctgtcttttaacctgcttttaaaccaatatttataaaccttgtttttaaccagggctgcgccctgtgcgcgtgaccgcgcacgccgaaggggggtgcccccccttctcgaaccctcccggcccgctaacgcgggcctcccatccccccaggggctgcgcccctcggccgcgaacggcctcaccccaaaaatggcagccaagctgacccgctagggacgtgaagtcgattccttcgatggttagcaatcaaagactcagagtgctgtctggagcgtgaatctaacggtacgtatctcgattgctcggtcgctattcgcactctgcgaaagttcgtaccgctcattcactaggttgcgaaaatttaaatcgtaattattggggacccctggattctcaccaataaaaaacgcccggcggcaaccgagcgttctgaacaaatccagatggagttctgaggtcattactggatctatcaacaggagtccaagactagtagcggataacaatttcacacaggattagccttcgatgccgattttcttcagccgataggccagtgccggtcggcttaggccgagcaagcgcgcggcaccggagacgttttggttggcctgttgcatggctttgcgcatcaggctttcctcgatctcgtcgaggctcaggccgctgctcaacaactggctgatccaactgccctggccattgcctggctgaatcagcacgccgtccgacgacacccgctcgctggcggtctgcggctcttccggcgcccgtgggaacagcgcctgcacgctgatgctttcgttcggatcggtgaggatgatgccgcgctcgatgacgttctccagctcacggatattgcccggccaactgtaatgcaggcaggcctccagggctttgtctgaaaggccgagggttctcttgccgtactcctggtggaagcgctgaaggaagtgctcaaccagcagtggaatgtcctcgcggcgttcgcgcaacgccgggatcgccaccgggaaaacgttcagccggtagtacaggtcggcgcgaaaacgcccggccttgaccgcttcggccaggtcctcgtgggtggctgcgataacccttacgtcgatcttgcgcgtgcggttgtcgccaactcgctccagctcgccttcttgcagcacgcgcagcaaactggcctgagcgcgcgggctgagttcgatcacctcgtcaaggaagatggtgcccttgtcggcccgctcgaagcggcccatgcgtgactgggtggcgccggtgaaggcgcctttttccacgccgaacaattcggactcgatcaggtccggcgggatcgccgcacagttcaccgcgacaaagggctcggcggcgcgtttgctgcgcaggtgcacgctacgcgcgatgacctccttgccgaccccggtctcgccaagcagcagcaccgagactttgccctgtgcggccttgtccatcatattgcgcacggtctggtaggccggggtctgaccgatgccgtagtactggccttcctgtttgtcgaggttggtacgcagcgacaccagttgcgattgcaactcgtagagttcctcgatgatggggtcgttcttgaaatactgtttgaagctggcaacgtcgtcccactcttcggccggcttgccaatgacccggcacttgtcgccgccgcagccgcggcagctgacttccttgaagatgatttcccggcccatgaacgccgaggaataggcgcaggcgtagccgagcagagtccagcacaccgggtcttgcatctgccccaggtcggtctggcagatttccacctcgaaggagtcgatccactccatctcggcatagaagcgcccgcattccttgtcgatatcgacctcggtggggcggaccttgaccagacccttgagcgaatgcagctgcgggccggcgaggaacatgtcgtactcgctggcattcggtctaagcttcctggccagttcggcatccttcaggccggactggtaaccctggcgcaggaagaagcccttggcgcgttcgatgcccagggtattgaccatttcccggcgaaagctggccattgctgaaacctgcagcaacagcatgcgttgttcgccaagccagatcttgccttccgtgctctggaagtggatcaggttggtcaggtccttgaaatcggagtgctggatttcaggcttgtacttgatcggcatgtaagcgaggcccctatttatttttagatggggaaatcagggtcgccgctatagcgcaaggcaggcggcgattccagatggggtcatggggaaaatcggcagttttttcacctgcgccagctccccatagccgacctcagtatctggcaaaagtcaaccaaatgatcaatcgacggcagtgactttagtgctagagatcagccttcagctgcgccatgagcatttgctcaagcggccttgggcaattgatcaaatgcttaaaaagcctgcgcaagcgcggcttaatttcgctcgctccgatcattctaaaaattagaaacacattgaaaaacaataccttgaagtcggttttcagaccttggcacagctgttgcactttgtcctgcgcaatccgccaacctggagatctagaaataattttgtttaactttaagaaggagatatacatatgagctcagagactggcccagtggctgtggaccccacattgagacggcggatcgagccccatgagtttgaggtattcttcgatccgagagagctccgcaaggagacctgcctgctttacgaaattaattgggggggccggcactccatttggcgacatacatcacagaacactaacaagcacgtcgaagtcaacttcatcgagaagttcacgacagaaagatatttctgtccgaacacaaggtgcagcattacctggtttctcagctggagcccatgcggcgaatgtagtagggccatcactgaattcctgtcaaggtatccccacgtcactctgtttatttacatcgcaaggctgtaccaccacgctgacccccgcaatcgacaaggcctgcgggatttgatctcttcaggtgtgactatccaaattatgactgagcaggagtcaggatactgctggagaaactttgtgaattatagcccgagtaatgaagcccactggcctaggtatccccatctgtgggtacgactgtacgttcttgaactgtactgcatcatactgggcctgcctccttgtctcaacattctgagaaggaagcagccacagctgacattctttaccatcgctcttcagtcttgtcattaccagcgactgcccccacacattctctgggccaccgggttgaaaagcggcagcgagactcccgggacctcagagtccgccacacccgaaagtgataagaaatactcaataggcttagctatcggcacaaatagcgtcggatgggcggtgatcactgatgaatataaggttccgtctaaaaagttcaaggttctgggaaatacagaccgccacagtatcaaaaaaaatcttataggggctcttttatttgacagtggagagacagcggaagcgactcgtctcaaacggacagctcgtagaaggtatacacgtcggaagaatcgtatttgttatctacaggagattttttcaaatgagatggcgaaagtagatgatagtttctttcatcgacttgaagagtcttttttggtggaagaagacaagaagcatgaacgtcatcctatttttggaaatatagtagatgaagttgcttatcatgagaaatatccaactatctatcatctgcgaaaaaaattggtagattctactgataaagcggatttgcgcttaatctatttggccttagcgcatatgattaagtttcgtggtcattttttgattgagggagatttaaatcctgataatagtgatgtggacaaactatttatccagttggtacaaacctacaatcaattatttgaagaaaaccctattaacgcaagtggagtagatgctaaagcgattctttctgcacgattgagtaaatcaagacgattagaaaatctcattgctcagctccccggtgagaagaaaaatggcttatttgggaatctcattgctttgtcattgggtttgacccctaattttaaatcaaattttgatttggcagaagatgctaaattacagctttcaaaagatacttacgatgatgatttagataatttattggcgcaaattggagatcaatatgctgatttgtttttggcagctaagaatttatcagatgctattttactttcagatatcctaagagtaaatactgaaataactaaggctcccctatcagcttcaatgattaaacgctacgatgaacatcatcaagacttgactcttttaaaagctttagttcgacaacaacttccagaaaagtataaagaaatcttttttgatcaatcaaaaaacggatatgcaggttatattgatgggggagctagccaagaagaattttataaatttatcaaaccaattttagaaaaaatggatggtactgaggaattattggtgaaactaaatcgtgaagatttgctgcgcaagcaacggacctttgacaacggctctattccccatcaaattcacttgggtgagctgcatgctattttgagaagacaagaagacttttatccatttttaaaagacaatcgtgagaagattgaaaaaatcttgacttttcgaattccttattatgttggtccattggcgcgtggcaatagtcgttttgcatggatgactcggaagtctgaagaaacaattaccccatggaattttgaagaagttgtcgataaaggtgcttcagctcaatcatttattgaacgcatgacaaactttgataaaaatcttccaaatgaaaaagtactaccaaaacatagtttgctttatgagtattttacggtttataacgaattgacaaaggtcaaatatgttactgaaggaatgcgaaaaccagcatttctttcaggtgaacagaagaaagccattgttgatttactcttcaaaacaaatcgaaaagtaaccgttaagcaattaaaagaagattatttcaaaaaaatagaatgttttgatagtgttgaaatttcaggagttgaagatagatttaatgcttcattaggtacctaccatgatttgctaaaaattattaaagataaagattttttggataatgaagaaaatgaagatatcttagaggatattgttttaacattgaccttatttgaagatagggagatgattgaggaaagacttaaaacatatgctcacctctttgatgataaggtgatgaaacagcttaaacgtcgccgttatactggttggggacgtttgtctcgaaaattgattaatggtattagggataagcaatctggcaaaacaatattagattttttgaaatcagatggttttgccaatcgcaattttatgcagctgatccatgatgatagtttgacatttaaagaagacattcaaaaagcacaagtgtctggacaaggcgatagtttacatgaacatattgcaaatttagctggtagccctgctattaaaaaaggtattttacagactgtaaaagttgttgatgaattggtcaaagtaatggggcggcataagccagaaaatatcgttattgaaatggcacgtgaaaatcagacaactcaaaagggccagaaaaattcgcgagagcgtatgaaacgaatcgaagaaggtatcaaagaattaggaagtcagattcttaaagagcatcctgttgaaaatactcaattgcaaaatgaaaagctctatctctattatctccaaaatggaagagacatgtatgtggaccaagaattagatattaatcgtttaagtgattatgatgtcgatcacattgttccacaaagtttccttaaagacgattcaatagacaataaggtcttaacgcgttctgataaaaatcgtggtaaatcggataacgttccaagtgaagaagtagtcaaaaagatgaaaaactattggagacaacttctaaacgccaagttaatcactcaacgtaagtttgataatttaacgaaagctgaacgtggaggtttgagtgaacttgataaagctggttttatcaaacgccaattggttgaaactcgccaaatcactaagcatgtggcacaaattttggatagtcgcatgaatactaaatacgatgaaaatgataaacttattcgagaggttaaagtgattaccttaaaatctaaattagtttctgacttccgaaaagatttccaattctataaagtacgtgagattaacaattaccatcatgcccatgatgcgtatctaaatgccgtcgttggaactgctttgattaagaaatatccaaaacttgaatcggagtttgtctatggtgattataaagtttatgatgttcgtaaaatgattgctaagtctgagcaagaaataggcaaagcaaccgcaaaatatttcttttactctaatatcatgaacttcttcaaaacagaaattacacttgcaaatggagagattcgcaaacgccctctaatcgaaactaatggggaaactggagaaattgtctgggataaagggcgagattttgccacagtgcgcaaagtattgtccatgccccaagtcaatattgtcaagaaaacagaagtacagacaggcggattctccaaggagtcaattttaccaaaaagaaattcggacaagcttattgctcgtaaaaaagactgggatccaaaaaaatatggtggttttgatagtccaacggtagcttattcagtcctagtggttgctaaggtggaaaaagggaaatcgaagaagttaaaatccgttaaagagttactagggatcacaattatggaaagaagttcctttgaaaaaaatccgattgactttttagaagctaaaggatataaggaagttaaaaaagacttaatcattaaactacctaaatatagtctttttgagttagaaaacggtcgtaaacggatgctggctagtgccggagaattacaaaaaggaaatgagctggctctgccaagcaaatatgtgaattttttatatttagctagtcattatgaaaagttgaagggtagtccagaagataacgaacaaaaacaattgtttgtggagcagcataagcattatttagatgagattattgagcaaatcagtgaattttctaagcgtgttattttagcagatgccaatttagataaagttcttagtgcatataacaaacatagagacaaaccaatacgtgaacaagcagaaaatattattcatttatttacgttgacgaatcttggagctcccgctgcttttaaatattttgatacaacaattgatcgtaaacgatatacgtctacaaaagaagttttagatgccactcttatccatcaatccatcactggtctttatgaaacacgcattgatttgagtcagctaggaggtgactctggtggttctactaatctgtcagatattattgaaaaggagaccggtaagcaactggttatccaggaatccatcctcatgctcccagaggaggtggaagaagtcattgggaacaagccggaaagcgatatactcgtgcacaccgcctacgacgagagcaccgacgagaatgtcatgcttctgactagcgacgcccctgaatacaagccttgggctctggtcatacaggatagcaacggtgagaacaagattaagatgctctaactgctgccaccgctgagcaataactcgagctgtcaccggatgtgctttccggtctgatgagtccgtgaggacgaaacagcctctacaaataattttgtttaagtttccagccgaggccgagcgttttagagctagaaatagcaagttaaaataaggctagtccgttatcaacttgaaaaagtggcaccgagtcggtgctttttttgacccggggcggccgcctcgattaattaaaggcatcaaataaaacgaaaggctcagtcgaaagactgggcctttcgttttatctgttgtttgtcggtgaacgctctcctgagtaggacaaatccgccgccctagacagctgggcgcgccattgtcgggaagatgcgtgatctgatccttccactcagcaaaagttcgatttattcaacaaagccgccgtcccgtcaagtcagcgtaatgctctgccagtgttacaaccaattaaccaattctgattagaaaaactcatcgagcatcaaatgaaactgcaatttattcatatcaggattatcaataccatatttttgaaaaagccgtttctgtaatgaaggagaaaactcaccgaggcagttccataggatggcaagatcctggtatcggtctgcgattccgactcgtccaacatcaatacaacctattaatttcccctcgtcaaaaataaggttatcaagtgagaaatcaccatgagtgacgactgaatccggtgagaatggcaaaagcttatgcatttctttccagacttgttcaacaggccagccattacgctcgtcatcaaaatcactcgcatcaaccaaaccgttattcattcgtgattgcgcctgagcgagacgaaatacgcgatcgctgttaaaaggacaattacaaacaggaatcgaatgcaaccggcgcaggaacactgccagcgcatcaacaatattttcacctgaatcaggatattcttctaatacctggaatgctgttttcccggggatcgcagtggtgagtaaccatgcatcatcaggagtacggataaaatgcttgatggtcggaagaggcataaattccgtcagccagtttagtctgaccatctcatctgtaacatcattggcaacgctacctttgccatgtttcagaaacaactctggcgcatcgggcttcccatacaatcgatagattgtcgcacctgattgcccgacattatcgcgagcccatttatacccatataaatcagcatccatgttggaatttaatcgcggcctcgagcaagacgtttcccgttgaatatggctcataacaccccttgtattactgtttatgtaagcagacagttttattgttcatgatgatatatttttatcttgtgcaatgtaacatcagagattttgagacacaacgtggctttcgacttccggcaagctatacgcgccctagaattgtcaattttaatcctctgtttatcggcagttcgtagagcgcgccgtgcgtcccgagcgatactgagcgaagcaagtgcgtcgagcagtgcccgcttgttcctgaaatgccagtaaagcgctggctgctgaacccccagccggaactgaccccacaaggccctagcgtttgcaatgcaccaggtcatcattgacccaggcgtgttccaccaggccgctgcctcgcaactcttcgcaggcttcgccgacctgctcgcgccacttcttcacgcgggtggaatccgatccgcacatgaggcggaaggtttccagcttgagcgggtacggctcccggtgcgagctgaaatagtcgaacatccgtcgggccgtcggcgacagcttgcggtacttctcccatatgaatttcgtgtagtggtcgccagcaaacagcacgacgatttcctcgtcgatcaggacctggcaacgggacgttttcttgccacggtccaggacgcggaagcggtgcagcagcgacaccgattccaggtgcccaacgcggtcggacgtgaagcccatcgccgtcgcctgtaggcgcgacaggcattcctcggccttcgtgtaataccggccattgatcgaccagcccaggtcctggcaaagctcgtagaacgtgaaggtgatcggctcgccgataggggtgcgcttcgcgtactccaacacctgctgccacaccagttcgtcatcgtcggcccgcagctcgacgccggtgtaggtgatcttcacgtccttgttgacgtggaaaatgaccttgttttgcagcgcctcgcgcgggattttcttgttgcgcgtggtgaacagggcagagcgggccgtgtcgtttggcatcgctcgcatcgtgtccggccacggcgcaatatcgaacaaggaaagctgcatttccttgatctgctgcttcgtgtgtttcagcaacgcggcctgcttggcctcgctgacctgttttgccaggtcctcgccggcggtttttcgcttcttggtcgtcatagttcctcgcgtgtcgatggtcatcgacttcgccaaacctgccgcctcctgttcgagacgacgcgaacgctccacggcggccgatggcgcgggcagggcagggggagccagttgcacgctgtcgcgctcgatcttggccgtagcttgctggaccatcgagccgacggactggaaggtttcgcggggcgcacgcatgacggtgcggcttgcgatggtttcggcatcctcggcggaaaaccccgcgtcgatcagttcttgcctgtatgccttccggtcaaacgtccgattcattcaccctccttgcgggattgccccgactcacgccggggcaatgtgcccttattcctgatttgacccgcctggtgccttggtgtccagataatccaccttatcggcaatgaagtcggtcccgtagaccgtctggccgtccttctcgtacttggtattccgaatcttgccctgcacgaataccagctccgcgaagtcgctcttcttgatggagcgcatggggacgtgcttggcaatcacgcgcaccccccggccgttttagcggctaaaaaagtcatggctctgccctcgggcggaccacgcccatcatgaccttgccaagctcgtcctgcttctcttcgatcttcgccagcagggcgaggatcgtggcatcaccgaaccgcgccgtgcgcgggtcgtcggtgagccagagtttcagcaggccgcccaggcggcccaggtcgccattgatgcgggccagctcgcggacgtgctcatagtccacgacgcccgtgattttgtagccctggccgacggccagcaggtaggcctacaggctcatgccggccgccgccgccttttcctcaatcgctcttcgttcgtctggaaggcagtacaccttgataggtgggctgcccttcctggttggcttggtttcatcagccatccgcttgccctcatctgttacgccggcggtagccggccagcctcgcagagcaggattcccgttgagcaccgccaggtgcgaataagggacagtgaagaaggaacacccgctcgcgggtgggcctacttcacctatcctgcccggctgacgccgttggatacaccaaggaaagtctacacgaaccctttggcaaaatcctgtatatcgtgcgaaaaaggatggatataccgaaaaaatcgctataatgaccccgaagcagggttatgcagcggaaaagatccgtc

SEQ ID NO: 59 - DNA, 12000 bp, Artificial Sequence
  pAWPSG-Po-nCas9-BE-pTac-RiboJ-sgRNA(McglgA4)
gaccctttccgacgctcaccgggctggttgccctcgccgctgggctggcggccgtctatggccctgcaaacgcgccagaaacgccgtcgaagccgtgtgcgagacaccgcggccgccggcgttgtggatacctcgcggaaaacttggccctcactgacagatgaggggcggacgttgacacttgaggggccgactcacccggcgcggcgttgacagatgaggggcaggctcgatttcggccggcgacgtggagctggccagcctcgcaaatcggcgaaaacgcctgattttacgcgagtttcccacagatgatgtggacaagcctggggataagtgccctgcggtattgacacttgaggggcgcgactactgacagatgaggggcgcgatccttgacacttgaggggcagagtgctgacagatgaggggcgcacctattgacatttgaggggctgtccacaggcagaaaatccagcatttgcaagggtttccgcccgtttttcggccaccgctaacctgtcttttaacctgcttttaaaccaatatttataaaccttgtttttaaccagggctgcgccctgtgcgcgtgaccgcgcacgccgaaggggggtgcccccccttctcgaaccctcccggcccgctaacgcgggcctcccatccccccaggggctgcgcccctcggccgcgaacggcctcaccccaaaaatggcagccaagctgacccgctagggacgtgaagtcgattccttcgatggttagcaatcaaagactcagagtgctgtctggagcgtgaatctaacggtacgtatctcgattgctcggtcgctattcgcactctgcgaaagttcgtaccgctcattcactaggttgcgaaaatttaaatcgtaattattggggacccctggattctcaccaataaaaaacgcccggcggcaaccgagcgttctgaacaaatccagatggagttctgaggtcattactggatctatcaacaggagtccaagactagtagcggataacaatttcacacaggattagccttcgatgccgattttcttcagccgataggccagtgccggtcggcttaggccgagcaagcgcgcggcaccggagacgttttggttggcctgttgcatggctttgcgcatcaggctttcctcgatctcgtcgaggctcaggccgctgctcaacaactggctgatccaactgccctggccattgcctggctgaatcagcacgccgtccgacgacacccgctcgctggcggtctgcggctcttccggcgcccgtgggaacagcgcctgcacgctgatgctttcgttcggatcggtgaggatgatgccgcgctcgatgacgttctccagctcacggatattgcccggccaactgtaatgcaggcaggcctccagggctttgtctgaaaggccgagggttctcttgccgtactcctggtggaagcgctgaaggaagtgctcaaccagcagtggaatgtcctcgcggcgttcgcgcaacgccgggatcgccaccgggaaaacgttcagccggtagtacaggtcggcgcgaaaacgcccggccttgaccgcttcggccaggtcctcgtgggtggctgcgataacccttacgtcgatcttgcgcgtgcggttgtcgccaactcgctccagctcgccttcttgcagcacgcgcagcaaactggcctgagcgcgcgggctgagttcgatcacctcgtcaaggaagatggtgcccttgtcggcccgctcgaagcggcccatgcgtgactgggtggcgccggtgaaggcgcctttttccacgccgaacaattcggactcgatcaggtccggcgggatcgccgcacagttcaccgcgacaaagggctcggcggcgcgtttgctgcgcaggtgcacgctacgcgcgatgacctccttgccgaccccggtctcgccaagcagcagcaccgagactttgccctgtgcggccttgtccatcatattgcgcacggtctggtaggccggggtctgaccgatgccgtagtactggccttcctgtttgtcgaggttggtacgcagcgacaccagttgcgattgcaactcgtagagttcctcgatgatggggtcgttcttgaaatactgtttgaagctggcaacgtcgtcccactcttcggccggcttgccaatgacccggcacttgtcgccgccgcagccgcggcagctgacttccttgaagatgatttcccggcccatgaacgccgaggaataggcgcaggcgtagccgagcagagtccagcacaccgggtcttgcatctgccccaggtcggtctggcagatttccacctcgaaggagtcgatccactccatctcggcatagaagcgcccgcattccttgtcgatatcgacctcggtggggcggaccttgaccagacccttgagcgaatgcagctgcgggccggcgaggaacatgtcgtactcgctggcattcggtctaagcttcctggccagttcggcatccttcaggccggactggtaaccctggcgcaggaagaagcccttggcgcgttcgatgcccagggtattgaccatttcccggcgaaagctggccattgctgaaacctgcagcaacagcatgcgttgttcgccaagccagatcttgccttccgtgctctggaagtggatcaggttggtcaggtccttgaaatcggagtgctggatttcaggcttgtacttgatcggcatgtaagcgaggcccctatttatttttagatggggaaatcagggtcgccgctatagcgcaaggcaggcggcgattccagatggggtcatggggaaaatcggcagttttttcacctgcgccagctccccatagccgacctcagtatctggcaaaagtcaaccaaatgatcaatcgacggcagtgactttagtgctagagatcagccttcagctgcgccatgagcatttgctcaagcggccttgggcaattgatcaaatgcttaaaaagcctgcgcaagcgcggcttaatttcgctcgctccgatcattctaaaaattagaaacacattgaaaaacaataccttgaagtcggttttcagaccttggcacagctgttgcactttgtcctgcgcaatccgccaacctggagatctagaaataattttgtttaactttaagaaggagatatacatatgagctcagagactggcccagtggctgtggaccccacattgagacggcggatcgagccccatgagtttgaggtattcttcgatccgagagagctccgcaaggagacctgcctgctttacgaaattaattgggggggccggcactccatttggcgacatacatcacagaacactaacaagcacgtcgaagtcaacttcatcgagaagttcacgacagaaagatatttctgtccgaacacaaggtgcagcattacctggtttctcagctggagcccatgcggcgaatgtagtagggccatcactgaattcctgtcaaggtatccccacgtcactctgtttatttacatcgcaaggctgtaccaccacgctgacccccgcaatcgacaaggcctgcgggatttgatctcttcaggtgtgactatccaaattatgactgagcaggagtcaggatactgctggagaaactttgtgaattatagcccgagtaatgaagcccactggcctaggtatccccatctgtgggtacgactgtacgttcttgaactgtactgcatcatactgggcctgcctccttgtctcaacattctgagaaggaagcagccacagctgacattctttaccatcgctcttcagtcttgtcattaccagcgactgcccccacacattctctgggccaccgggttgaaaagcggcagcgagactcccgggacctcagagtccgccacacccgaaagtgataagaaatactcaataggcttagctatcggcacaaatagcgtcggatgggcggtgatcactgatgaatataaggttccgtctaaaaagttcaaggttctgggaaatacagaccgccacagtatcaaaaaaaatcttataggggctcttttatttgacagtggagagacagcggaagcgactcgtctcaaacggacagctcgtagaaggtatacacgtcggaagaatcgtatttgttatctacaggagattttttcaaatgagatggcgaaagtagatgatagtttctttcatcgacttgaagagtcttttttggtggaagaagacaagaagcatgaacgtcatcctatttttggaaatatagtagatgaagttgcttatcatgagaaatatccaactatctatcatctgcgaaaaaaattggtagattctactgataaagcggatttgcgcttaatctatttggccttagcgcatatgattaagtttcgtggtcattttttgattgagggagatttaaatcctgataatagtgatgtggacaaactatttatccagttggtacaaacctacaatcaattatttgaagaaaaccctattaacgcaagtggagtagatgctaaagcgattctttctgcacgattgagtaaatcaagacgattagaaaatctcattgctcagctccccggtgagaagaaaaatggcttatttgggaatctcattgctttgtcattgggtttgacccctaattttaaatcaaattttgatttggcagaagatgctaaattacagctttcaaaagatacttacgatgatgatttagataatttattggcgcaaattggagatcaatatgctgatttgtttttggcagctaagaatttatcagatgctattttactttcagatatcctaagagtaaatactgaaataactaaggctcccctatcagcttcaatgattaaacgctacgatgaacatcatcaagacttgactcttttaaaagctttagttcgacaacaacttccagaaaagtataaagaaatcttttttgatcaatcaaaaaacggatatgcaggttatattgatgggggagctagccaagaagaattttataaatttatcaaaccaattttagaaaaaatggatggtactgaggaattattggtgaaactaaatcgtgaagatttgctgcgcaagcaacggacctttgacaacggctctattccccatcaaattcacttgggtgagctgcatgctattttgagaagacaagaagacttttatccatttttaaaagacaatcgtgagaagattgaaaaaatcttgacttttcgaattccttattatgttggtccattggcgcgtggcaatagtcgttttgcatggatgactcggaagtctgaagaaacaattaccccatggaattttgaagaagttgtcgataaaggtgcttcagctcaatcatttattgaacgcatgacaaactttgataaaaatcttccaaatgaaaaagtactaccaaaacatagtttgctttatgagtattttacggtttataacgaattgacaaaggtcaaatatgttactgaaggaatgcgaaaaccagcatttctttcaggtgaacagaagaaagccattgttgatttactcttcaaaacaaatcgaaaagtaaccgttaagcaattaaaagaagattatttcaaaaaaatagaatgttttgatagtgttgaaatttcaggagttgaagatagatttaatgcttcattaggtacctaccatgatttgctaaaaattattaaagataaagattttttggataatgaagaaaatgaagatatcttagaggatattgttttaacattgaccttatttgaagatagggagatgattgaggaaagacttaaaacatatgctcacctctttgatgataaggtgatgaaacagcttaaacgtcgccgttatactggttggggacgtttgtctcgaaaattgattaatggtattagggataagcaatctggcaaaacaatattagattttttgaaatcagatggttttgccaatcgcaattttatgcagctgatccatgatgatagtttgacatttaaagaagacattcaaaaagcacaagtgtctggacaaggcgatagtttacatgaacatattgcaaatttagctggtagccctgctattaaaaaaggtattttacagactgtaaaagttgttgatgaattggtcaaagtaatggggcggcataagccagaaaatatcgttattgaaatggcacgtgaaaatcagacaactcaaaagggccagaaaaattcgcgagagcgtatgaaacgaatcgaagaaggtatcaaagaattaggaagtcagattcttaaagagcatcctgttgaaaatactcaattgcaaaatgaaaagctctatctctattatctccaaaatggaagagacatgtatgtggaccaagaattagatattaatcgtttaagtgattatgatgtcgatcacattgttccacaaagtttccttaaagacgattcaatagacaataaggtcttaacgcgttctgataaaaatcgtggtaaatcggataacgttccaagtgaagaagtagtcaaaaagatgaaaaactattggagacaacttctaaacgccaagttaatcactcaacgtaagtttgataatttaacgaaagctgaacgtggaggtttgagtgaacttgataaagctggttttatcaaacgccaattggttgaaactcgccaaatcactaagcatgtggcacaaattttggatagtcgcatgaatactaaatacgatgaaaatgataaacttattcgagaggttaaagtgattaccttaaaatctaaattagtttctgacttccgaaaagatttccaattctataaagtacgtgagattaacaattaccatcatgcccatgatgcgtatctaaatgccgtcgttggaactgctttgattaagaaatatccaaaacttgaatcggagtttgtctatggtgattataaagtttatgatgttcgtaaaatgattgctaagtctgagcaagaaataggcaaagcaaccgcaaaatatttcttttactctaatatcatgaacttcttcaaaacagaaattacacttgcaaatggagagattcgcaaacgccctctaatcgaaactaatggggaaactggagaaattgtctgggataaagggcgagattttgccacagtgcgcaaagtattgtccatgccccaagtcaatattgtcaagaaaacagaagtacagacaggcggattctccaaggagtcaattttaccaaaaagaaattcggacaagcttattgctcgtaaaaaagactgggatccaaaaaaatatggtggttttgatagtccaacggtagcttattcagtcctagtggttgctaaggtggaaaaagggaaatcgaagaagttaaaatccgttaaagagttactagggatcacaattatggaaagaagttcctttgaaaaaaatccgattgactttttagaagctaaaggatataaggaagttaaaaaagacttaatcattaaactacctaaatatagtctttttgagttagaaaacggtcgtaaacggatgctggctagtgccggagaattacaaaaaggaaatgagctggctctgccaagcaaatatgtgaattttttatatttagctagtcattatgaaaagttgaagggtagtccagaagataacgaacaaaaacaattgtttgtggagcagcataagcattatttagatgagattattgagcaaatcagtgaattttctaagcgtgttattttagcagatgccaatttagataaagttcttagtgcatataacaaacatagagacaaaccaatacgtgaacaagcagaaaatattattcatttatttacgttgacgaatcttggagctcccgctgcttttaaatattttgatacaacaattgatcgtaaacgatatacgtctacaaaagaagttttagatgccactcttatccatcaatccatcactggtctttatgaaacacgcattgatttgagtcagctaggaggtgactctggtggttctactaatctgtcagatattattgaaaaggagaccggtaagcaactggttatccaggaatccatcctcatgctcccagaggaggtggaagaagtcattgggaacaagccggaaagcgatatactcgtgcacaccgcctacgacgagagcaccgacgagaatgtcatgcttctgactagcgacgcccctgaatacaagccttgggctctggtcatacaggatagcaacggtgagaacaagattaagatgctctaactgctgccaccgctgagcaaagctgctctgaaatgagctgttgacaattaatcatcggctcgtataatgtgtggactgcagctgtcaccggatgtgctttccggtctgatgagtccgtgaggacgaaacagcctctacaaataattttgtttaagtttccagccgaggccgagcgttttagagctagaaatagcaagttaaaataaggctagtccgttatcaacttgaaaaagtggcaccgagtcggtgctttttttgacccggggcggccgcctcgattaattaaaggcatcaaataaaacgaaaggctcagtcgaaagactgggcctttcgttttatctgttgtttgtcggtgaacgctctcctgagtaggacaaatccgccgccctagacagctgggcgcgccattgtcgggaagatgcgtgatctgatccttccactcagcaaaagttcgatttattcaacaaagccgccgtcccgtcaagtcagcgtaatgctctgccagtgttacaaccaattaaccaattctgattagaaaaactcatcgagcatcaaatgaaactgcaatttattcatatcaggattatcaataccatatttttgaaaaagccgtttctgtaatgaaggagaaaactcaccgaggcagttccataggatggcaagatcctggtatcggtctgcgattccgactcgtccaacatcaatacaacctattaatttcccctcgtcaaaaataaggttatcaagtgagaaatcaccatgagtgacgactgaatccggtgagaatggcaaaagcttatgcatttctttccagacttgttcaacaggccagccattacgctcgtcatcaaaatcactcgcatcaaccaaaccgttattcattcgtgattgcgcctgagcgagacgaaatacgcgatcgctgttaaaaggacaattacaaacaggaatcgaatgcaaccggcgcaggaacactgccagcgcatcaacaatattttcacctgaatcaggatattcttctaatacctggaatgctgttttcccggggatcgcagtggtgagtaaccatgcatcatcaggagtacggataaaatgcttgatggtcggaagaggcataaattccgtcagccagtttagtctgaccatctcatctgtaacatcattggcaacgctacctttgccatgtttcagaaacaactctggcgcatcgggcttcccatacaatcgatagattgtcgcacctgattgcccgacattatcgcgagcccatttatacccatataaatcagcatccatgttggaatttaatcgcggcctcgagcaagacgtttcccgttgaatatggctcataacaccccttgtattactgtttatgtaagcagacagttttattgttcatgatgatatatttttatcttgtgcaatgtaacatcagagattttgagacacaacgtggctttcgacttccggcaagctatacgcgccctagaattgtcaattttaatcctctgtttatcggcagttcgtagagcgcgccgtgcgtcccgagcgatactgagcgaagcaagtgcgtcgagcagtgcccgcttgttcctgaaatgccagtaaagcgctggctgctgaacccccagccggaactgaccccacaaggccctagcgtttgcaatgcaccaggtcatcattgacccaggcgtgttccaccaggccgctgcctcgcaactcttcgcaggcttcgccgacctgctcgcgccacttcttcacgcgggtggaatccgatccgcacatgaggcggaaggtttccagcttgagcgggtacggctcccggtgcgagctgaaatagtcgaacatccgtcgggccgtcggcgacagcttgcggtacttctcccatatgaatttcgtgtagtggtcgccagcaaacagcacgacgatttcctcgtcgatcaggacctggcaacgggacgttttcttgccacggtccaggacgcggaagcggtgcagcagcgacaccgattccaggtgcccaacgcggtcggacgtgaagcccatcgccgtcgcctgtaggcgcgacaggcattcctcggccttcgtgtaataccggccattgatcgaccagcccaggtcctggcaaagctcgtagaacgtgaaggtgatcggctcgccgataggggtgcgcttcgcgtactccaacacctgctgccacaccagttcgtcatcgtcggcccgcagctcgacgccggtgtaggtgatcttcacgtccttgttgacgtggaaaatgaccttgttttgcagcgcctcgcgcgggattttcttgttgcgcgtggtgaacagggcagagcgggccgtgtcgtttggcatcgctcgcatcgtgtccggccacggcgcaatatcgaacaaggaaagctgcatttccttgatctgctgcttcgtgtgtttcagcaacgcggcctgcttggcctcgctgacctgttttgccaggtcctcgccggcggtttttcgcttcttggtcgtcatagttcctcgcgtgtcgatggtcatcgacttcgccaaacctgccgcctcctgttcgagacgacgcgaacgctccacggcggccgatggcgcgggcagggcagggggagccagttgcacgctgtcgcgctcgatcttggccgtagcttgctggaccatcgagccgacggactggaaggtttcgcggggcgcacgcatgacggtgcggcttgcgatggtttcggcatcctcggcggaaaaccccgcgtcgatcagttcttgcctgtatgccttccggtcaaacgtccgattcattcaccctccttgcgggattgccccgactcacgccggggcaatgtgcccttattcctgatttgacccgcctggtgccttggtgtccagataatccaccttatcggcaatgaagtcggtcccgtagaccgtctggccgtccttctcgtacttggtattccgaatcttgccctgcacgaataccagctccgcgaagtcgctcttcttgatggagcgcatggggacgtgcttggcaatcacgcgcaccccccggccgttttagcggctaaaaaagtcatggctctgccctcgggcggaccacgcccatcatgaccttgccaagctcgtcctgcttctcttcgatcttcgccagcagggcgaggatcgtggcatcaccgaaccgcgccgtgcgcgggtcgtcggtgagccagagtttcagcaggccgcccaggcggcccaggtcgccattgatgcgggccagctcgcggacgtgctcatagtccacgacgcccgtgattttgtagccctggccgacggccagcaggtaggcctacaggctcatgccggccgccgccgccttttcctcaatcgctcttcgttcgtctggaaggcagtacaccttgataggtgggctgcccttcctggttggcttggtttcatcagccatccgcttgccctcatctgttacgccggcggtagccggccagcctcgcagagcaggattcccgttgagcaccgccaggtgcgaataagggacagtgaagaaggaacacccgctcgcgggtgggcctacttcacctatcctgcccggctgacgccgttggatacaccaaggaaagtctacacgaaccctttggcaaaatcctgtatatcgtgcgaaaaaggatggatataccgaaaaaatcgctataatgaccccgaagcagggttatgcagcggaaaagatccgtc

SEQ ID NO: 60 - DNA, 30 bp, Artificial Sequence
  DA-R
cgcttacatgaacgaccccatcatcgagga

SEQ ID NO: 61 - DNA, 30 bp, Artificial Sequence
  DA-F
tggggtcgttcatgtaagcgaggcccctat

SEQ ID NO: 62 - DNA, 20 bp, Artificial Sequence
  DmpR(PstI)-F
ggccattgctgaaacctgca

SEQ ID NO: 63 - DNA, 20 bp, Artificial Sequence
  RBS-R
tctagatctccaggttggcg

SEQ ID NO: 64 - DNA, 20 bp, Artificial Sequence
  dTomato(PstI)-R
gatcagcgtgccgtcctgca

SEQ ID NO: 65 - DNA, 76 bp, Artificial Sequence
  RBS(MDH)-F
cgccaacctggagatctagatgcagggtcggcatcaatcattcttggaggagacacatggtgagcaagggcgagga

SEQ ID NO: 66 - DNA, 76 bp, Artificial Sequence
  RBS(MmoX)-F
cgccaacctggagatctagacatcattcatagaatgtgttacggaggaaacaagtaatggtgagcaagggcgagga

SEQ ID NO: 67 - DNA, 76 bp, Artificial Sequence
  RBS(MmoY)-F
cgccaacctggagatctagacgttcgatcaacctcaaaccaaaaaggaacatcgatatggtgagcaagggcgagga

SEQ ID NO: 68 - DNA, 76 bp, Artificial Sequence
  RBS(MmoZ)-F
cgccaacctggagatctagatggacactttttcaacggcctgttaaggagaatgacatggtgagcaagggcgagga

SEQ ID NO: 69 - DNA, 76 bp, Artificial Sequence
  RBS(PmoA1)-F
cgccaacctggagatctagagaaaataagaaaacgacaaatttggaggtaactttaatggtgagcaagggcgagga

SEQ ID NO: 70 - DNA, 76 bp, Artificial Sequence
  RBS(PmoB1)-F
cgccaacctggagatctagagtgacccaacagcaagaactcgaaagaggagagatcatggtgagcaagggcgagga

SEQ ID NO: 71 - DNA, 76 bp, Artificial Sequence
  RBS(PmoC1)-F
cgccaacctggagatctagaggcccctgtcaaccatcactttaggaggaacaaacaatggtgagcaagggcgagga

SEQ ID NO: 72 - DNA, 76 bp, Artificial Sequence
  RBS(PmoC2)-F
cgccaacctggagatctagaccggtgttcacatcgatataacagttggaggtaaaaatggtgagcaagggcgagga

SEQ ID NO: 73 - DNA, 76 bp, Artificial Sequence
  RBS(PmoC3)-F
cgccaacctggagatctagagtggcatcaatccaacaccaactcaggagaaatcagatggtgagcaagggcgagga